European Patent Application EP 4 682 162 A1, published January 21, 2026. Title: TCR SPECIFICALLY RECOGNIZING PRAME ANTIGEN, AND CO-EXPRESSING SAME WITH CD8 FOR REDIRECTING CD4 T CELLS. Applicant: Neowise Biotechnology Co., Ltd. Application US. The sequence listing filed with the application follows.

SEQUENCE LISTING (550 sequences)

SEQ ID NO: 1 - protein, 6 aa, synthetic construct
DRVSQS

SEQ ID NO: 2 - protein, 6 aa, synthetic construct
IYSNGD

SEQ ID NO: 3 - protein, 9 aa, synthetic construct
AVDSSYKLI

SEQ ID NO: 4 - protein, 6 aa, synthetic construct
NSASQS

SEQ ID NO: 5 - protein, 6 aa, synthetic construct
VYSSGN

SEQ ID NO: 6 - protein, 10 aa, synthetic construct
VVTQAGTALI

SEQ ID NO: 7 - protein, 7 aa, synthetic construct
TISGTDY

SEQ ID NO: 8 - protein, 5 aa, synthetic construct
GLTSN

SEQ ID NO: 9 - protein, 12 aa, synthetic construct
ILRAGGSGDKLT

SEQ ID NO: 10 - protein, 6 aa, synthetic construct
DRGSQS

SEQ ID NO: 11 - protein, 6 aa, synthetic construct
IYSNGD

SEQ ID NO: 12 - protein, 11 aa, synthetic construct
AVLRSNDYKLS

SEQ ID NO: 13 - protein, 6 aa, synthetic construct
SSYSPS

SEQ ID NO: 14 - protein, 8 aa, synthetic construct
YTSAATLV

SEQ ID NO: 15 - protein, 11 aa, synthetic construct
VVSITGFQKLV

SEQ ID NO: 16 - protein, 6 aa, synthetic construct
DSSSTY

SEQ ID NO: 17 - protein, 7 aa, synthetic construct
IFSNMDM

SEQ ID NO: 18 - protein, 14 aa, synthetic construct
AESVGYGGSQGNLI

SEQ ID NO: 19 - protein, 6 aa, synthetic construct
DRGSQS

SEQ ID NO: 20 - protein, 6 aa, synthetic construct
IYSNGD

SEQ ID NO: 21 - protein, 12 aa, synthetic construct
AVPGGTSYGKLT

SEQ ID NO: 22 - protein, 5 aa, synthetic construct
KALYS

SEQ ID NO: 23 - protein, 7 aa, synthetic construct
LLKGGEQ

SEQ ID NO: 24 - protein, 14 aa, synthetic construct
GTESGRGSTLGRLY

SEQ ID NO: 25 - protein, 5 aa, synthetic construct
TSINN

SEQ ID NO: 26 - protein, 7 aa, synthetic construct
IRSNERE

SEQ ID NO: 27 - protein, 11 aa, synthetic construct
ATLTLNDYKLS

SEQ ID NO: 28 - protein, 5 aa, synthetic construct
SIFNT

SEQ ID NO: 29 - protein, 7 aa, synthetic construct
LYKAGEL

SEQ ID NO: 30 - protein, 11 aa, synthetic construct
AGQASGTYKYI

SEQ ID NO: 31 - protein, 6 aa, synthetic construct
DRGSQS

SEQ ID NO: 32 - protein, 6 aa, synthetic construct
IYSNGD

SEQ ID NO: 33 - protein, 9 aa, synthetic construct
AGHTGNQFY

SEQ ID NO: 34 - protein, 5 aa, synthetic construct
VGISA

SEQ ID NO: 35 - protein, 5 aa, synthetic construct
LSSGK

SEQ ID NO: 36 - protein, 11 aa, synthetic construct
ALNSDSNYQLI

SEQ ID NO: 37 - protein, 5 aa, synthetic construct
SIFNT

SEQ ID NO: 38 - protein, 7 aa, synthetic construct
LYKAGEL

SEQ ID NO: 39 - protein, 9 aa, synthetic construct
AGPEDDKII

SEQ ID NO: 40 - protein, 5 aa, synthetic construct
SVFSS

SEQ ID NO: 41 - protein, 7 aa, synthetic construct
VVTGGEV

SEQ ID NO: 42 - protein, 11 aa, synthetic construct
AGVDNYGQNFV

SEQ ID NO: 43 - protein, 6 aa, synthetic construct
DRGSQS

SEQ ID NO: 44 - protein, 6 aa, synthetic construct
IYSNGD

SEQ ID NO: 45 - protein, 10 aa, synthetic construct
AVNTGFQKLV

SEQ ID NO: 46 - protein, 5 aa, synthetic construct
DSVNN

SEQ ID NO: 47 - protein, 5 aa, synthetic construct
IPSGT

SEQ ID NO: 48 - protein, 11 aa, synthetic construct
AVMPSGTYKYI

SEQ ID NO: 49 - protein, 6 aa, synthetic construct
NSMFDY

SEQ ID NO: 50 - protein, 7 aa, synthetic construct
ISSIKDK

SEQ ID NO: 51 - protein, 11 aa, synthetic construct
AASGVRGQNFV

SEQ ID NO: 52 - protein, 5 aa, synthetic construct
KTLYG

SEQ ID NO: 53 - protein, 7 aa, synthetic construct
LQKGGEE

SEQ ID NO: 54 - protein, 11 aa, synthetic construct
GADVINDYKLS

SEQ ID NO: 55 - protein, 6 aa, synthetic construct
NSASQS

SEQ ID NO: 56 - protein, 6 aa, synthetic construct
VYSSGN

SEQ ID NO: 57 - protein, 11 aa, synthetic construct
VVNRGSQGNLI

SEQ ID NO: 58 - protein, 6 aa, synthetic construct
YGGTVN

SEQ ID NO: 59 - protein, 8 aa, synthetic construct
YFSGDPLV

SEQ ID NO: 60 - protein, 11 aa, synthetic construct
AVKMDSSYKLI

SEQ ID NO: 61 - protein, 6 aa, synthetic construct
TSGFYG

SEQ ID NO: 62 - protein, 6 aa, synthetic construct
NALDGL

SEQ ID NO: 63 - protein, 9 aa, synthetic construct
ALGTEDKII

SEQ ID NO: 64 - protein, 7 aa, synthetic construct
TSENNYY

SEQ ID NO: 65 - protein, 8 aa, synthetic construct
QEAYKQQN

SEQ ID NO: 66 - protein, 9 aa, synthetic construct
AFDNNARLM

SEQ ID NO: 67 - protein, 5 aa, synthetic construct
SIFNT

SEQ ID NO: 68 - protein, 7 aa, synthetic construct
LYKAGEL

SEQ ID NO: 69 - protein, 12 aa, synthetic construct
AGFSQGGSEKLV

SEQ ID NO: 70 - protein, 5 aa, synthetic construct
DSVNN

SEQ ID NO: 71 - protein, 5 aa, synthetic construct
IPSGT

SEQ ID NO: 72 - protein, 11 aa, synthetic construct
AVLAPGTYKYI

SEQ ID NO: 73 - protein, 5 aa, synthetic construct
TSINN

SEQ ID NO: 74 - protein, 7 aa, synthetic construct
IRSNERE

SEQ ID NO: 75 - protein, 13 aa, synthetic construct
ATDLSGAGSYQLT

SEQ ID NO: 76 - protein, 6 aa, synthetic construct
DRVSQS

SEQ ID NO: 77 - protein, 6 aa, synthetic construct
IYSNGD

SEQ ID NO: 78 - protein, 11 aa, synthetic construct
AVVSSNDYKLS

SEQ ID NO: 79 - protein, 6 aa, synthetic construct
DRVSQS

SEQ ID NO: 80 - protein, 6 aa, synthetic construct
IYSNGD

SEQ ID NO: 81 - protein, 11 aa, synthetic construct
AVASGGSYIPT

SEQ ID NO: 82 - protein, 6 aa, synthetic construct
NSASDY

SEQ ID NO: 83 - protein, 7 aa, synthetic construct
IRSNMDK

SEQ ID NO: 84 - protein, 9 aa, synthetic construct
AESYGQKLL

SEQ ID NO: 85 - protein, 5 aa, synthetic construct
SIFNT

SEQ ID NO: 86 - protein, 7 aa, synthetic construct
LYKAGEL

SEQ ID NO: 87 - protein, 13 aa, synthetic construct
AGQDDGGSQGNLI

SEQ ID NO: 88 - protein, 5 aa, synthetic construct
KALYS

SEQ ID NO: 89 - protein, 7 aa, synthetic construct
LLKGGEQ

SEQ ID NO: 90 - protein, 11 aa, synthetic construct
GTEFRNDYKLS

SEQ ID NO: 91 - protein, 5 aa, synthetic construct
TSINN

SEQ ID NO: 92 - protein, 7 aa, synthetic construct
IRSNERE

SEQ ID NO: 93 - protein, 11 aa, synthetic construct
ATDVKSSYKLI

SEQ ID NO: 94 - protein, 6 aa, synthetic construct
NSMFDY

SEQ ID NO: 95 - protein, 7 aa, synthetic construct
ISSIKDK

SEQ ID NO: 96 - protein, 12 aa, synthetic construct
AAFASDSNYQLI

SEQ ID NO: 97 - protein, 6 aa, synthetic construct
DRVSQS

SEQ ID NO: 98 - protein, 6 aa, synthetic construct
IYSNGD

SEQ ID NO: 99 - protein, 10 aa, synthetic construct
ALVSGTYKYI

SEQ ID NO: 100 - protein, 5 aa, synthetic construct
TSINN

SEQ ID NO: 101 - protein, 7 aa, synthetic construct
IRSNERE

SEQ ID NO: 102 - protein, 10 aa, synthetic construct
ATYANDYKLS

SEQ ID NO: 103 - protein, 6 aa, synthetic construct
NSMFDY

SEQ ID NO: 104 - protein, 7 aa, synthetic construct
ISSIKDK

SEQ ID NO: 105 - protein, 8 aa, synthetic construct
AAKPDKLI

SEQ ID NO: 106 - protein, 6 aa, synthetic construct
DRGSQS

SEQ ID NO: 107 - protein, 6 aa, synthetic construct
IYSNGD

SEQ ID NO: 108 - protein, 9 aa, synthetic construct
AVPSGNMLT

SEQ ID NO: 109 - protein, 5 aa, synthetic construct
KTLYG

SEQ ID NO: 110 - protein, 7 aa, synthetic construct
LQKGGEE

SEQ ID NO: 111 - protein, 11 aa, synthetic construct
GAVPINDYKLS

SEQ ID NO: 112 - protein, 6 aa, synthetic construct
DRGSQS

SEQ ID NO: 113 - protein, 6 aa, synthetic construct
IYSNGD

SEQ ID NO: 114 - protein, 11 aa, synthetic construct
AVVSGGYNKLI

SEQ ID NO: 115 - protein, 91 aa, synthetic construct
QKEVEQNSGPLSVPEGAIASLNCTYSDRVSQSFFWYRQYSGKSPELIMSIYSNGDKEDGRFTAQLNKASQYVSLLIRDSQPSDSATYLCAV

SEQ ID NO: 116 - protein, 90 aa, synthetic construct
RKEVEQDPGPFNVPEGATVAFNCTYSNSASQSFFWYRQDCRKEPKLLMSVYSSGNEDGRFTAQLNRASQYISLLIRDSKLSDSATYLCVV

SEQ ID NO: 117 - protein, 90 aa, synthetic construct
DAKTTQPNSMESNEEEPVHLPCNHSTISGTDYIHWYRQLPSQGPEYVIHGLTSNVNNRMASLAIAEDRKSSTLILHRATLRDAAVYYCIL

SEQ ID NO: 118 - protein, 91 aa, synthetic construct
QKEVEQNSGPLSVPEGAIASLNCTYSDRGSQSFFWYRQYSGKSPELIMSIYSNGDKEDGRFTAQLNKASQYVSLLIRDSQPSDSATYLCAV

SEQ ID NO: 119 - protein, 93 aa, synthetic construct
AQSVTQLDSHVSVSEGTPVLLRCNYSSSYSPSLFWYVQHPNKGLQLLLKYTSAATLVKGINGFEAEFKKSETSFHLTKPSAHMSDAAEYFCVV

SEQ ID NO: 120 - protein, 91 aa, synthetic construct
GEDVEQSLFLSVREGDSSVINCTYTDSSSTYLYWYKQEPGAGLQLLTYIFSNMDMKQDQRLTVLLNKKDKHLSLRIADTQTGDSAIYFCAE

SEQ ID NO: 121 - protein, 91 aa, synthetic construct
QKEVEQNSGPLSVPEGAIASLNCTYSDRGSQSFFWYRQYSGKSPELIMFIYSNGDKEDGRFTAQLNKASQYVSLLIRDSQPSDSATYLCAV

SEQ ID NO: 122 - protein, 87 aa, synthetic construct
QQPVQSPQAVILREGEDAVINCSSSKALYSVHWYRQKHGEAPVFLMILLKGGEQKGHDKISASFNEKKQQSSLYLTASQLSYSGTYF

SEQ ID NO: 123 - protein, 91 aa, synthetic construct
SQQGEEDPQALSIQEGENATMNCSYKTSINNLQWYRQNSGRGLVHLILIRSNEREKHSGRLRVTLDTSKKSSSLLITASRAADTASYFCAT

SEQ ID NO: 124 - protein, 90 aa, synthetic construct
GQQLNQSPQSMFIQEGEDVSMNCTSSSIFNTWLWYKQDPGEGPVLLIALYKAGELTSNGRLTAQFGITRKDSFLNISASIPSDVGIYFCA

SEQ ID NO: 125 - protein, 90 aa, synthetic construct
QKEVEQNSGPLSVPEGAIASLNCTYSDRGSQSFFWYRQYSGKSPELIMFIYSNGDKEDGRFTAQLNKASQYVSLLIRDSQPSDSATYLCA

SEQ ID NO: 126 - protein, 88 aa, synthetic construct
KNEVEQSPQNLTAQEGEFITINCSYSVGISALHWLQQHPGGGIVSLFMLSSGKKKHGRLIATINIQEKHSSLHITASHPRDSAVYICA

SEQ ID NO: 127 - protein, 90 aa, synthetic construct; identical to SEQ ID NO: 124

SEQ ID NO: 128 - protein, 91 aa, synthetic construct
TQLLEQSPQFLSIQEGENLTVYCNSSSVFSSLQWYRQEPGEGPVLLVTVVTGGEVKKLKRLTFQFGDARKDSSLHITAAQPGDTGLYLCAG

SEQ ID NO: 129 - protein, 92 aa, synthetic construct
QKEVEQNSGPLSVPEGAIASLNCTYSDRGSQSFFWYRQYSGKSPELIMFIYSNGDKEDGRFTAQLNKASQYVSLLIRDSQPSDSATYLCAVN

SEQ ID NO: 130 - protein, 89 aa, synthetic construct
GIQVEQSPPDLILQEGANSTLRCNFSDSVNNLQWFHQNPWGQLINLFYIPSGTKQNGRLSATTVATERYSLLYISSSQTTDSGVYFCAV

SEQ ID NO: 131 - protein, 92 aa, synthetic construct
DQQVKQNSPSLSVQEGRISILNCDYTNSMFDYFLWYKKYPAEGPTFLISISSIKDKNEDGRFTVFLNKSAKHLSLHIVPSQPGDSAVYFCAA

SEQ ID NO: 132 - protein, 92 aa, synthetic construct
SQELEQSPQSLIVQEGKNLTINCTSSKTLYGLYWYKQKYGEGLIFLMMLQKGGEEKSHEKITAKLDEKKQQSSLHITASQPSHAGIYLCGAD

SEQ ID NO: 133 - protein, 91 aa, synthetic construct
RKEVEQDPGPFNVPEGATVAFNCTYSNSASQSFFWYRQDCRKEPKLLMSVYSSGNEDGRFTAQLNRASQYISLLIRDSKLSDSATYLCVVN

SEQ ID NO: 134 - protein, 93 aa, synthetic construct
AQSVSQHNHHVILSEAASLELGCNYSYGGTVNLFWYVQYPGQHLQLLLKYFSGDPLVKGIKGFEAEFIKSKFSFNLRKPSVQWSDTAEYFCAV

SEQ ID NO: 135 - protein, 89 aa, synthetic construct
GQSLEQPSEVTAVEGAIVQINCTYQTSGFYGLSWYQQHDGGAPTFLSYNALDGLEETGRFSSFLSRSDSYGYLLLQELQMKDSASYFCA

SEQ ID NO: 136 - protein, 94 aa, synthetic construct
AQTVTQSQPEMSVQEAETVTLSCTYDTSENNYYLFWYKQPPSRQMILVIRQEAYKQQNATENRFSVNFQKAAKSFSLKISDSQLGDTAMYFCAF

SEQ ID NO: 137 - protein, 90 aa, synthetic construct; identical to SEQ ID NO: 124

SEQ ID NO: 138 - protein, 89 aa, synthetic construct; identical to SEQ ID NO: 130

SEQ ID NO: 139 - protein, 92 aa, synthetic construct
SQQGEEDPQALSIQEGENATMNCSYKTSINNLQWYRQNSGRGLVHLILIRSNEREKHSGRLRVTLDTSKKSSSLLITASRAADTASYFCATD

SEQ ID NO: 140 - protein, 91 aa, synthetic construct; identical to SEQ ID NO: 115

SEQ ID NO: 141 - protein, 91 aa, synthetic construct; identical to SEQ ID NO: 115

SEQ ID NO: 142 - protein, 92 aa, synthetic construct
GESVGLHLPTLSVQEGDNSIINCAYSNSASDYFIWYKQESGKGPQFIIDIRSNMDKRQGQRVTVLLNKTVKHLSLQIAATQPGDSAVYFCAE

SEQ ID NO: 143 - protein, 92 aa, synthetic construct
GQQLNQSPQSMFIQEGEDVSMNCTSSSIFNTWLWYKQDPGEGPVLLIALYKAGELTSNGRLTAQFGITRKDSFLNISASIPSDVGIYFCAGQ

SEQ ID NO: 144 - protein, 87 aa, synthetic construct; identical to SEQ ID NO: 122

SEQ ID NO: 145 - protein, 92 aa, synthetic construct; identical to SEQ ID NO: 139

SEQ ID NO: 146 - protein, 92 aa, synthetic construct; identical to SEQ ID NO: 131

SEQ ID NO: 147 - protein, 90 aa, synthetic construct
QKEVEQNSGPLSVPEGAIASLNCTYSDRVSQSFFWYRQYSGKSPELIMSIYSNGDKEDGRFTAQLNKASQYVSLLIRDSQPSDSATYLCA

SEQ ID NO: 148 - protein, 91 aa, synthetic construct; identical to SEQ ID NO: 123

SEQ ID NO: 149 - protein, 92 aa, synthetic construct; identical to SEQ ID NO: 131

SEQ ID NO: 150 - protein, 90 aa, synthetic construct
QKEVEQNSGPLSVPEGAIASLNCTYSDRGSQSFFWYRQYSGKSPELIMSIYSNGDKEDGRFTAQLNKASQYVSLLIRDSQPSDSATYLCA

SEQ ID NO: 151 - protein, 91 aa, synthetic construct
SQELEQSPQSLIVQEGKNLTINCTSSKTLYGLYWYKQKYGEGLIFLMMLQKGGEEKSHEKITAKLDEKKQQSSLHITASQPSHAGIYLCGA

SEQ ID NO: 152 - protein, 90 aa, synthetic construct; identical to SEQ ID NO: 150

SEQ ID NO: 153 - DNA, 273 bp, synthetic construct
  source 1..273: mol_type = other DNA
cagaaggaggtggagcagaattctggacccctcagtgttccagagggagccattgcctctctcaactgcacttacagtgaccgagtttcccagtccttcttctggtacagacaatattctgggaaaagccctgagttgataatgtccatatactccaatggtgacaaagaagatggaaggtttacagcacagctcaataaagccagccagtatgtttctctgctcatcagagactcccagcccagtgattcagccacctacctctgtgccgtg

SEQ ID NO: 154 - DNA, 270 bp, synthetic construct
  source 1..270: mol_type = other DNA
cggaaggaggtggagcaggatcctggacccttcaatgttccagagggagccactgtcgctttcaactgtacttacagcaacagtgcttctcagtctttcttctggtacagacaggattgcaggaaagaacctaagttgctgatgtccgtatactccagtggtaatgaagatggaaggtttacagcacagctcaatagagccagccagtatatttccctgctcatcagagactccaagctcagtgattcagccacctacctctgtgtggtg

SEQ ID NO: 155 - DNA, 270 bp, synthetic construct
  source 1..270: mol_type = other DNA
gatgctaagaccacacagccaaattcaatggagagtaacgaagaagagcctgttcacttgccttgtaaccactccacaatcagtggaactgattacatacattggtatcgacagcttccctcccagggtccagagtacgtgattcatggtcttacaagcaatgtgaacaacagaatggcctctctggcaatcgctgaagacagaaagtccagtaccttgatcctgcaccgtgctaccttgagagatgctgctgtgtactactgcatcctg

SEQ ID NO: 156 - DNA, 273 bp, synthetic construct
  source 1..273: mol_type = other DNA
cagaaggaggtggagcagaattctggacccctcagtgttccagagggagccattgcctctctcaactgcacttacagtgaccgaggttcccagtccttcttctggtacagacaatattctgggaaaagccctgagttgataatgtccatatactccaatggtgacaaagaagatggaaggtttacagcacagctcaataaagccagccagtatgtttctctgctcatcagagactcccagcccagtgattcagccacctacctctgtgccgtg

SEQ ID NO: 157 - DNA, 279 bp, synthetic construct
  source 1..279: mol_type = other DNA
gcccagtcggtgacccagcttgacagccacgtctctgtctctgaaggaaccccggtgctgctgaggtgcaactactcatcttcttattcaccatctctcttctggtatgtgcaacaccccaacaaaggactccagcttctcctgaagtacacatcagcggccaccctggttaaaggcatcaacggttttgaggctgaatttaagaagagtgaaacctccttccacctgacgaaaccctcagcccatatgagcgacgcggctgagtacttctgtgttgtg

SEQ ID NO: 158 - DNA, 273 bp, synthetic construct
  source 1..273: mol_type = other DNA
ggagaggatgtggagcagagtcttttcctgagtgtccgagagggagacagctccgttataaactgcacttacacagacagctcctccacctacttatactggtataagcaagaacctggagcaggtctccagttgctgacgtatattttttcaaatatggacatgaaacaagaccaaagactcactgttctattgaataaaaaggataaacatctgtctctgcgcattgcagacacccagactggggactcagctatctacttctgtgcagag

SEQ ID NO: 159 - DNA, 273 bp, synthetic construct
  source 1..273: mol_type = other DNA
cagaaggaggtggagcagaattctggacccctcagtgttccagagggagccattgcctctctcaactgcacttacagtgaccgaggttcccagtccttcttctggtacagacaatattctgggaaaagccctgagttgataatgttcatatactccaatggtgacaaagaagatggaaggtttacagcacagctcaataaagccagccagtatgtttctctgctcatcagagactcccagcccagtgattcagccacctacctctgtgccgtg

SEQ ID NO: 160 - DNA, 261 bp, synthetic construct
  source 1..261: mol_type = other DNA
caacaaccagtgcagagtcctcaagccgtgatcctccgagaaggggaagatgctgtcatcaactgcagttcctccaaggctttatattctgtacactggtacaggcagaagcatggtgaagcacccgtcttcctgatgatattactgaagggtggagaacagaagggtcatgacaaaatatctgcttcatttaatgaaaaaaagcagcaaagctccctgtaccttacggcctcccagctcagttactcaggaacctacttc

SEQ ID NO: 161 - DNA, 273 bp, synthetic construct
  source 1..273: mol_type = other DNA
agtcaacagggagaagaggatcctcaggccttgagcatccaggagggtgaaaatgccaccatgaactgcagttacaaaactagtataaacaatttacagtggtatagacaaaattcaggtagaggccttgtccacctaattttaatacgttcaaatgaaagagagaaacacagtggaagattaagagtcacgcttgacacttccaagaaaagcagttccttgttgatcacggcttcccgggcagcagacactgcttcttacttctgtgctacg

SEQ ID NO: 162 - DNA, 270 bp, synthetic construct
  source 1..270: mol_type = other DNA
ggtcaacagctgaatcagagtcctcaatctatgtttatccaggaaggagaagatgtctccatgaactgcacttcttcaagcatatttaacacctggctatggtacaagcaggaccctggggaaggtcctgtcctcttgatagccttatataaggctggtgaattgacctcaaatggaagactgactgctcagtttggtataaccagaaaggacagcttcctgaatatctcagcatccatacctagtgatgtaggcatctacttctgtgct

SEQ ID NO: 163 - DNA, 270 bp, synthetic construct
  source 1..270: mol_type = other DNA
cagaaggaggtggagcagaattctggacccctcagtgttccagagggagccattgcctctctcaactgcacttacagtgaccgaggttcccagtccttcttctggtacagacaatattctgggaaaagccctgagttgataatgttcatatactccaatggtgacaaagaagatggaaggtttacagcacagctcaataaagccagccagtatgtttctctgctcatcagagactcccagcccagtgattcagccacctacctctgtgcc

SEQ ID NO: 164 - DNA, 264 bp, synthetic construct
  source 1..264: mol_type = other DNA
aaaaatgaagtggagcagagtcctcagaacctgactgcccaggaaggagaatttatcacaatcaactgcagttactcggtaggaataagtgccttacactggctgcaacagcatccaggaggaggcattgtttccttgtttatgctgagctcagggaagaagaagcatggaagattaattgccacaataaacatacaggaaaagcacagctccctgcacatcacagcctcccatcccagagactctgccgtctacatctgtgct

SEQ ID NO: 165 - DNA, 270 bp, synthetic construct; identical to SEQ ID NO: 162
  source 1..270: mol_type = other DNA

SEQ ID NO: 166 - DNA, 273 bp, synthetic construct
  source 1..273: mol_type = other DNA
acccagctgctggagcagagccctcagtttctaagcatccaagagggagaaaatctcactgtgtactgcaactcctcaagtgttttttccagcttacaatggtacagacaggagcctggggaaggtcctgtcctcctggtgacagtagttacgggtggagaagtgaagaagctgaagagactaacctttcagtttggtgatgcaagaaaggacagttctctccacatcactgcggcccagcctggtgatacaggcctctacctctgtgcagga

SEQ ID NO: 167 - DNA, 276 bp, synthetic construct
  source 1..276: mol_type = other DNA
cagaaggaggtggagcagaattctggacccctcagtgttccagagggagccattgcctctctcaactgcacttacagtgaccgaggttcccagtccttcttctggtacagacaatattctgggaaaagccctgagttgataatgttcatatactccaatggtgacaaagaagatggaaggtttacagcacagctcaataaagccagccagtatgtttctctgctcatcagagactcccagcccagtgattcagccacctacctctgtgccgtgaac

SEQ ID NO: 168 - DNA, 267 bp, synthetic construct
  source 1..267: mol_type = other DNA
ggaatacaagtggagcagagtcctccagacctgattctccaggagggagccaattccacgctgcggtgcaatttttctgactctgtgaacaatttgcagtggtttcatcaaaacccttggggacagctcatcaacctgttttacattccctcagggacaaaacagaatggaagattaagcgccacgactgtcgctacggaacgctacagcttattgtacatttcctcttcccagaccacagactcaggcgtttatttctgtgctgtg

SEQ ID NO: 169 - DNA, 276 bp, synthetic construct
  source 1..276: mol_type = other DNA
gaccagcaagttaagcaaaattcaccatccctgagcgtccaggaaggaagaatttctattctgaactgtgactatactaacagcatgtttgattatttcctatggtacaaaaaataccctgctgaaggtcctacattcctgatatctataagttccattaaggataaaaatgaagatggaagattcactgttttcttaaacaaaagtgccaagcacctctctctgcacattgtgccctcccagcctggagactctgcagtgtacttctgtgcagca

SEQ ID NO: 170 - DNA, 276 bp, synthetic construct
  source 1..276: mol_type = other DNA
agccaagaactggagcagagtcctcagtccttgatcgtccaagagggaaagaatctcaccataaactgcacgtcatcaaagacgttatatggcttatactggtataagcaaaagtatggtgaaggtcttatcttcttgatgatgctacagaaaggtggggaagagaaaagtcatgaaaagataactgccaagttggatgagaaaaagcagcaaagttccctgcatatcacagcctcccagcccagccatgcaggcatctacctctgtggagcagac

SEQ ID NO: 171 - DNA, 273 bp, synthetic construct
  source 1..273: mol_type = other DNA
cggaaggaggtggagcaggatcctggacccttcaatgttccagagggagccactgtcgctttcaactgtacttacagcaacagtgcttctcagtctttcttctggtacagacaggattgcaggaaagaacctaagttgctgatgtccgtatactccagtggtaatgaagatggaaggtttacagcacagctcaatagagccagccagtatatttccctgctcatcagagactccaagctcagtgattcagccacctacctctgtgtggtgaac

SEQ ID NO: 172 - DNA, 279 bp, synthetic construct
  source 1..279: mol_type = other DNA
gcccagtctgtgagccagcataaccaccacgtaattctctctgaagcagcctcactggagttgggatgcaactattcctatggtggaactgttaatctcttctggtatgtccagtaccctggtcaacaccttcagcttctcctcaagtacttttcaggggatccactggttaaaggcatcaagggctttgaggctgaatttataaagagtaaattctcctttaatctgaggaaaccctctgtgcagtggagtgacacagctgagtacttctgtgccgtg

SEQ ID NO: 173 - DNA, 267 bp, synthetic construct
  source 1..267: mol_type = other DNA
ggacaaagccttgagcagccctctgaagtgacagctgtggaaggagccattgtccagataaactgcacgtaccagacatctgggttttatgggctgtcctggtaccagcaacatgatggcggagcacccacatttctttcttacaatgctctggatggtttggaggagacaggtcgtttttcttcattccttagtcgctctgatagttatggttacctccttctacaggagctccagatgaaagactctgcctcttacttctgcgct

SEQ ID NO: 174 - DNA, 282 bp, synthetic construct
  source 1..282: mol_type = other DNA
gcccagacagtcactcagtctcaaccagagatgtctgtgcaggaggcagagactgtgaccctgagttgcacatatgacaccagtgagaataattattatttgttctggtacaagcagcctcccagcaggcagatgattctcgttattcgccaagaagcttataagcaacagaatgcaacggagaatcgtttctctgtgaacttccagaaagcagccaaatccttcagtctcaagatctcagactcacagctgggggacactgcgatgtatttctgtgctttc

SEQ ID NO: 175 - DNA, 270 bp, synthetic construct; identical to SEQ ID NO: 162
  source 1..270: mol_type = other DNA

SEQ ID NO: 176 - DNA, 267 bp, synthetic construct; identical to SEQ ID NO: 168
  source 1..267: mol_type = other DNA

SEQ ID NO: 177 - DNA, 276 bp, synthetic construct
  source 1..276: mol_type = other DNA
agtcaacagggagaagaggatcctcaggccttgagcatccaggagggtgaaaatgccaccatgaactgcagttacaaaactagtataaacaatttacagtggtatagacaaaattcaggtagaggccttgtccacctaattttaatacgttcaaatgaaagagagaaacacagtggaagattaagagtcacgcttgacacttccaagaaaagcagttccttgttgatcacggcttcccgggcagcagacactgcttcttacttctgtgctacggac

SEQ ID NO: 178 - DNA, 273 bp, synthetic construct; identical to SEQ ID NO: 153
  source 1..273: mol_type = other DNA

SEQ ID NO: 179 - DNA, 273 bp, synthetic construct; identical to SEQ ID NO: 153
  source 1..273: mol_type = other DNA

SEQ ID NO: 180 - DNA, 276 bp, synthetic construct
  source 1..276: mol_type = other DNA
ggagagagtgtggggctgcatcttcctaccctgagtgtccaggagggtgacaactctattatcaactgtgcttattcaaacagcgcctcagactacttcatttggtacaagcaagaatctggaaaaggtcctcaattcattatagacattcgttcaaatatggacaaaaggcaaggccaaagagtcaccgttttattgaataagacagtgaaacatctctctctgcaaattgcagctactcaacctggagactcagctgtctacttttgtgcagag

SEQ ID NO: 181 - DNA, 276 bp, synthetic construct
  source 1..276: mol_type = other DNA
ggtcaacagctgaatcagagtcctcaatctatgtttatccaggaaggagaagatgtctccatgaactgcacttcttcaagcatatttaacacctggctatggtacaagcaggaccctggggaaggtcctgtcctcttgatagccttatataaggctggtgaattgacctcaaatggaagactgactgctcagtttggtataaccagaaaggacagcttcctgaatatctcagcatccatacctagtgatgtaggcatctacttctgtgctgggcag

SEQ ID NO: 182 - DNA, 261 bp, synthetic construct; identical to SEQ ID NO: 160
  source 1..261: mol_type = other DNA

SEQ ID NO: 183 - DNA, 276 bp, synthetic construct; identical to SEQ ID NO: 177
  source 1..276: mol_type = other DNA

SEQ ID NO: 184 - DNA, 276 bp, synthetic construct; identical to SEQ ID NO: 169
  source 1..276: mol_type = other DNA

SEQ ID NO: 185 - DNA, 270 bp, synthetic construct
  source 1..270: mol_type = other DNA
cagaaggaggtggagcagaattctggacccctcagtgttccagagggagccattgcctctctcaactgcacttacagtgaccgagtttcccagtccttcttctggtacagacaatattctgggaaaagccctgagttgataatgtccatatactccaatggtgacaaagaagatggaaggtttacagcacagctcaataaagccagccagtatgtttctctgctcatcagagactcccagcccagtgattcagccacctacctctgtgcc

SEQ ID NO: 186 - DNA, 273 bp, synthetic construct; identical to SEQ ID NO: 161
  source 1..273: mol_type = other DNA

SEQ ID NO: 187 - DNA, 276 bp, synthetic construct; identical to SEQ ID NO: 169
  source 1..276: mol_type = other DNA

SEQ ID NO: 188 - DNA, 270 bp, synthetic construct
  source 1..270: mol_type = other DNA
cagaaggaggtggagcagaattctggacccctcagtgttccagagggagccattgcctctctcaactgcacttacagtgaccgaggttcccagtccttcttctggtacagacaatattctgggaaaagccctgagttgataatgtccatatactccaatggtgacaaagaagatggaaggtttacagcacagctcaataaagccagccagtatgtttctctgctcatcagagactcccagcccagtgattcagccacctacctctgtgcc

SEQ ID NO: 189 - DNA, 273 bp, synthetic construct
  source 1..273: mol_type = other DNA
agccaagaactggagcagagtcctcagtccttgatcgtccaagagggaaagaatctcaccataaactgcacgtcatcaaagacgttatatggcttatactggtataagcaaaagtatggtgaaggtcttatcttcttgatgatgctacagaaaggtggggaagagaaaagtcatgaaaagataactgccaagttggatgagaaaaagcagcaaagttccctgcatatcacagcctcccagcccagccatgcaggcatctacctctgtggagca

SEQ ID NO: 190 - DNA, 270 bp, synthetic construct; identical to SEQ ID NO: 188
  source 1..270: mol_type = other DNA

SEQ ID NO: 191 - protein, 250 aa, synthetic construct
QKEVEQNSGPLSVPEGAIASLNCTYSDRVSQSFFWYRQYSGKSPELIMSIYSNGDKEDGRFTAQLNKASQYVSLLIRDSQPSDSATYLCAVDSSYKLIFGSGTRLLVRPDIQNPDPAVYQLRDSKSSDKSVCLFTDFDSQTNVSQSKDSDVYITDKTVLDMRSMDFKSNSAVAWSNKSDFACANAFNNSIIPEDTFFPSPESSCDVKLVEKSFETDTNLNFQNLSVIGFRILLLKVAGFNLLMTLRLWSS

SEQ ID NO: 192 - protein, 250 aa, synthetic construct
RKEVEQDPGPFNVPEGATVAFNCTYSNSASQSFFWYRQDCRKEPKLLMSVYSSGNEDGRFTAQLNRASQYISLLIRDSKLSDSATYLCVVTQAGTALIFGKGTTLSVSSNIQNPDPAVYQLRDSKSSDKSVCLFTDFDSQTNVSQSKDSDVYITDKTVLDMRSMDFKSNSAVAWSNKSDFACANAFNNSIIPEDTFFPSPESSCDVKLVEKSFETDTNLNFQNLSVIGFRILLLKVAGFNLLMTLRLWSS

SEQ ID NO: 193 - protein, 252 aa, synthetic construct
DAKTTQPNSMESNEEEPVHLPCNHSTISGTDYIHWYRQLPSQGPEYVIHGLTSNVNNRMASLAIAEDRKSSTLILHRATLRDAAVYYCILRAGGSGDKLTFGTGTRLAVRPNIQNPDPAVYQLRDSKSSDKSVCLFTDFDSQTNVSQSKDSDVYITDKTVLDMRSMDFKSNSAVAWSNKSDFACANAFNNSIIPEDTFFPSPESSCDVKLVEKSFETDTNLNFQNLSVIGFRILLLKVAGFNLLMTLRLWSS

SEQ ID NO: 194 - protein, 252 aa, synthetic construct
QKEVEQNSGPLSVPEGAIASLNCTYSDRGSQSFFWYRQYSGKSPELIMSIYSNGDKEDGRFTAQLNKASQYVSLLIRDSQPSDSATYLCAVLRSNDYKLSFGAGTTVTVRANIQNPDPAVYQLRDSKSSDKSVCLFTDFDSQTNVSQSKDSDVYITDKTVLDMRSMDFKSNSAVAWSNKSDFACANAFNNSIIPEDTFFPSPESSCDVKLVEKSFETDTNLNFQNLSVIGFRILLLKVAGFNLLMTLRLWSS

SEQ ID NO: 195 - protein, 254 aa, synthetic construct
AQSVTQLDSHVSVSEGTPVLLRCNYSSSYSPSLFWYVQHPNKGLQLLLKYTSAATLVKGINGFEAEFKKSETSFHLTKPSAHMSDAAEYFCVVSITGFQKLVFGTGTRLLVSPNIQNPDPAVYQLRDSKSSDKSVCLFTDFDSQTNVSQSKDSDVYITDKTVLDMRSMDFKSNSAVAWSNKSDFACANAFNNSIIPEDTFFPSPESSCDVKLVEKSFETDTNLNFQNLSVIGFRILLLKVAGFNLLMTLRLWSS

SEQ ID NO: 196 - protein, 255 aa, synthetic construct
GEDVEQSLFLSVREGDSSVINCTYTDSSSTYLYWYKQEPGAGLQLLTYIFSNMDMKQDQRLTVLLNKKDKHLSLRIADTQTGDSAIYFCAESVGYGGSQGNLIFGKGTKLSVKPNIQNPDPAVYQLRDSKSSDKSVCLFTDFDSQTNVSQSKDSDVYITDKTVLDMRSMDFKSNSAVAWSNKSDFACANAFNNSIIPEDTFFPSPESSCDVKLVEKSFETDTNLNFQNLSVIGFRILLLKVAGFNLLMTLRLWSS

SEQ ID NO: 197 - protein, 253 aa, synthetic construct
QKEVEQNSGPLSVPEGAIASLNCTYSDRGSQSFFWYRQYSGKSPELIMFIYSNGDKEDGRFTAQLNKASQYVSLLIRDSQPSDSATYLCAVPGGTSYGKLTFGQGTILTVHPNIQNPDPAVYQLRDSKSSDKSVCLFTDFDSQTNVSQSKDSDVYITDKTVLDMRSMDFKSNSAVAWSNKSDFACANAFNNSIIPEDTFFPSPESSCDVKLVEKSFETDTNLNFQNLSVIGFRILLLKVAGFNLLMTLRLWSS

SEQ ID NO: 198 - protein, 254 aa, synthetic construct
QQPVQSPQAVILREGEDAVINCSSSKALYSVHWYRQKHGEAPVFLMILLKGGEQKGHDKISASFNEKKQQSSLYLTASQLSYSGTYFCGTESGRGSTLGRLYFGRGTQLTVWPDIQNPDPAVYQLRDSKSSDKSVCLFTDFDSQTNVSQSKDSDVYITDKTVLDMRSMDFKSNSAVAWSNKSDFACANAFNNSIIPEDTFFPSPESSCDVKLVEKSFETDTNLNFQNLSVIGFRILLLKVAGFNLLMTLRLWSS

SEQ ID NO: 199 - protein, 252 aa, synthetic construct
SQQGEEDPQALSIQEGENATMNCSYKTSINNLQWYRQNSGRGLVHLILIRSNEREKHSGRLRVTLDTSKKSSSLLITASRAADTASYFCATLTLNDYKLSFGAGTTVTVRANIQNPDPAVYQLRDSKSSDKSVCLFTDFDSQTNVSQSKDSDVYITDKTVLDMRSMDFKSNSAVAWSNKSDFACANAFNNSIIPEDTFFPSPESSCDVKLVEKSFETDTNLNFQNLSVIGFRILLLKVAGFNLLMTLRLWSS

SEQ ID NO: 200 - protein, 252 aa, synthetic construct
GQQLNQSPQSMFIQEGEDVSMNCTSSSIFNTWLWYKQDPGEGPVLLIALYKAGELTSNGRLTAQFGITRKDSFLNISASIPSDVGIYFCAGQASGTYKYIFGTGTRLKVLANIQNPDPAVYQLRDSKSSDKSVCLFTDFDSQTNVSQSKDSDVYITDKTVLDMRSMDFKSNSAVAWSNKSDFACANAFNNSIIPEDTFFPSPESSCDVKLVEKSFETDTNLNFQNLSVIGFRILLLKVAGFNLLMTLRLWSS

SEQ ID NO: 201 - protein, 250 aa, synthetic construct
QKEVEQNSGPLSVPEGAIASLNCTYSDRGSQSFFWYRQYSGKSPELIMFIYSNGDKEDGRFTAQLNKASQYVSLLIRDSQPSDSATYLCAGHTGNQFYFGTGTSLTVIPNIQNPDPAVYQLRDSKSSDKSVCLFTDFDSQTNVSQSKDSDVYITDKTVLDMRSMDFKSNSAVAWSNKSDFACANAFNNSIIPEDTFFPSPESSCDVKLVEKSFETDTNLNFQNLSVIGFRILLLKVAGFNLLMTLRLWSS

SEQ ID NO: 202 - protein, 250 aa, synthetic construct
KNEVEQSPQNLTAQEGEFITINCSYSVGISALHWLQQHPGGGIVSLFMLSSGKKKHGRLIATINIQEKHSSLHITASHPRDSAVYICALNSDSNYQLIWGAGTKLIIKPDIQNPDPAVYQLRDSKSSDKSVCLFTDFDSQTNVSQSKDSDVYITDKTVLDMRSMDFKSNSAVAWSNKSDFACANAFNNSIIPEDTFFPSPESSCDVKLVEKSFETDTNLNFQNLSVIGFRILLLKVAGFNLLMTLRLWSS

SEQ ID NO: 203 - protein, 250 aa, synthetic construct
GQQLNQSPQSMFIQEGEDVSMNCTSSSIFNTWLWYKQDPGEGPVLLIALYKAGELTSNGRLTAQFGITRKDSFLNISASIPSDVGIYFCAGPEDDKIIFGKGTRLHILPNIQNPDPAVYQLRDSKSSDKSVCLFTDFDSQTNVSQSKDSDVYITDKTVLDMRSMDFKSNSAVAWSNKSDFACANAFNNSIIPEDTFFPSPESSCDVKLVEKSFETDTNLNFQNLSVIGFRILLLKVAGFNLLMTLRLWSS

SEQ ID NO: 204 - protein, 252 aa, synthetic construct
TQLLEQSPQFLSIQEGENLTVYCNSSSVFSSLQWYRQEPGEGPVLLVTVVTGGEVKKLKRLTFQFGDARKDSSLHITAAQPGDTGLYLCAGVDNYGQNFVFGPGTRLSVLPYIQNPDPAVYQLRDSKSSDKSVCLFTDFDSQTNVSQSKDSDVYITDKTVLDMRSMDFKSNSAVAWSNKSDFACANAFNNSIIPEDTFFPSPESSCDVKLVEKSFETDTNLNFQNLSVIGFRILLLKVAGFNLLMTLRLWSS

SEQ ID NO: 205 - protein, 251 aa, synthetic construct
QKEVEQNSGPLSVPEGAIASLNCTYSDRGSQSFFWYRQYSGKSPELIMFIYSNGDKEDGRFTAQLNKASQYVSLLIRDSQPSDSATYLCAVNTGFQKLVFGTGTRLLVSPNIQNPDPAVYQLRDSKSSDKSVCLFTDFDSQTNVSQSKDSDVYITDKTVLDMRSMDFKSNSAVAWSNKSDFACANAFNNSIIPEDTFFPSPESSCDVKLVEKSFETDTNLNFQNLSVIGFRILLLKVAGFNLLMTLRLWSS

SEQ ID NO: 206 - protein, 250 aa, synthetic construct
GIQVEQSPPDLILQEGANSTLRCNFSDSVNNLQWFHQNPWGQLINLFYIPSGTKQNGRLSATTVATERYSLLYISSSQTTDSGVYFCAVMPSGTYKYIFGTGTRLKVLANIQNPDPAVYQLRDSKSSDKSVCLFTDFDSQTNVSQSKDSDVYITDKTVLDMRSMDFKSNSAVAWSNKSDFACANAFNNSIIPEDTFFPSPESSCDVKLVEKSFETDTNLNFQNLSVIGFRILLLKVAGFNLLMTLRLWSS

SEQ ID NO: 207 - protein, 253 aa, synthetic construct
DQQVKQNSPSLSVQEGRISILNCDYTNSMFDYFLWYKKYPAEGPTFLISISSIKDKNEDGRFTVFLNKSAKHLSLHIVPSQPGDSAVYFCAASGVRGQNFVFGPGTRLSVLPYIQNPDPAVYQLRDSKSSDKSVCLFTDFDSQTNVSQSKDSDVYITDKTVLDMRSMDFKSNSAVAWSNKSDFACANAFNNSIIPEDTFFPSPESSCDVKLVEKSFETDTNLNFQNLSVIGFRILLLKVAGFNLLMTLRLWSS

SEQ ID NO: 208 - protein, 252 aa, synthetic construct
SQELEQSPQSLIVQEGKNLTINCTSSKTLYGLYWYKQKYGEGLIFLMMLQKGGEEKSHEKITAKLDEKKQQSSLHITASQPSHAGIYLCGADVINDYKLSFGAGTTVTVRANIQNPDPAVYQLRDSKSSDKSVCLFTDFDSQTNVSQSKDSDVYITDKTVLDMRSMDFKSNSAVAWSNKSDFACANAFNNSIIPEDTFFPSPESSCDVKLVEKSFETDTNLNFQNLSVIGFRILLLKVAGFNLLMTLRLWSS

SEQ ID NO: 209 - protein, 251 aa, synthetic construct
RKEVEQDPGPFNVPEGATVAFNCTYSNSASQSFFWYRQDCRKEPKLLMSVYSSGNEDGRFTAQLNRASQYISLLIRDSKLSDSATYLCVVNRGSQGNLIFGKGTKLSVKPNIQNPDPAVYQLRDSKSSDKSVCLFTDFDSQTNVSQSKDSDVYITDKTVLDMRSMDFKSNSAVAWSNKSDFACANAFNNSIIPEDTFFPSPESSCDVKLVEKSFETDTNLNFQNLSVIGFRILLLKVAGFNLLMTLRLWSS

SEQ ID NO: 210 - protein, 254 aa, synthetic construct
AQSVSQHNHHVILSEAASLELGCNYSYGGTVNLFWYVQYPGQHLQLLLKYFSGDPLVKGIKGFEAEFIKSKFSFNLRKPSVQWSDTAEYFCAVKMDSSYKLIFGSGTRLLVRPDIQNPDPAVYQLRDSKSSDKSVCLFTDFDSQTNVSQSKDSDVYITDKTVLDMRSMDFKSNSAVAWSNKSDFACANAFNNSIIPEDTFFPSPESSCDVKLVEKSFETDTNLNFQNLSVIGFRILLLKVAGFNLLMTLRLWSS

SEQ ID NO: 211 - protein, 249 aa, synthetic construct
GQSLEQPSEVTAVEGAIVQINCTYQTSGFYGLSWYQQHDGGAPTFLSYNALDGLEETGRFSSFLSRSDSYGYLLLQELQMKDSASYFCALGTEDKIIFGKGTRLHILPNIQNPDPAVYQLRDSKSSDKSVCLFTDFDSQTNVSQSKDSDVYITDKTVLDMRSMDFKSNSAVAWSNKSDFACANAFNNSIIPEDTFFPSPESSCDVKLVEKSFETDTNLNFQNLSVIGFRILLLKVAGFNLLMTLRLWSS

SEQ ID NO: 212 - protein, 246 aa, synthetic construct
AQTVTQSQPEMSVQEAETVTLSCTYDTSENNYYLFWYKQPPSRQMILVIRQEAYKQQNATENRFSVNFQKAAKSFSLKISDSQLGDTAMYFCAFDNNARLMFGDGTQLVVKPISRTLTLPCTSETLNPVTSLSAYSPILILKQMCHKVRILMCISQTKLCTGLWTSRATVLWPGATNLTLHVQTPSTTALFQKTPSSPAQKVPVMSSWSRKALKQIRTTFKTCQLGSESSSKWPGLICSRCGCGPA

SEQ ID NO: 213 - protein, 253 aa, synthetic construct
GQQLNQSPQSMFIQEGEDVSMNCTSSSIFNTWLWYKQDPGEGPVLLIALYKAGELTSNGRLTAQFGITRKDSFLNISASIPSDVGIYFCAGFSQGGSEKLVFGKGTKLTVNPYIQNPDPAVYQLRDSKSSDKSVCLFTDFDSQTNVSQSKDSDVYITDKTVLDMRSMDFKSNSAVAWSNKSDFACANAFNNSIIPEDTFFPSPESSCDVKLVEKSFETDTNLNFQNLSVIGFRILLLKVAGFNLLMTLRLWSS

SEQ ID NO: 214 - protein, 250 aa, synthetic construct
GIQVEQSPPDLILQEGANSTLRCNFSDSVNNLQWFHQNPWGQLINLFYIPSGTKQNGRLSATTVATERYSLLYISSSQTTDSGVYFCAVLAPGTYKYIFGTGTRLKVLANIQNPDPAVYQLRDSKSSDKSVCLFTDFDSQTNVSQSKDSDVYITDKTVLDMRSMDFKSNSAVAWSNKSDFACANAFNNSIIPEDTFFPSPESSCDVKLVEKSFETDTNLNFQNLSVIGFRILLLKVAGFNLLMTLRLWSS

SEQ ID NO: 215 - protein, 254 aa, synthetic construct
SQQGEEDPQALSIQEGENATMNCSYKTSINNLQWYRQNSGRGLVHLILIRSNEREKHSGRLRVTLDTSKKSSSLLITASRAADTASYFCATDLSGAGSYQLTFGKGTKLSVIPNIQNPDPAVYQLRDSKSSDKSVCLFTDFDSQTNVSQSKDSDVYITDKTVLDMRSMDFKSNSAVAWSNKSDFACANAFNNSIIPEDTFFPSPESSCDVKLVEKSFETDTNLNFQNLSVIGFRILLLKVAGFNLLMTLRLWSS

SEQ ID NO: 216 - protein, 252 aa, synthetic construct
QKEVEQNSGPLSVPEGAIASLNCTYSDRVSQSFFWYRQYSGKSPELIMSIYSNGDKEDGRFTAQLNKASQYVSLLIRDSQPSDSATYLCAVVSSNDYKLSFGAGTTVTVRANIQNPDPAVYQLRDSKSSDKSVCLFTDFDSQTNVSQSKDSDVYITDKTVLDMRSMDFKSNSAVAWSNKSDFACANAFNNSIIPEDTFFPSPESSCDVKLVEKSFETDTNLNFQNLSVIGFRILLLKVAGFNLLMTLRLWSS

SEQ ID NO: 217 - protein, 252 aa, synthetic construct
QKEVEQNSGPLSVPEGAIASLNCTYSDRVSQSFFWYRQYSGKSPELIMSIYSNGDKEDGRFTAQLNKASQYVSLLIRDSQPSDSATYLCAVASGGSYIPTFGRGTSLIVHPYIQNPDPAVYQLRDSKSSDKSVCLFTDFDSQTNVSQSKDSDVYITDKTVLDMRSMDFKSNSAVAWSNKSDFACANAFNNSIIPEDTFFPSPESSCDVKLVEKSFETDTNLNFQNLSVIGFRILLLKVAGFNLLMTLRLWSS

SEQ ID NO: 218 - protein, 251 aa, synthetic construct
GESVGLHLPTLSVQEGDNSIINCAYSNSASDYFIWYKQESGKGPQFIIDIRSNMDKRQGQRVTVLLNKTVKHLSLQIAATQPGDSAVYFCAESYGQKLLFARGTMLKVDLNIQNPDPAVYQLRDSKSSDKSVCLFTDFDSQTNVSQSKDSDVYITDKTVLDMRSMDFKSNSAVAWSNKSDFACANAFNNSIIPEDTFFPSPESSCDVKLVEKSFETDTNLNFQNLSVIGFRILLLKVAGFNLLMTLRLWSS

SEQ ID NO: 219 - protein, 254 aa, synthetic construct
GQQLNQSPQSMFIQEGEDVSMNCTSSSIFNTWLWYKQDPGEGPVLLIALYKAGELTSNGRLTAQFGITRKDSFLNISASIPSDVGIYFCAGQDDGGSQGNLIFGKGTKLSVKPNIQNPDPAVYQLRDSKSSDKSVCLFTDFDSQTNVSQSKDSDVYITDKTVLDMRSMDFKSNSAVAWSNKSDFACANAFNNSIIPEDTFFPSPESSCDVKLVEKSFETDTNLNFQNLSVIGFRILLLKVAGFNLLMTLRLWSS

SEQ ID NO: 220 - protein, 251 aa, synthetic construct
QQPVQSPQAVILREGEDAVINCSSSKALYSVHWYRQKHGEAPVFLMILLKGGEQKGHDKISASFNEKKQQSSLYLTASQLSYSGTYFCGTEFRNDYKLSFGAGTTVTVRANIQNPDPAVYQLRDSKSSDKSVCLFTDFDSQTNVSQSKDSDVYITDKTVLDMRSMDFKSNSAVAWSNKSDFACANAFNNSIIPEDTFFPSPESSCDVKLVEKSFETDTNLNFQNLSVIGFRILLLKVAGFNLLMTLRLWSS

SEQ ID NO: 221 - protein, 252 aa, synthetic construct
SQQGEEDPQALSIQEGENATMNCSYKTSINNLQWYRQNSGRGLVHLILIRSNEREKHSGRLRVTLDTSKKSSSLLITASRAADTASYFCATDVKSSYKLIFGSGTRLLVRPDIQNPDPAVYQLRDSKSSDKSVCLFTDFDSQTNVSQSKDSDVYITDKTVLDMRSMDFKSNSAVAWSNKSDFACANAFNNSIIPEDTFFPSPESSCDVKLVEKSFETDTNLNFQNLSVIGFRILLLKVAGFNLLMTLRLWSS

SEQ ID NO: 222 - protein, 254 aa, synthetic construct
DQQVKQNSPSLSVQEGRISILNCDYTNSMFDYFLWYKKYPAEGPTFLISISSIKDKNEDGRFTVFLNKSAKHLSLHIVPSQPGDSAVYFCAAFASDSNYQLIWGAGTKLIIKPDIQNPDPAVYQLRDSKSSDKSVCLFTDFDSQTNVSQSKDSDVYITDKTVLDMRSMDFKSNSAVAWSNKSDFACANAFNNSIIPEDTFFPSPESSCDVKLVEKSFETDTNLNFQNLSVIGFRILLLKVAGFNLLMTLRLWSS

SEQ ID NO: 223 - protein, 251 aa, synthetic construct
QKEVEQNSGPLSVPEGAIASLNCTYSDRVSQSFFWYRQYSGKSPELIMSIYSNGDKEDGRFTAQLNKASQYVSLLIRDSQPSDSATYLCALVSGTYKYIFGTGTRLKVLANIQNPDPAVYQLRDSKSSDKSVCLFTDFDSQTNVSQSKDSDVYITDKTVLDMRSMDFKSNSAVAWSNKSDFACANAFNNSIIPEDTFFPSPESSCDVKLVEKSFETDTNLNFQNLSVIGFRILLLKVAGFNLLMTLRLWSS

SEQ ID NO: 224 - protein, 251 aa, synthetic construct
SQQGEEDPQALSIQEGENATMNCSYKTSINNLQWYRQNSGRGLVHLILIRSNEREKHSGRLRVTLDTSKKSSSLLITASRAADTASYFCATYANDYKLSFGAGTTVTVRANIQNPDPAVYQLRDSKSSDKSVCLFTDFDSQTNVSQSKDSDVYITDKTVLDMRSMDFKSNSAVAWSNKSDFACANAFNNSIIPEDTFFPSPESSCDVKLVEKSFETDTNLNFQNLSVIGFRILLLKVAGFNLLMTLRLWSS

SEQ ID NO: 225 - protein, 250 aa, synthetic construct
DQQVKQNSPSLSVQEGRISILNCDYTNSMFDYFLWYKKYPAEGPTFLISISSIKDKNEDGRFTVFLNKSAKHLSLHIVPSQPGDSAVYFCAAKPDKLIFGTGTRLQVFPNIQNPDPAVYQLRDSKSSDKSVCLFTDFDSQTNVSQSKDSDVYITDKTVLDMRSMDFKSNSAVAWSNKSDFACANAFNNSIIPEDTFFPSPESSCDVKLVEKSFETDTNLNFQNLSVIGFRILLLKVAGFNLLMTLRLWSS

SEQ ID NO: 226 - protein, 250 aa, synthetic construct
QKEVEQNSGPLSVPEGAIASLNCTYSDRGSQSFFWYRQYSGKSPELIMSIYSNGDKEDGRFTAQLNKASQYVSLLIRDSQPSDSATYLCAVPSGNMLTFGGGTRLMVKPHIQNPDPAVYQLRDSKSSDKSVCLFTDFDSQTNVSQSKDSDVYITDKTVLDMRSMDFKSNSAVAWSNKSDFACANAFNNSIIPEDTFFPSPESSCDVKLVEKSFETDTNLNFQNLSVIGFRILLLKVAGFNLLMTLRLWSS

SEQ ID NO: 227 - protein, 252 aa, synthetic construct
SQELEQSPQSLIVQEGKNLTINCTSSKTLYGLYWYKQKYGEGLIFLMMLQKGGEEKSHEKITAKLDEKKQQSSLHITASQPSHAGIYLCGAVPINDYKLSFGAGTTVTVRANIQNPDPAVYQLRDSKSSDKSVCLFTDFDSQTNVSQSKDSDVYITDKTVLDMRSMDFKSNSAVAWSNKSDFACANAFNNSIIPEDTFFPSPESSCDVKLVEKSFETDTNLNFQNLSVIGFRILLLKVAGFNLLMTLRLWSS

SEQ ID NO: 228 - protein, 252 aa, synthetic construct
QKEVEQNSGPLSVPEGAIASLNCTYSDRGSQSFFWYRQYSGKSPELIMSIYSNGDKEDGRFTAQLNKASQYVSLLIRDSQPSDSATYLCAVVSGGYNKLIFGAGTRLAVHPYIQNPDPAVYQLRDSKSSDKSVCLFTDFDSQTNVSQSKDSDVYITDKTVLDMRSMDFKSNSAVAWSNKSDFACANAFNNSIIPEDTFFPSPESSCDVKLVEKSFETDTNLNFQNLSVIGFRILLLKVAGFNLLMTLRLWSS

SEQ ID NO: 229 - DNA, 750 bp, synthetic construct
  source 1..750: mol_type = other DNA
cagaaggaggtggagcagaattctggacccctcagtgttccagagggagccattgcctctctcaactgcacttacagtgaccgagtttcccagtccttcttctggtacagacaatattctgggaaaagccctgagttgataatgtccatatactccaatggtgacaaagaagatggaaggtttacagcacagctcaataaagccagccagtatgtttctctgctcatcagagactcccagcccagtgattcagccacctacctctgtgccgtggatagcagctataaattgatcttcgggagtgggaccagactgctggtcaggcctgatatccagaaccctgaccctgccgtgtaccagctgagagactctaaatccagtgacaagtctgtctgcctattcaccgattttgattctcaaacaaatgtgtcacaaagtaaggattctgatgtgtatatcacagacaaaactgtgctagacatgaggtctatggacttcaagagcaacagtgctgtggcctggagcaacaaatctgactttgcatgtgcaaacgccttcaacaacagcattattccagaagacaccttcttccccagcccagaaagttcctgtgatgtcaagctggtcgagaaaagctttgaaacagatacgaacctaaactttcaaaacctgtcagtgattgggttccgaatcctcctcctgaaagtggccgggtttaatctgctcatgacgctgcggctgtggtccagc

SEQ ID NO: 230 - DNA, 750 bp, synthetic construct
  source 1..750: mol_type = other DNA
cggaaggaggtggagcaggatcctggacccttcaatgttccagagggagccactgtcgctttcaactgtacttacagcaacagtgcttctcagtctttcttctggtacagacaggattgcaggaaagaacctaagttgctgatgtccgtatactccagtggtaatgaagatggaaggtttacagcacagctcaatagagccagccagtatatttccctgctcatcagagactccaagctcagtgattcagccacctacctctgtgtggtgacccaagcaggaactgctctgatctttgggaagggaaccaccttatcagtgagttccaatatccagaaccctgaccctgccgtgtaccagctgagagactctaaatccagtgacaagtctgtctgcctattcaccgattttgattctcaaacaaatgtgtcacaaagtaaggattctgatgtgtatatcacagacaaaactgtgctagacatgaggtctatggacttcaagagcaacagtgctgtggcctggagcaacaaatctgactttgcatgtgcaaacgccttcaacaacagcattattccagaagacaccttcttccccagcccagaaagttcctgtgatgtcaagctggtcgagaaaagctttgaaacagatacgaacctaaactttcaaaacctgtcagtgattgggttccgaatcctcctcctgaaagtggccgggtttaatctgctcatgacgctgcggctgtggtccagc

SEQ ID NO: 231 - DNA, 756 bp, synthetic construct
  source 1..756: mol_type = other DNA
gatgctaagaccacacagccaaattcaatggagagtaacgaagaagagcctgttcacttgccttgtaaccactccacaatcagtggaactgattacatacattggtatcgacagcttccctcccagggtccagagtacgtgattcatggtcttacaagcaatgtgaacaacagaatggcctctctggcaatcgctgaagacagaaagtccagtaccttgatcctgcaccgtgctaccttgagagatgctgctgtgtactactgcatcctgagggccgggggcagcggagacaagctgacttttgggaccgggactcgtttagcagttaggcccaatatccagaaccctgaccctgccgtgtaccagctgagagactctaaatccagtgacaagtctgtctgcctattcaccgattttgattctcaaacaaatgtgtcacaaagtaaggattctgatgtgtatatcacagacaaaactgtgctagacatgaggtctatggacttcaagagcaacagtgctgtggcctggagcaacaaatctgactttgcatgtgcaaacgccttcaacaacagcattattccagaagacaccttcttccccagcccagaaagttcctgtgatgtcaagctggtcgagaaaagctttgaaacagatacgaacctaaactttcaaaacctgtcagtgattgggttccgaatcctcctcctgaaagtggccgggtttaatctgctcatgacgctgcggctgtggtccagc

SEQ ID NO: 232 - DNA, 756 bp, synthetic construct
  source 1..756: mol_type = other DNA
cagaaggaggtggagcagaattctggacccctcagtgttccagagggagccattgcctctctcaactgcacttacagtgaccgaggttcccagtccttcttctggtacagacaatattctgggaaaagccctgagttgataatgtccatatactccaatggtgacaaagaagatggaaggtttacagcacagctcaataaagccagccagtatgtttctctgctcatcagagactcccagcccagtgattcagccacctacctctgtgccgtgctacgttctaacgactacaagctcagctttggagccggaaccacagtaactgtaagagcaaatatccagaaccctgaccctgccgtgtaccagctgagagactctaaatccagtgacaagtctgtctgcctattcaccgattttgattctcaaacaaatgtgtcacaaagtaaggattctgatgtgtatatcacagacaaaactgtgctagacatgaggtctatggacttcaagagcaacagtgctgtggcctggagcaacaaatctgactttgcatgtgcaaacgccttcaacaacagcattattccagaagacaccttcttccccagcccagaaagttcctgtgatgtcaagctggtcgagaaaagctttgaaacagatacgaacctaaactttcaaaacctgtcagtgattgggttccgaatcctcctcctgaaagtggccgggtttaatctgctcatgacgctgcggctgtggtccagc

SEQ ID NO: 233 - DNA, 762 bp, synthetic construct
  source 1..762: mol_type = other DNA
gcccagtcggtgacccagcttgacagccacgtctctgtctctgaaggaaccccggtgctgctgaggtgcaactactcatcttcttattcaccatctctcttctggtatgtgcaacaccccaacaaaggactccagcttctcctgaagtacacatcagcggccaccctggttaaaggcatcaacggttttgaggctgaatttaagaagagtgaaacctccttccacctgacgaaaccctcagcccatatgagcgacgcggctgagtacttctgtgttgtgagcatcacaggctttcagaaacttgtatttggaactggcacccgacttctggtcagtccaaatatccagaaccctgaccctgccgtgtaccagctgagagactctaaatccagtgacaagtctgtctgcctattcaccgattttgattctcaaacaaatgtgtcacaaagtaaggattctgatgtgtatatcacagacaaaactgtgctagacatgaggtctatggacttcaagagcaacagtgctgtggcctggagcaacaaatctgactttgcatgtgcaaacgccttcaacaacagcattattccagaagacaccttcttccccagcccagaaagttcctgtgatgtcaagctggtcgagaaaagctttgaaacagatacgaacctaaactttcaaaacctgtcagtgattgggttccgaatcctcctcctgaaagtggccgggtttaatctgctcatgacgctgcggctgtggtccagc

SEQ ID NO: 234 - DNA, 765 bp, synthetic construct
  source 1..765: mol_type = other DNA
ggagaggatgtggagcagagtcttttcctgagtgtccgagagggagacagctccgttataaactgcacttacacagacagctcctccacctacttatactggtataagcaagaacctggagcaggtctccagttgctgacgtatattttttcaaatatggacatgaaacaagaccaaagactcactgttctattgaataaaaaggataaacatctgtctctgcgcattgcagacacccagactggggactcagctatctacttctgtgcagagagcgtggggtatggaggaagccaaggaaatctcatctttggaaaaggcactaaactctctgttaaaccaaatatccagaaccctgaccctgccgtgtaccagctgagagactctaaatccagtgacaagtctgtctgcctattcaccgattttgattctcaaacaaatgtgtcacaaagtaaggattctgatgtgtatatcacagacaaaactgtgctagacatgaggtctatggacttcaagagcaacagtgctgtggcctggagcaacaaatctgactttgcatgtgcaaacgccttcaacaacagcattattccagaagacaccttcttccccagcccagaaagttcctgtgatgtcaagctggtcgagaaaagctttgaaacagatacgaacctaaactttcaaaacctgtcagtgattgggttccgaatcctcctcctgaaagtggccgggtttaatctgctcatgacgctgcggctgtggtccagc

SEQ ID NO: 235 - DNA, 759 bp, synthetic construct
  source 1..759: mol_type = other DNA
cagaaggaggtggagcagaattctggacccctcagtgttccagagggagccattgcctctctcaactgcacttacagtgaccgaggttcccagtccttcttctggtacagacaatattctgggaaaagccctgagttgataatgttcatatactccaatggtgacaaagaagatggaaggtttacagcacagctcaataaagccagccagtatgtttctctgctcatcagagactcccagcccagtgattcagccacctacctctgtgccgtgcctggtggtactagctatggaaagctgacatttggacaagggaccatcttgactgtccatccaaatatccagaaccctgaccctgccgtgtaccagctgagagactctaaatccagtgacaagtctgtctgcctattcaccgattttgattctcaaacaaatgtgtcacaaagtaaggattctgatgtgtatatcacagacaaaactgtgctagacatgaggtctatggacttcaagagcaacagtgctgtggcctggagcaacaaatctgactttgcatgtgcaaacgccttcaacaacagcattattccagaagacaccttcttccccagcccagaaagttcctgtgatgtcaagctggtcgagaaaagctttgaaacagatacgaacctaaactttcaaaacctgtcagtgattgggttccgaatcctcctcctgaaagtggccgggtttaatctgctcatgacgctgcggctgtggtccagc

SEQ ID NO: 236 - DNA, 762 bp, synthetic construct
  source 1..762: mol_type = other DNA
caacaaccagtgcagagtcctcaagccgtgatcctccgagaaggggaagatgctgtcatcaactgcagttcctccaaggctttatattctgtacactggtacaggcagaagcatggtgaagcacccgtcttcctgatgatattactgaagggtggagaacagaagggtcatgacaaaatatctgcttcatttaatgaaaaaaagcagcaaagctccctgtaccttacggcctcccagctcagttactcaggaacctacttctgtggcacagagagcgggagaggctcaaccctggggaggctatactttggaagaggaactcagttgactgtctggcctgatatccagaaccctgaccctgccgtgtaccagctgagagactctaaatccagtgacaagtctgtctgcctattcaccgattttgattctcaaacaaatgtgtcacaaagtaaggattctgatgtgtatatcacagacaaaactgtgctagacatgaggtctatggacttcaagagcaacagtgctgtggcctggagcaacaaatctgactttgcatgtgcaaacgccttcaacaacagcattattccagaagacaccttcttccccagcccagaaagttcctgtgatgtcaagctggtcgagaaaagctttgaaacagatacgaacctaaactttcaaaacctgtcagtgattgggttccgaatcctcctcctgaaagtggccgggtttaatctgctcatgacgctgcggctgtggtccagc

SEQ ID NO: 237 - DNA, 756 bp, synthetic construct
  source 1..756: mol_type = other DNA
agtcaacagggagaagaggatcctcaggccttgagcatccaggagggtgaaaatgccaccatgaactgcagttacaaaactagtataaacaatttacagtggtatagacaaaattcaggtagaggccttgtccacctaattttaatacgttcaaatgaaagagagaaacacagtggaagattaagagtcacgcttgacacttccaagaaaagcagttccttgttgatcacggcttcccgggcagcagacactgcttcttacttctgtgctacgttgacccttaacgactacaagctcagctttggagccggaaccacagtaactgtaagagcaaatatccagaaccctgaccctgccgtgtaccagctgagagactctaaatccagtgacaagtctgtctgcctattcaccgattttgattctcaaacaaatgtgtcacaaagtaaggattctgatgtgtatatcacagacaaaactgtgctagacatgaggtctatggacttcaagagcaacagtgctgtggcctggagcaacaaatctgactttgcatgtgcaaacgccttcaacaacagcattattccagaagacaccttcttccccagcccagaaagttcctgtgatgtcaagctggtcgagaaaagctttgaaacagatacgaacctaaactttcaaaacctgtcagtgattgggttccgaatcctcctcctgaaagtggccgggtttaatctgctcatgacgctgcggctgtggtccagc

SEQ ID NO: 238 - DNA, 756 bp, synthetic construct
  source 1..756: mol_type = other DNA
ggtcaacagctgaatcagagtcctcaatctatgtttatccaggaaggagaagatgtctccatgaactgcacttcttcaagcatatttaacacctggctatggtacaagcaggaccctggggaaggtcctgtcctcttgatagccttatataaggctggtgaattgacctcaaatggaagactgactgctcagtttggtataaccagaaaggacagcttcctgaatatctcagcatccatacctagtgatgtaggcatctacttctgtgctggccaggcctcaggaacctacaaatacatctttggaacaggcaccaggctgaaggttttagcaaatatccagaaccctgaccctgccgtgtaccagctgagagactctaaatccagtgacaagtctgtctgcctattcaccgattttgattctcaaacaaatgtgtcacaaagtaaggattctgatgtgtatatcacagacaaaactgtgctagacatgaggtctatggacttcaagagcaacagtgctgtggcctggagcaacaaatctgactttgcatgtgcaaacgccttcaacaacagcattattccagaagacaccttcttccccagcccagaaagttcctgtgatgtcaagctggtcgagaaaagctttgaaacagatacgaacctaaactttcaaaacctgtcagtgattgggttccgaatcctcctcctgaaagtggccgggtttaatctgctcatgacgctgcggctgtggtccagc

SEQ ID NO: 239 - DNA, 750 bp, synthetic construct
  source 1..750: mol_type = other DNA
cagaaggaggtggagcagaattctggacccctcagtgttccagagggagccattgcctctctcaactgcacttacagtgaccgaggttcccagtccttcttctggtacagacaatattctgggaaaagccctgagttgataatgttcatatactccaatggtgacaaagaagatggaaggtttacagcacagctcaataaagccagccagtatgtttctctgctcatcagagactcccagcccagtgattcagccacctacctctgtgccggtcacaccggtaaccagttctattttgggacagggacaagtttgacggtcattccaaatatccagaaccctgaccctgccgtgtaccagctgagagactctaaatccagtgacaagtctgtctgcctattcaccgattttgattctcaaacaaatgtgtcacaaagtaaggattctgatgtgtatatcacagacaaaactgtgctagacatgaggtctatggacttcaagagcaacagtgctgtggcctggagcaacaaatctgactttgcatgtgcaaacgccttcaacaacagcattattccagaagacaccttcttccccagcccagaaagttcctgtgatgtcaagctggtcgagaaaagctttgaaacagatacgaacctaaactttcaaaacctgtcagtgattgggttccgaatcctcctcctgaaagtggccgggtttaatctgctcatgacgctgcggctgtggtccagc

SEQ ID NO: 240 - DNA, 750 bp, synthetic construct
  source 1..750: mol_type = other DNA
aaaaatgaagtggagcagagtcctcagaacctgactgcccaggaaggagaatttatcacaatcaactgcagttactcggtaggaataagtgccttacactggctgcaacagcatccaggaggaggcattgtttccttgtttatgctgagctcagggaagaagaagcatggaagattaattgccacaataaacatacaggaaaagcacagctccctgcacatcacagcctcccatcccagagactctgccgtctacatctgtgctttaaattcggatagcaactatcagttaatctggggcgctgggaccaagctaattataaagccagatatccagaaccctgaccctgccgtgtaccagctgagagactctaaatccagtgacaagtctgtctgcctattcaccgattttgattctcaaacaaatgtgtcacaaagtaaggattctgatgtgtatatcacagacaaaactgtgctagacatgaggtctatggacttcaagagcaacagtgctgtggcctggagcaacaaatctgactttgcatgtgcaaacgccttcaacaacagcattattccagaagacaccttcttccccagcccagaaagttcctgtgatgtcaagctggtcgagaaaagctttgaaacagatacgaacctaaactttcaaaacctgtcagtgattgggttccgaatcctcctcctgaaagtggccgggtttaatctgctcatgacgctgcggctgtggtccagc

SEQ ID NO: 241 - DNA, 750 bp, synthetic construct
  source 1..750: mol_type = other DNA
ggtcaacagctgaatcagagtcctcaatctatgtttatccaggaaggagaagatgtctccatgaactgcacttcttcaagcatatttaacacctggctatggtacaagcaggaccctggggaaggtcctgtcctcttgatagccttatataaggctggtgaattgacctcaaatggaagactgactgctcagtttggtataaccagaaaggacagcttcctgaatatctcagcatccatacctagtgatgtaggcatctacttctgtgctggtccggaagatgacaagatcatctttggaaaagggacacgacttcatattctccccaatatccagaaccctgaccctgccgtgtaccagctgagagactctaaatccagtgacaagtctgtctgcctattcaccgattttgattctcaaacaaatgtgtcacaaagtaaggattctgatgtgtatatcacagacaaaactgtgctagacatgaggtctatggacttcaagagcaacagtgctgtggcctggagcaacaaatctgactttgcatgtgcaaacgccttcaacaacagcattattccagaagacaccttcttccccagcccagaaagttcctgtgatgtcaagctggtcgagaaaagctttgaaacagatacgaacctaaactttcaaaacctgtcagtgattgggttccgaatcctcctcctgaaagtggccgggtttaatctgctcatgacgctgcggctgtggtccagc

SEQ ID NO: 242 - DNA, 756 bp, synthetic construct
  source 1..756: mol_type = other DNA
acccagctgctggagcagagccctcagtttctaagcatccaagagggagaaaatctcactgtgtactgcaactcctcaagtgttttttccagcttacaatggtacagacaggagcctggggaaggtcctgtcctcctggtgacagtagttacgggtggagaagtgaagaagctgaagagactaacctttcagtttggtgatgcaagaaaggacagttctctccacatcactgcggcccagcctggtgatacaggcctctacctctgtgcaggagttgataactatggtcagaattttgtctttggtcccggaaccagattgtccgtgctgccctatatccagaaccctgaccctgccgtgtaccagctgagagactctaaatccagtgacaagtctgtctgcctattcaccgattttgattctcaaacaaatgtgtcacaaagtaaggattctgatgtgtatatcacagacaaaactgtgctagacatgaggtctatggacttcaagagcaacagtgctgtggcctggagcaacaaatctgactttgcatgtgcaaacgccttcaacaacagcattattccagaagacaccttcttccccagcccagaaagttcctgtgatgtcaagctggtcgagaaaagctttgaaacagatacgaacctaaactttcaaaacctgtcagtgattgggttccgaatcctcctcctgaaagtggccgggtttaatctgctcatgacgctgcggctgtggtccagc

SEQ ID NO: 243 - DNA, 753 bp, synthetic construct
  source 1..753: mol_type = other DNA
cagaaggaggtggagcagaattctggacccctcagtgttccagagggagccattgcctctctcaactgcacttacagtgaccgaggttcccagtccttcttctggtacagacaatattctgggaaaagccctgagttgataatgttcatatactccaatggtgacaaagaagatggaaggtttacagcacagctcaataaagccagccagtatgtttctctgctcatcagagactcccagcccagtgattcagccacctacctctgtgccgtgaacacaggctttcagaaacttgtatttggaactggcacccgacttctggtcagtccaaatatccagaaccctgaccctgccgtgtaccagctgagagactctaaatccagtgacaagtctgtctgcctattcaccgattttgattctcaaacaaatgtgtcacaaagtaaggattctgatgtgtatatcacagacaaaactgtgctagacatgaggtctatggacttcaagagcaacagtgctgtggcctggagcaacaaatctgactttgcatgtgcaaacgccttcaacaacagcattattccagaagacaccttcttccccagcccagaaagttcctgtgatgtcaagctggtcgagaaaagctttgaaacagatacgaacctaaactttcaaaacctgtcagtgattgggttccgaatcctcctcctgaaagtggccgggtttaatctgctcatgacgctgcggctgtggtccagc

SEQ ID NO: 244 - DNA, 750 bp, synthetic construct
  source 1..750: mol_type = other DNA
ggaatacaagtggagcagagtcctccagacctgattctccaggagggagccaattccacgctgcggtgcaatttttctgactctgtgaacaatttgcagtggtttcatcaaaacccttggggacagctcatcaacctgttttacattccctcagggacaaaacagaatggaagattaagcgccacgactgtcgctacggaacgctacagcttattgtacatttcctcttcccagaccacagactcaggcgtttatttctgtgctgtgatgccctcaggaacctacaaatacatctttggaacaggcaccaggctgaaggttttagcaaatatccagaaccctgaccctgccgtgtaccagctgagagactctaaatccagtgacaagtctgtctgcctattcaccgattttgattctcaaacaaatgtgtcacaaagtaaggattctgatgtgtatatcacagacaaaactgtgctagacatgaggtctatggacttcaagagcaacagtgctgtggcctggagcaacaaatctgactttgcatgtgcaaacgccttcaacaacagcattattccagaagacaccttcttccccagcccagaaagttcctgtgatgtcaagctggtcgagaaaagctttgaaacagatacgaacctaaactttcaaaacctgtcagtgattgggttccgaatcctcctcctgaaagtggccgggtttaatctgctcatgacgctgcggctgtggtccagc

SEQ ID NO: 245 - DNA, 759 bp, synthetic construct
  source 1..759: mol_type = other DNA
gaccagcaagttaagcaaaattcaccatccctgagcgtccaggaaggaagaatttctattctgaactgtgactatactaacagcatgtttgattatttcctatggtacaaaaaataccctgctgaaggtcctacattcctgatatctataagttccattaaggataaaaatgaagatggaagattcactgttttcttaaacaaaagtgccaagcacctctctctgcacattgtgccctcccagcctggagactctgcagtgtacttctgtgcagcaagtggagtgcgtggtcagaattttgtctttggtcccggaaccagattgtccgtgctgccctatatccagaaccctgaccctgccgtgtaccagctgagagactctaaatccagtgacaagtctgtctgcctattcaccgattttgattctcaaacaaatgtgtcacaaagtaaggattctgatgtgtatatcacagacaaaactgtgctagacatgaggtctatggacttcaagagcaacagtgctgtggcctggagcaacaaatctgactttgcatgtgcaaacgccttcaacaacagcattattccagaagacaccttcttccccagcccagaaagttcctgtgatgtcaagctggtcgagaaaagctttgaaacagatacgaacctaaactttcaaaacctgtcagtgattgggttccgaatcctcctcctgaaagtggccgggtttaatctgctcatgacgctgcggctgtggtccagc

SEQ ID NO: 246 - DNA, 756 bp, synthetic construct
  source 1..756: mol_type = other DNA
agccaagaactggagcagagtcctcagtccttgatcgtccaagagggaaagaatctcaccataaactgcacgtcatcaaagacgttatatggcttatactggtataagcaaaagtatggtgaaggtcttatcttcttgatgatgctacagaaaggtggggaagagaaaagtcatgaaaagataactgccaagttggatgagaaaaagcagcaaagttccctgcatatcacagcctcccagcccagccatgcaggcatctacctctgtggagcagacgtaattaacgactacaagctcagctttggagccggaaccacagtaactgtaagagcaaatatccagaaccctgaccctgccgtgtaccagctgagagactctaaatccagtgacaagtctgtctgcctattcaccgattttgattctcaaacaaatgtgtcacaaagtaaggattctgatgtgtatatcacagacaaaactgtgctagacatgaggtctatggacttcaagagcaacagtgctgtggcctggagcaacaaatctgactttgcatgtgcaaacgccttcaacaacagcattattccagaagacaccttcttccccagcccagaaagttcctgtgatgtcaagctggtcgagaaaagctttgaaacagatacgaacctaaactttcaaaacctgtcagtgattgggttccgaatcctcctcctgaaagtggccgggtttaatctgctcatgacgctgcggctgtggtccagc

SEQ ID NO: 247 - DNA, 753 bp, synthetic construct
  source 1..753: mol_type = other DNA
cggaaggaggtggagcaggatcctggacccttcaatgttccagagggagccactgtcgctttcaactgtacttacagcaacagtgcttctcagtctttcttctggtacagacaggattgcaggaaagaacctaagttgctgatgtccgtatactccagtggtaatgaagatggaaggtttacagcacagctcaatagagccagccagtatatttccctgctcatcagagactccaagctcagtgattcagccacctacctctgtgtggtgaaccggggaagccaaggaaatctcatctttggaaaaggcactaaactctctgttaaaccaaatatccagaaccctgaccctgccgtgtaccagctgagagactctaaatccagtgacaagtctgtctgcctattcaccgattttgattctcaaacaaatgtgtcacaaagtaaggattctgatgtgtatatcacagacaaaactgtgctagacatgaggtctatggacttcaagagcaacagtgctgtggcctggagcaacaaatctgactttgcatgtgcaaacgccttcaacaacagcattattccagaagacaccttcttccccagcccagaaagttcctgtgatgtcaagctggtcgagaaaagctttgaaacagatacgaacctaaactttcaaaacctgtcagtgattgggttccgaatcctcctcctgaaagtggccgggtttaatctgctcatgacgctgcggctgtggtccagc

SEQ ID NO: 248 - DNA, 762 bp, synthetic construct
  source 1..762: mol_type = other DNA
gcccagtctgtgagccagcataaccaccacgtaattctctctgaagcagcctcactggagttgggatgcaactattcctatggtggaactgttaatctcttctggtatgtccagtaccctggtcaacaccttcagcttctcctcaagtacttttcaggggatccactggttaaaggcatcaagggctttgaggctgaatttataaagagtaaattctcctttaatctgaggaaaccctctgtgcagtggagtgacacagctgagtacttctgtgccgtgaagatggatagcagctataaattgatcttcgggagtgggaccagactgctggtcaggcctgatatccagaaccctgaccctgccgtgtaccagctgagagactctaaatccagtgacaagtctgtctgcctattcaccgattttgattctcaaacaaatgtgtcacaaagtaaggattctgatgtgtatatcacagacaaaactgtgctagacatgaggtctatggacttcaagagcaacagtgctgtggcctggagcaacaaatctgactttgcatgtgcaaacgccttcaacaacagcattattccagaagacaccttcttccccagcccagaaagttcctgtgatgtcaagctggtcgagaaaagctttgaaacagatacgaacctaaactttcaaaacctgtcagtgattgggttccgaatcctcctcctgaaagtggccgggtttaatctgctcatgacgctgcggctgtggtccagc

SEQ ID NO: 249 - DNA, 747 bp, synthetic construct
  source 1..747: mol_type = other DNA
ggacaaagccttgagcagccctctgaagtgacagctgtggaaggagccattgtccagataaactgcacgtaccagacatctgggttttatgggctgtcctggtaccagcaacatgatggcggagcacccacatttctttcttacaatgctctggatggtttggaggagacaggtcgtttttcttcattccttagtcgctctgatagttatggttacctccttctacaggagctccagatgaaagactctgcctcttacttctgcgctttaggaaccgaggacaagatcatctttggaaaagggacacgacttcatattctccccaatatccagaaccctgaccctgccgtgtaccagctgagagactctaaatccagtgacaagtctgtctgcctattcaccgattttgattctcaaacaaatgtgtcacaaagtaaggattctgatgtgtatatcacagacaaaactgtgctagacatgaggtctatggacttcaagagcaacagtgctgtggcctggagcaacaaatctgactttgcatgtgcaaacgccttcaacaacagcattattccagaagacaccttcttccccagcccagaaagttcctgtgatgtcaagctggtcgagaaaagctttgaaacagatacgaacctaaactttcaaaacctgtcagtgattgggttccgaatcctcctcctgaaagtggccgggtttaatctgctcatgacgctgcggctgtggtccagc

SEQ ID NO: 250 - DNA, 758 bp, synthetic construct
  source 1..758: mol_type = other DNA
gcccagacagtcactcagtctcaaccagagatgtctgtgcaggaggcagagactgtgaccctgagttgcacatatgacaccagtgagaataattattatttgttctggtacaagcagcctcccagcaggcagatgattctcgttattcgccaagaagcttataagcaacagaatgcaacggagaatcgtttctctgtgaacttccagaaagcagccaaatccttcagtctcaagatctcagactcacagctgggggacactgcgatgtatttctgtgctttcgataacaatgccagactcatgttcggagatggaactcagctggtggtgaagcccatatccagaaccctgaccctgccgtgtaccagctgagagactctaaatccagtgacaagtctgtctgcctattcaccgattttgattctcaaacaaatgtgtcacaaagtaaggattctgatgtgtatatcacagacaaaactgtgctagacatgaggtctatggacttcaagagcaacagtgctgtggcctggagcaacaaatctgactttgcatgtgcaaacgccttcaacaacagcattattccagaagacaccttcttccccagcccagaaagttcctgtgatgtcaagctggtcgagaaaagctttgaaacagatacgaacctaaactttcaaaacctgtcagtgattgggttccgaatcctcctcctgaaagtggccgggtttaatctgctcatgacgctgcggctgtggtccagc

SEQ ID NO: 251 - DNA, 759 bp, synthetic construct
  source 1..759: mol_type = other DNA
ggtcaacagctgaatcagagtcctcaatctatgtttatccaggaaggagaagatgtctccatgaactgcacttcttcaagcatatttaacacctggctatggtacaagcaggaccctggggaaggtcctgtcctcttgatagccttatataaggctggtgaattgacctcaaatggaagactgactgctcagtttggtataaccagaaaggacagcttcctgaatatctcagcatccatacctagtgatgtaggcatctacttctgtgctggattttctcagggcggatctgaaaagctggtctttggaaagggaacgaaactgacagtaaacccatatatccagaaccctgaccctgccgtgtaccagctgagagactctaaatccagtgacaagtctgtctgcctattcaccgattttgattctcaaacaaatgtgtcacaaagtaaggattctgatgtgtatatcacagacaaaactgtgctagacatgaggtctatggacttcaagagcaacagtgctgtggcctggagcaacaaatctgactttgcatgtgcaaacgccttcaacaacagcattattccagaagacaccttcttccccagcccagaaagttcctgtgatgtcaagctggtcgagaaaagctttgaaacagatacgaacctaaactttcaaaacctgtcagtgattgggttccgaatcctcctcctgaaagtggccgggtttaatctgctcatgacgctgcggctgtggtccagc

SEQ ID NO: 252 - DNA, 750 bp, synthetic construct
  source 1..750: mol_type = other DNA
ggaatacaagtggagcagagtcctccagacctgattctccaggagggagccaattccacgctgcggtgcaatttttctgactctgtgaacaatttgcagtggtttcatcaaaacccttggggacagctcatcaacctgttttacattccctcagggacaaaacagaatggaagattaagcgccacgactgtcgctacggaacgctacagcttattgtacatttcctcttcccagaccacagactcaggcgtttatttctgtgctgtgttagccccaggaacctacaaatacatctttggaacaggcaccaggctgaaggttttagcaaatatccagaaccctgaccctgccgtgtaccagctgagagactctaaatccagtgacaagtctgtctgcctattcaccgattttgattctcaaacaaatgtgtcacaaagtaaggattctgatgtgtatatcacagacaaaactgtgctagacatgaggtctatggacttcaagagcaacagtgctgtggcctggagcaacaaatctgactttgcatgtgcaaacgccttcaacaacagcattattccagaagacaccttcttccccagcccagaaagttcctgtgatgtcaagctggtcgagaaaagctttgaaacagatacgaacctaaactttcaaaacctgtcagtgattgggttccgaatcctcctcctgaaagtggccgggtttaatctgctcatgacgctgcggctgtggtccagc

SEQ ID NO: 253 - DNA, 762 bp, synthetic construct
  source 1..762: mol_type = other DNA
agtcaacagggagaagaggatcctcaggccttgagcatccaggagggtgaaaatgccaccatgaactgcagttacaaaactagtataaacaatttacagtggtatagacaaaattcaggtagaggccttgtccacctaattttaatacgttcaaatgaaagagagaaacacagtggaagattaagagtcacgcttgacacttccaagaaaagcagttccttgttgatcacggcttcccgggcagcagacactgcttcttacttctgtgctacggacctctctggggctgggagttaccaactcactttcgggaaggggaccaaactctcggtcataccaaatatccagaaccctgaccctgccgtgtaccagctgagagactctaaatccagtgacaagtctgtctgcctattcaccgattttgattctcaaacaaatgtgtcacaaagtaaggattctgatgtgtatatcacagacaaaactgtgctagacatgaggtctatggacttcaagagcaacagtgctgtggcctggagcaacaaatctgactttgcatgtgcaaacgccttcaacaacagcattattccagaagacaccttcttccccagcccagaaagttcctgtgatgtcaagctggtcgagaaaagctttgaaacagatacgaacctaaactttcaaaacctgtcagtgattgggttccgaatcctcctcctgaaagtggccgggtttaatctgctcatgacgctgcggctgtggtccagc

SEQ ID NO: 254 - DNA, 756 bp, synthetic construct
  source 1..756: mol_type = other DNA
cagaaggaggtggagcagaattctggacccctcagtgttccagagggagccattgcctctctcaactgcacttacagtgaccgagtttcccagtccttcttctggtacagacaatattctgggaaaagccctgagttgataatgtccatatactccaatggtgacaaagaagatggaaggtttacagcacagctcaataaagccagccagtatgtttctctgctcatcagagactcccagcccagtgattcagccacctacctctgtgccgtggtcagttctaacgactacaagctcagctttggagccggaaccacagtaactgtaagagcaaatatccagaaccctgaccctgccgtgtaccagctgagagactctaaatccagtgacaagtctgtctgcctattcaccgattttgattctcaaacaaatgtgtcacaaagtaaggattctgatgtgtatatcacagacaaaactgtgctagacatgaggtctatggacttcaagagcaacagtgctgtggcctggagcaacaaatctgactttgcatgtgcaaacgccttcaacaacagcattattccagaagacaccttcttccccagcccagaaagttcctgtgatgtcaagctggtcgagaaaagctttgaaacagatacgaacctaaactttcaaaacctgtcagtgattgggttccgaatcctcctcctgaaagtggccgggtttaatctgctcatgacgctgcggctgtggtccagc

SEQ ID NO: 255 - DNA, 756 bp, synthetic construct
  source 1..756: mol_type = other DNA
cagaaggaggtggagcagaattctggacccctcagtgttccagagggagccattgcctctctcaactgcacttacagtgaccgagtttcccagtccttcttctggtacagacaatattctgggaaaagccctgagttgataatgtccatatactccaatggtgacaaagaagatggaaggtttacagcacagctcaataaagccagccagtatgtttctctgctcatcagagactcccagcccagtgattcagccacctacctctgtgccgtggcatcaggaggaagctacatacctacatttggaagaggaaccagccttattgttcatccgtatatccagaaccctgaccctgccgtgtaccagctgagagactctaaatccagtgacaagtctgtctgcctattcaccgattttgattctcaaacaaatgtgtcacaaagtaaggattctgatgtgtatatcacagacaaaactgtgctagacatgaggtctatggacttcaagagcaacagtgctgtggcctggagcaacaaatctgactttgcatgtgcaaacgccttcaacaacagcattattccagaagacaccttcttccccagcccagaaagttcctgtgatgtcaagctggtcgagaaaagctttgaaacagatacgaacctaaactttcaaaacctgtcagtgattgggttccgaatcctcctcctgaaagtggccgggtttaatctgctcatgacgctgcggctgtggtccagc

SEQ ID NO: 256 - DNA, 753 bp, synthetic construct
  source 1..753: mol_type = other DNA
ggagagagtgtggggctgcatcttcctaccctgagtgtccaggagggtgacaactctattatcaactgtgcttattcaaacagcgcctcagactacttcatttggtacaagcaagaatctggaaaaggtcctcaattcattatagacattcgttcaaatatggacaaaaggcaaggccaaagagtcaccgttttattgaataagacagtgaaacatctctctctgcaaattgcagctactcaacctggagactcagctgtctacttttgtgcagagagttatggccagaagctgctctttgcaagggggaccatgttaaaggtggatcttaatatccagaaccctgaccctgccgtgtaccagctgagagactctaaatccagtgacaagtctgtctgcctattcaccgattttgattctcaaacaaatgtgtcacaaagtaaggattctgatgtgtatatcacagacaaaactgtgctagacatgaggtctatggacttcaagagcaacagtgctgtggcctggagcaacaaatctgactttgcatgtgcaaacgccttcaacaacagcattattccagaagacaccttcttccccagcccagaaagttcctgtgatgtcaagctggtcgagaaaagctttgaaacagatacgaacctaaactttcaaaacctgtcagtgattgggttccgaatcctcctcctgaaagtggccgggtttaatctgctcatgacgctgcggctgtggtccagc

SEQ ID NO: 257 - DNA, 762 bp, synthetic construct
  source 1..762: mol_type = other DNA
ggtcaacagctgaatcagagtcctcaatctatgtttatccaggaaggagaagatgtctccatgaactgcacttcttcaagcatatttaacacctggctatggtacaagcaggaccctggggaaggtcctgtcctcttgatagccttatataaggctggtgaattgacctcaaatggaagactgactgctcagtttggtataaccagaaaggacagcttcctgaatatctcagcatccatacctagtgatgtaggcatctacttctgtgctgggcaggacgatggaggaagccaaggaaatctcatctttggaaaaggcactaaactctctgttaaaccaaatatccagaaccctgaccctgccgtgtaccagctgagagactctaaatccagtgacaagtctgtctgcctattcaccgattttgattctcaaacaaatgtgtcacaaagtaaggattctgatgtgtatatcacagacaaaactgtgctagacatgaggtctatggacttcaagagcaacagtgctgtggcctggagcaacaaatctgactttgcatgtgcaaacgccttcaacaacagcattattccagaagacaccttcttccccagcccagaaagttcctgtgatgtcaagctggtcgagaaaagctttgaaacagatacgaacctaaactttcaaaacctgtcagtgattgggttccgaatcctcctcctgaaagtggccgggtttaatctgctcatgacgctgcggctgtggtccagc

SEQ ID NO: 258 - DNA, 753 bp, synthetic construct
  source 1..753: mol_type = other DNA
caacaaccagtgcagagtcctcaagccgtgatcctccgagaaggggaagatgctgtcatcaactgcagttcctccaaggctttatattctgtacactggtacaggcagaagcatggtgaagcacccgtcttcctgatgatattactgaagggtggagaacagaagggtcatgacaaaatatctgcttcatttaatgaaaaaaagcagcaaagctccctgtaccttacggcctcccagctcagttactcaggaacctacttctgtggcacagagtttcggaacgactacaagctcagctttggagccggaaccacagtaactgtaagagcaaatatccagaaccctgaccctgccgtgtaccagctgagagactctaaatccagtgacaagtctgtctgcctattcaccgattttgattctcaaacaaatgtgtcacaaagtaaggattctgatgtgtatatcacagacaaaactgtgctagacatgaggtctatggacttcaagagcaacagtgctgtggcctggagcaacaaatctgactttgcatgtgcaaacgccttcaacaacagcattattccagaagacaccttcttccccagcccagaaagttcctgtgatgtcaagctggtcgagaaaagctttgaaacagatacgaacctaaactttcaaaacctgtcagtgattgggttccgaatcctcctcctgaaagtggccgggtttaatctgctcatgacgctgcggctgtggtccagc

SEQ ID NO: 259 - DNA, 756 bp, synthetic construct
  source 1..756: mol_type = other DNA
agtcaacagggagaagaggatcctcaggccttgagcatccaggagggtgaaaatgccaccatgaactgcagttacaaaactagtataaacaatttacagtggtatagacaaaattcaggtagaggccttgtccacctaattttaatacgttcaaatgaaagagagaaacacagtggaagattaagagtcacgcttgacacttccaagaaaagcagttccttgttgatcacggcttcccgggcagcagacactgcttcttacttctgtgctacggacgtaaagagcagctataaattgatcttcgggagtgggaccagactgctggtcaggcctgatatccagaaccctgaccctgccgtgtaccagctgagagactctaaatccagtgacaagtctgtctgcctattcaccgattttgattctcaaacaaatgtgtcacaaagtaaggattctgatgtgtatatcacagacaaaactgtgctagacatgaggtctatggacttcaagagcaacagtgctgtggcctggagcaacaaatctgactttgcatgtgcaaacgccttcaacaacagcattattccagaagacaccttcttccccagcccagaaagttcctgtgatgtcaagctggtcgagaaaagctttgaaacagatacgaacctaaactttcaaaacctgtcagtgattgggttccgaatcctcctcctgaaagtggccgggtttaatctgctcatgacgctgcggctgtggtccagc

SEQ ID NO: 260 - DNA, 762 bp, synthetic construct
  source 1..762: mol_type = other DNA
gaccagcaagttaagcaaaattcaccatccctgagcgtccaggaaggaagaatttctattctgaactgtgactatactaacagcatgtttgattatttcctatggtacaaaaaataccctgctgaaggtcctacattcctgatatctataagttccattaaggataaaaatgaagatggaagattcactgttttcttaaacaaaagtgccaagcacctctctctgcacattgtgccctcccagcctggagactctgcagtgtacttctgtgcagcatttgcttcggatagcaactatcagttaatctggggcgctgggaccaagctaattataaagccagatatccagaaccctgaccctgccgtgtaccagctgagagactctaaatccagtgacaagtctgtctgcctattcaccgattttgattctcaaacaaatgtgtcacaaagtaaggattctgatgtgtatatcacagacaaaactgtgctagacatgaggtctatggacttcaagagcaacagtgctgtggcctggagcaacaaatctgactttgcatgtgcaaacgccttcaacaacagcattattccagaagacaccttcttccccagcccagaaagttcctgtgatgtcaagctggtcgagaaaagctttgaaacagatacgaacctaaactttcaaaacctgtcagtgattgggttccgaatcctcctcctgaaagtggccgggtttaatctgctcatgacgctgcggctgtggtccagc

SEQ ID NO: 261 - DNA, 753 bp, synthetic construct
  source 1..753: mol_type = other DNA
cagaaggaggtggagcagaattctggacccctcagtgttccagagggagccattgcctctctcaactgcacttacagtgaccgagtttcccagtccttcttctggtacagacaatattctgggaaaagccctgagttgataatgtccatatactccaatggtgacaaagaagatggaaggtttacagcacagctcaataaagccagccagtatgtttctctgctcatcagagactcccagcccagtgattcagccacctacctctgtgcccttgtctcaggaacctacaaatacatctttggaacaggcaccaggctgaaggttttagcaaatatccagaaccctgaccctgccgtgtaccagctgagagactctaaatccagtgacaagtctgtctgcctattcaccgattttgattctcaaacaaatgtgtcacaaagtaaggattctgatgtgtatatcacagacaaaactgtgctagacatgaggtctatggacttcaagagcaacagtgctgtggcctggagcaacaaatctgactttgcatgtgcaaacgccttcaacaacagcattattccagaagacaccttcttccccagcccagaaagttcctgtgatgtcaagctggtcgagaaaagctttgaaacagatacgaacctaaactttcaaaacctgtcagtgattgggttccgaatcctcctcctgaaagtggccgggtttaatctgctcatgacgctgcggctgtggtccagc

SEQ ID NO: 262 - DNA, 753 bp, synthetic construct
  source 1..753: mol_type = other DNA
agtcaacagggagaagaggatcctcaggccttgagcatccaggagggtgaaaatgccaccatgaactgcagttacaaaactagtataaacaatttacagtggtatagacaaaattcaggtagaggccttgtccacctaattttaatacgttcaaatgaaagagagaaacacagtggaagattaagagtcacgcttgacacttccaagaaaagcagttccttgttgatcacggcttcccgggcagcagacactgcttcttacttctgtgctacgtatgctaacgactacaagctcagctttggagccggaaccacagtaactgtaagagcaaatatccagaaccctgaccctgccgtgtaccagctgagagactctaaatccagtgacaagtctgtctgcctattcaccgattttgattctcaaacaaatgtgtcacaaagtaaggattctgatgtgtatatcacagacaaaactgtgctagacatgaggtctatggacttcaagagcaacagtgctgtggcctggagcaacaaatctgactttgcatgtgcaaacgccttcaacaacagcattattccagaagacaccttcttccccagcccagaaagttcctgtgatgtcaagctggtcgagaaaagctttgaaacagatacgaacctaaactttcaaaacctgtcagtgattgggttccgaatcctcctcctgaaagtggccgggtttaatctgctcatgacgctgcggctgtggtccagc

SEQ ID NO: 263 - DNA, 750 bp, synthetic construct
  source 1..750: mol_type = other DNA
gaccagcaagttaagcaaaattcaccatccctgagcgtccaggaaggaagaatttctattctgaactgtgactatactaacagcatgtttgattatttcctatggtacaaaaaataccctgctgaaggtcctacattcctgatatctataagttccattaaggataaaaatgaagatggaagattcactgttttcttaaacaaaagtgccaagcacctctctctgcacattgtgccctcccagcctggagactctgcagtgtacttctgtgcagcaaagcccgacaagctcatctttgggactgggaccagattacaagtctttccaaatatccagaaccctgaccctgccgtgtaccagctgagagactctaaatccagtgacaagtctgtctgcctattcaccgattttgattctcaaacaaatgtgtcacaaagtaaggattctgatgtgtatatcacagacaaaactgtgctagacatgaggtctatggacttcaagagcaacagtgctgtggcctggagcaacaaatctgactttgcatgtgcaaacgccttcaacaacagcattattccagaagacaccttcttccccagcccagaaagttcctgtgatgtcaagctggtcgagaaaagctttgaaacagatacgaacctaaactttcaaaacctgtcagtgattgggttccgaatcctcctcctgaaagtggccgggtttaatctgctcatgacgctgcggctgtggtccagc

SEQ ID NO: 264 - DNA, 750 bp, synthetic construct
  source 1..750: mol_type = other DNA
cagaaggaggtggagcagaattctggacccctcagtgttccagagggagccattgcctctctcaactgcacttacagtgaccgaggttcccagtccttcttctggtacagacaatattctgggaaaagccctgagttgataatgtccatatactccaatggtgacaaagaagatggaaggtttacagcacagctcaataaagccagccagtatgtttctctgctcatcagagactcccagcccagtgattcagccacctacctctgtgccgtcccctcggggaacatgctcacctttggagggggaacaaggttaatggtcaaaccccatatccagaaccctgaccctgccgtgtaccagctgagagactctaaatccagtgacaagtctgtctgcctattcaccgattttgattctcaaacaaatgtgtcacaaagtaaggattctgatgtgtatatcacagacaaaactgtgctagacatgaggtctatggacttcaagagcaacagtgctgtggcctggagcaacaaatctgactttgcatgtgcaaacgccttcaacaacagcattattccagaagacaccttcttccccagcccagaaagttcctgtgatgtcaagctggtcgagaaaagctttgaaacagatacgaacctaaactttcaaaacctgtcagtgattgggttccgaatcctcctcctgaaagtggccgggtttaatctgctcatgacgctgcggctgtggtccagc

SEQ ID NO: 265 - DNA, 756 bp, synthetic construct
  source 1..756: mol_type = other DNA
agccaagaactggagcagagtcctcagtccttgatcgtccaagagggaaagaatctcaccataaactgcacgtcatcaaagacgttatatggcttatactggtataagcaaaagtatggtgaaggtcttatcttcttgatgatgctacagaaaggtggggaagagaaaagtcatgaaaagataactgccaagttggatgagaaaaagcagcaaagttccctgcatatcacagcctcccagcccagccatgcaggcatctacctctgtggagcagtcccgattaacgactacaagctcagctttggagccggaaccacagtaactgtaagagcaaatatccagaaccctgaccctgccgtgtaccagctgagagactctaaatccagtgacaagtctgtctgcctattcaccgattttgattctcaaacaaatgtgtcacaaagtaaggattctgatgtgtatatcacagacaaaactgtgctagacatgaggtctatggacttcaagagcaacagtgctgtggcctggagcaacaaatctgactttgcatgtgcaaacgccttcaacaacagcattattccagaagacaccttcttccccagcccagaaagttcctgtgatgtcaagctggtcgagaaaagctttgaaacagatacgaacctaaactttcaaaacctgtcagtgattgggttccgaatcctcctcctgaaagtggccgggtttaatctgctcatgacgctgcggctgtggtccagc

SEQ ID NO: 266 - DNA, 756 bp, synthetic construct
  source 1..756: mol_type = other DNA
cagaaggaggtggagcagaattctggacccctcagtgttccagagggagccattgcctctctcaactgcacttacagtgaccgaggttcccagtccttcttctggtacagacaatattctgggaaaagccctgagttgataatgtccatatactccaatggtgacaaagaagatggaaggtttacagcacagctcaataaagccagccagtatgtttctctgctcatcagagactcccagcccagtgattcagccacctacctctgtgccgttgtttctggtggctacaataagctgatttttggagcagggaccaggctggctgtacacccatatatccagaaccctgaccctgccgtgtaccagctgagagactctaaatccagtgacaagtctgtctgcctattcaccgattttgattctcaaacaaatgtgtcacaaagtaaggattctgatgtgtatatcacagacaaaactgtgctagacatgaggtctatggacttcaagagcaacagtgctgtggcctggagcaacaaatctgactttgcatgtgcaaacgccttcaacaacagcattattccagaagacaccttcttccccagcccagaaagttcctgtgatgtcaagctggtcgagaaaagctttgaaacagatacgaacctaaactttcaaaacctgtcagtgattgggttccgaatcctcctcctgaaagtggccgggtttaatctgctcatgacgctgcggctgtggtccagc

SEQ ID NO: 267 - protein, 5 aa, synthetic construct
KGHDR

SEQ ID NO: 268 - protein, 6 aa, synthetic construct
SFDVKD

SEQ ID NO: 269 - protein, 11 aa, synthetic construct
ATSDLLGRAQH

SEQ ID NO: 270 - protein, 5 aa, synthetic construct
KGHDR

SEQ ID NO: 271 - protein, 6 aa, synthetic construct
SFDVKD

SEQ ID NO: 272 - protein, 12 aa, synthetic construct
ATSDSRGGVEQY

SEQ ID NO: 273 - protein, 5 aa, synthetic construct
MGHRA

SEQ ID NO: 274 - protein, 6 aa, synthetic construct
YSYEKL

SEQ ID NO: 275 - protein, 14 aa, synthetic construct
ASSQDPFWGAGELF

SEQ ID NO: 276 - protein, 5 aa, synthetic construct
MNHEY

SEQ ID NO: 277 - protein, 6 aa, synthetic construct
SMNVEV

SEQ ID NO: 278 - protein, 12 aa, synthetic construct
ASSPGTSGNEQF

SEQ ID NO: 279 - protein, 6 aa, synthetic construct
DFQATT

SEQ ID NO: 280 - protein, 7 aa, synthetic construct
SNEGSKA

SEQ ID NO: 281 - protein, 10 aa, synthetic construct
SATEDNEKLF

SEQ ID NO: 282 - protein, 5 aa, synthetic construct
SGHRS

SEQ ID NO: 283 - protein, 6 aa, synthetic construct
YFSETQ

SEQ ID NO: 284 - protein, 13 aa, synthetic construct
ASSLEAGSFYEQY

SEQ ID NO: 285 - protein, 5 aa, synthetic construct
LGHDT

SEQ ID NO: 286 - protein, 6 aa, synthetic construct
YNNKEL

SEQ ID NO: 287 - protein, 12 aa, synthetic construct
ASSQGISGNTIY

SEQ ID NO: 288 - protein, 5 aa, synthetic construct
SGDLS

SEQ ID NO: 289 - protein, 6 aa, synthetic construct
YYNGEE

SEQ ID NO: 290 - protein, 13 aa, synthetic construct
ASSPWTSGSYEQY

SEQ ID NO: 291 - protein, 5 aa, synthetic construct
MNHEY

SEQ ID NO: 292 - protein, 6 aa, synthetic construct
SMNVEV

SEQ ID NO: 293 - protein, 13 aa, synthetic construct
ATQWASGSTDTQY

SEQ ID NO: 294 - protein, 5 aa, synthetic construct
MNHEY

SEQ ID NO: 295 - protein, 6 aa, synthetic construct
SMNVEV

SEQ ID NO: 296 - protein, 11 aa, synthetic construct
ASSSGTSDEQY

SEQ ID NO: 297 - protein, 5 aa, synthetic construct
SNHLY

SEQ ID NO: 298 - protein, 6 aa, synthetic construct
FYNNEI

SEQ ID NO: 299 - protein, 10 aa, synthetic construct
ASREDGYEQY

SEQ ID NO: 300 - protein, 5 aa, synthetic construct
MNHEY

SEQ ID NO: 301 - protein, 6 aa, synthetic construct
SMNVEV

SEQ ID NO: 302 - protein, 11 aa, synthetic construct
ATSPGTLYEQY

SEQ ID NO: 303 - protein, 5 aa, synthetic construct
SGDLS

SEQ ID NO: 304 - protein, 6 aa, synthetic construct
YYNGEE

SEQ ID NO: 305 - protein, 13 aa, synthetic construct
ASSPWLQGGNEQF

SEQ ID NO: 306 - protein, 5 aa, synthetic construct
SGHNS

SEQ ID NO: 307 - protein, 6 aa, synthetic construct
FNNNVP

SEQ ID NO: 308 - protein, 13 aa, synthetic construct
ASSIAALGFGELF

SEQ ID NO: 309 - protein, 5 aa, synthetic construct
SGDLS

SEQ ID NO: 310 - protein, 6 aa, synthetic construct
YYNGEE

SEQ ID NO: 311 - protein, 13 aa, synthetic construct
ASSVWSSGGNEQF

SEQ ID NO: 312 - protein, 5 aa, synthetic construct
MNHEY

SEQ ID NO: 313 - protein, 6 aa, synthetic construct
SMNVEV

SEQ ID NO: 314 - protein, 12 aa, synthetic construct
ASSPSSGYNEQF

SEQ ID NO: 315 - protein, 5 aa, synthetic construct
SGDLS

SEQ ID NO: 316 - protein, 6 aa, synthetic construct
YYNGEE

SEQ ID NO: 317 - protein, 13 aa, synthetic construct
ASSPWLAGGREQY

SEQ ID NO: 318 - protein, 5 aa, synthetic construct
MNHEY

SEQ ID NO: 319 - protein, 6 aa, synthetic construct
SMNVEV

SEQ ID NO: 320 - protein, 11 aa, synthetic construct
ASRWGLGGELF

SEQ ID NO: 321 - protein, 5 aa, synthetic construct
SGHDT

SEQ ID NO: 322 - protein, 6 aa, synthetic construct
YYEEEE

SEQ ID NO: 323 - protein, 10 aa, synthetic construct
ASSLVDYEQY

SEQ ID NO: 324 - protein, 5 aa, synthetic construct
LNHDA

SEQ ID NO: 325 - protein, 6 aa, synthetic construct
SQIVND

SEQ ID NO: 326 - protein, 11 aa, synthetic construct
ASLGLNYNEQF

SEQ ID NO: 327 - protein, 5 aa, synthetic construct
MNHEY

SEQ ID NO: 328 - protein, 6 aa, synthetic construct
SMNVEV

SEQ ID NO: 329 - protein, 13 aa, synthetic construct
ASRISLGANYGYT

SEQ ID NO: 330 - protein, 6 aa, synthetic construct
DFQATT

SEQ ID NO: 331 - protein, 7 aa, synthetic construct
SNEGSKA

SEQ ID NO: 332 - protein, 12 aa, synthetic construct
SATRDSSYNEQF

SEQ ID NO: 333 - protein, 5 aa, synthetic construct
SGDLS

SEQ ID NO: 334 - protein, 6 aa, synthetic construct
YYNGEE

SEQ ID NO: 335 - protein, 13 aa, synthetic construct
ASSPWTAGGNTIY

SEQ ID NO: 336 - protein, 5 aa, synthetic construct
MNHEY

SEQ ID NO: 337 - protein, 6 aa, synthetic construct
SMNVEV

SEQ ID NO: 338 - protein, 11 aa, synthetic construct
ASSWGSGYEQY

SEQ ID NO: 339 - protein, 5 aa, synthetic construct
MNHEY

SEQ ID NO: 340 - protein, 6 aa, synthetic construct
SMNVEV

SEQ ID NO: 341 - protein, 12 aa, synthetic construct
ASSLGTGFGELF

SEQ ID NO: 342 - protein, 5 aa, synthetic construct
MNHEY

SEQ ID NO: 343 - protein, 6 aa, synthetic construct
SMNVEV

SEQ ID NO: 344 - protein, 11 aa, synthetic construct
ASSPGTIGELF

SEQ ID NO: 345 - protein, 5 aa, synthetic construct
PRHDT

SEQ ID NO: 346 - protein, 6 aa, synthetic construct
FYEKMQ

SEQ ID NO: 347 - protein, 11 aa, synthetic construct
ASSLGRPEKLF

SEQ ID NO: 348 - protein, 5 aa, synthetic construct
MNHEY

SEQ ID NO: 349 - protein, 6 aa, synthetic construct
SMNVEV

SEQ ID NO: 350 - protein, 11 aa, synthetic construct
ASSFWSAGELF

SEQ ID NO: 351 - protein, 5 aa, synthetic construct
SGDLS

SEQ ID NO: 352 - protein, 6 aa, synthetic construct
YYNGEE

SEQ ID NO: 353 - protein, 14 aa, synthetic construct
ASSPWTSGGDGELF

SEQ ID NO: 354 - protein, 5 aa, synthetic construct
MNHEY

SEQ ID NO: 355 - protein, 6 aa, synthetic construct
SMNVEV

SEQ ID NO: 356 - protein, 12 aa, synthetic construct
ASSPGTGGYGYT

SEQ ID NO: 357 - protein, 5 aa, synthetic construct
PRHDT

SEQ ID NO: 358 - protein, 6 aa, synthetic construct
FYEKMQ

SEQ ID NO: 359 - protein, 12 aa, synthetic construct
ASSLGLLGNEQF

SEQ ID NO: 360 - protein, 5 aa, synthetic construct
LGHDT

SEQ ID NO: 361 - protein, 6 aa, synthetic construct
YNNKEL

SEQ ID NO: 362 - protein, 14 aa, synthetic construct
ASSPWTSGGNGELF

SEQ ID NO: 363 - protein, 5 aa, synthetic construct
LGHDT

SEQ ID NO: 364 - protein, 6 aa, synthetic construct
YNNKEL

SEQ ID NO: 365 - protein, 11 aa, synthetic construct
ASSPGLAYEQY

SEQ ID NO: 366 - protein, 5 aa, synthetic construct
MNHEY

SEQ ID NO: 367 - protein, 6 aa, synthetic construct
SMNVEV

SEQ ID NO: 368 - protein, 13 aa, synthetic construct
ASSAGTGGFVGYT

SEQ ID NO: 369 - protein, 5 aa, synthetic construct
SQVTM

SEQ ID NO: 370 - protein, 7 aa, synthetic construct
ANQGSEA

SEQ ID NO: 371 - protein, 14 aa, synthetic construct
SVWGAGLAIYNEQF

SEQ ID NO: 372 - protein, 5 aa, synthetic construct
MDHEN

SEQ ID NO: 373 - protein, 6 aa, synthetic construct
SYDVKM

SEQ ID NO: 374 - protein, 13 aa, synthetic construct
ASSSATSGSGEQY

SEQ ID NO: 375 - protein, 5 aa, synthetic construct
MNHEY

SEQ ID NO: 376 - protein, 6 aa, synthetic construct
SMNVEV

SEQ ID NO: 377 - protein, 14 aa, synthetic construct
ASSIDSGSSYNEQF

SEQ ID NO: 378 - protein, 5 aa, synthetic construct
SNHLY

SEQ ID NO: 379 - protein, 6 aa, synthetic construct
FYNNEI

SEQ ID NO: 380 - protein, 12 aa, synthetic construct
ASSEGWGGTEAF

SEQ ID NO: 381 - protein, 95 aa, synthetic construct
DADVTQTPRNRITKTGKRIMLECSQTKGHDRMYWYRQDPGLGLRLIYYSFDVKDINKGEISDGYSVSRQAQAKFSLSLESAIPNQTALYFCATSD

SEQ ID NO: 382 - protein, 95 aa, synthetic construct; identical to SEQ ID NO: 381

SEQ ID NO: 383 - protein, 95 aa, synthetic construct
DTEVTQTPKHLVMGMTNKKSLKCEQHMGHRAMYWYKQKAKKPPELMFVYSYEKLSINESVPSRFSPECPNSSLLNLHLHALQPEDSALYLCASSQ

SEQ ID NO: 384 - protein, 94 aa, synthetic construct
EAQVTQNPRYLITVTGKKLTVTCSQNMNHEYMSWYRQDPGLGLRQIYYSMNVEVTDKGDVPEGYKVSRKEKRNFPLILESPSPNQTSLYFCASS

SEQ ID NO: 385 - protein, 96 aa, synthetic construct
GAVVSQHPSRVICKSGTSVKIECRSLDFQATTMFWYRQFPKQSLMLMATSNEGSKATYEQGVEKDKFLINHASLTLSTLTVTSAHPEDSSFYICSA

SEQ ID NO: 386 - protein, 95 aa, synthetic construct
KAGVTQTPRYLIKTRGQQVTLSCSPISGHRSVSWYQQTPGQGLQFLFEYFSETQRNKGNFPGRFSGRQFSNSRSEMNVSTLELGDSALYLCASSL

SEQ ID NO: 387 - protein, 95 aa, synthetic construct
DTAVSQTPKYLVTQMGNDKSIKCEQNLGHDTMYWYKQDSKKFLKIMFSYNNKELIINETVPNRFSPKSPDKAHLNLHINSLELGDSAVYFCASSQ

SEQ ID NO: 388 - protein, 94 aa, synthetic construct
DSGVTQTPKHLITATGQRVTLRCSPRSGDLSVYWYQQSLDQGLQFLIQYYNGEERAKGNILERFSAQQFPDLHSELNLSSLELGDSALYFCASS

SEQ ID NO: 389 - protein, 92 aa, synthetic construct
EAQVTQNPRYLITVTGKKLTVTCSQNMNHEYMSWYRQDPGLGLRQIYYSMNVEVTDKGDVPEGYKVSRKEKRNFPLILESPSPNQTSLYFCA

SEQ ID NO: 390 - protein, 94 aa, synthetic construct; identical to SEQ ID NO: 384

SEQ ID NO: 391 - protein, 94 aa, synthetic construct
EPEVTQTPSHQVTQMGQEVILRCVPISNHLYFYWYRQILGQKVEFLVSFYNNEISEKSEIFDDQFSVERPDGSNFTLKIRSTKLEDSAMYFCAS

SEQ ID NO: 392 - protein, 92 aa, synthetic construct; identical to SEQ ID NO: 389

SEQ ID NO: 393 - protein, 94 aa, synthetic construct; identical to SEQ ID NO: 388

SEQ ID NO: 394 - protein, 95 aa, synthetic construct
DAGVIQSPRHEVTEMGQEVTLRCKPISGHNSLFWYRQTMMRGLELLIYFNNNVPIDDSGMPEDRFSAKMPNASFSTLKIQPSEPRDSAVYFCASS

SEQ ID NO: 395 - protein, 95 aa, synthetic construct
DSGVTQTPKHLITATGQRVTLRCSPRSGDLSVYWYQQSLDQGLQFLIQYYNGEERAKGNILERFSAQQFPDLHSELNLSSLELGDSALYFCASSV

SEQ ID NO: 396 - protein, 93 aa, synthetic construct
EAQVTQNPRYLITVTGKKLTVTCSQNMNHEYMSWYRQDPGLGLRQIYYSMNVEVTDKGDVPEGYKVSRKEKRNFPLILESPSPNQTSLYFCAS

SEQ ID NO: 397 - protein, 94 aa, synthetic construct; identical to SEQ ID NO: 388

SEQ ID NO: 398 - protein, 92 aa, synthetic construct; identical to SEQ ID NO: 389

SEQ ID NO: 399 - protein, 95 aa, synthetic construct
DAGVTQSPTHLIKTRGQQVTLRCSPKSGHDTVSWYQQALGQGPQFIFQYYEEEERQRGNFPDRFSGHQFPNYSSELNVNALLLGDSALYLCASSL

SEQ ID NO: 400 - protein, 92 aa, synthetic construct
DGGITQSPKYLFRKEGQNVTLSCEQNLNHDAMYWYRQDPGQGLRLIYYSQIVNDFQKGDIAEGYSVSREKKESFPLTVTSAQKNPTAFYLCA

SEQ ID NO: 401 - protein, 93 aa, synthetic construct; identical to SEQ ID NO: 396

SEQ ID NO: 402 - protein, 96 aa, synthetic construct
GAVVSQHPSWVICKSGTSVKIECRSLDFQATTMFWYRQFPKQSLMLMATSNEGSKATYEQGVEKDKFLINHASLTLSTLTVTSAHPEDSSFYICSA

SEQ ID NO: 403 - protein, 94 aa, synthetic construct; identical to SEQ ID NO: 388

SEQ ID NO: 404 - protein, 94 aa, synthetic construct; identical to SEQ ID NO: 384

SEQ ID NO: 405 - protein, 95 aa, synthetic construct
EAQVTQNPRYLITVTGKKLTVTCSQNMNHEYMSWYRQDPGLGLRQIYYSMNVEVTDKGDVPEGYKVSRKEKRNFPLILESPSPNQTSLYFCASSL

SEQ ID NO: 406 - protein, 93 aa, synthetic construct; identical to SEQ ID NO: 396

SEQ ID NO: 407 - protein, 94 aa, synthetic construct
AAGVIQSPRHLIKEKRETATLKCYPIPRHDTVYWYQQGPGQDPQFLISFYEKMQSDKGSIPDRFSAQQFSDYHSELNMSSLELGDSALYFCASS

SEQ ID NO: 408 - protein, 94 aa, synthetic construct; identical to SEQ ID NO: 384

SEQ ID NO: 409 - protein, 94 aa, synthetic construct; identical to SEQ ID NO: 388

SEQ ID NO: 410 - protein, 94 aa, synthetic construct; identical to SEQ ID NO: 384

SEQ ID NO: 411 - protein, 95 aa, synthetic construct
AAGVIQSPRHLIKEKRETATLKCYPIPRHDTVYWYQQGPGQDPQFLISFYEKMQSDKGSIPDRFSAQQFSDYHSELNMSSLELGDSALYFCASSL

SEQ ID NO: 412 - protein, 94 aa, synthetic construct
DTAVSQTPKYLVTQMGNDKSIKCEQNLGHDTMYWYKQDSKKFLKIMFSYNNKELIINETVPNRFSPKSPDKAHLNLHINSLELGDSAVYFCASS

SEQ ID NO: 413 - protein, 94 aa, synthetic construct; identical to SEQ ID NO: 412

SEQ ID NO: 414 - protein, 94 aa, synthetic construct; identical to SEQ ID NO: 384

SEQ ID NO: 415 - protein, 95 aa, synthetic construct
SAVISQKPSRDICQRGTSLTIQCQVDSQVTMMFWYRQQPGQSLTLIATANQGSEATYESGFVIDKFPISRPNLTFSTLTVSNMSPEDSSIYLCSV

SEQ ID NO: 416 - protein, 94 aa, synthetic construct
DVKVTQSSRYLVKRTGEKVFLECVQDMDHENMFWYRQDPGLGLRLIYFSYDVKMKEKGDIPEGYSVSREKKERFSLILESASTNQTSMYLCASS

SEQ ID NO: 417 - protein, 94 aa, synthetic construct; identical to SEQ ID NO: 384

SEQ ID NO: 418 - protein, 96 aa, synthetic construct
EPEVTQTPSHQVTQMGQEVILRCVPISNHLYFYWYRQILGQKVEFLVSFYNNEISEKSEIFDDQFSVERPDGSNFTLKIRSTKLEDSAMYFCASSE

SEQ ID NO: 419 - DNA, 285 bp, synthetic construct
  source 1..285: mol_type = other DNA
gatgctgatgttacccagaccccaaggaataggatcacaaagacaggaaagaggattatgctggaatgttctcagactaagggtcatgatagaatgtactggtatcgacaagacccaggactgggcctacggttgatctattactcctttgatgtcaaagatataaacaaaggagagatctctgatggatacagtgtctctcgacaggcacaggctaaattctccctgtccctagagtctgccatccccaaccagacagctctttacttctgtgccaccagtgat

SEQ ID NO: 420 - DNA, 285 bp, synthetic construct; identical to SEQ ID NO: 419
  source 1..285: mol_type = other DNA

SEQ ID NO: 421 - DNA, 285 bp, synthetic construct
  source 1..285: mol_type = other DNA
gacactgaagttacccagacaccaaaacacctggtcatgggaatgacaaataagaagtctttgaaatgtgaacaacatatggggcacagggctatgtattggtacaagcagaaagctaagaagccaccggagctcatgtttgtctacagctatgagaaactctctataaatgaaagtgtgccaagtcgcttctcacctgaatgccccaacagctctctcttaaaccttcacctacacgccctgcagccagaagactcagccctgtatctctgcgccagcagccaa

SEQ ID NO: 422 - DNA, 282 bp, synthetic construct
  source 1..282: mol_type = other DNA
gaagcccaagtgacccagaacccaagatacctcatcacagtgactggaaagaagttaacagtgacttgttctcagaatatgaaccatgagtatatgtcctggtatcgacaagacccagggctgggcttaaggcagatctactattcaatgaatgttgaggtgactgataagggagatgttcctgaagggtacaaagtctctcgaaaagagaagaggaatttccccctgatcctggagtcgcccagccccaaccagacctctctgtacttctgtgccagcagt

SEQ ID NO: 423 - DNA, 288 bp, synthetic construct
  source 1..288: mol_type = other DNA
ggtgctgtcgtctctcaacatccgagcagggttatctgtaagagtggaacctctgtgaagatcgagtgccgttccctggactttcaggccacaactatgttttggtatcgtcagttcccgaaacagagtctcatgctgatggcaacttccaatgagggctccaaggccacatacgagcaaggcgtcgagaaggacaagtttctcatcaaccatgcaagcctgaccttgtccactctgacagtgaccagtgcccatcctgaagacagcagcttctacatctgcagtgct

SEQ ID NO: 424 - DNA, 285 bp, synthetic construct
  source 1..285: mol_type = other DNA
aaggctggagtcactcaaactccaagatatctgatcaaaacgagaggacagcaagtgacactgagctgctcccctatctctgggcataggagtgtatcctggtaccaacagaccccaggacagggccttcagttcctctttgaatacttcagtgagacacagagaaacaaaggaaacttccctggtcgattctcagggcgccagttctctaactctcgctctgagatgaatgtgagcaccttggagctgggggactcggccctttatctttgcgccagcagcttg

SEQ ID NO: 425 - DNA, 285 bp, synthetic construct
  source 1..285: mol_type = other DNA
gacacagctgtttcccagactccaaaatacctggtcacacagatgggaaacgacaagtccattaaatgtgaacaaaatctgggccatgatactatgtattggtataaacaggactctaagaaatttctgaagataatgtttagctacaataataaggagctcattataaatgaaacagttccaaatcgcttctcacctaaatctccagacaaagctcacttaaatcttcacatcaattccctggagcttggtgactctgctgtgtatttctgtgccagcagccaa

SEQ ID NO: 426 - DNA, 282 bp, synthetic construct
  source 1..282: mol_type = other DNA
gattctggagtcacacaaaccccaaagcacctgatcacagcaactggacagcgagtgacgctgagatgctcccctaggtctggagacctctctgtgtactggtaccaacagagcctggaccagggcctccagttcctcattcagtattataatggagaagagagagcaaaaggaaacattcttgaacgattctccgcacaacagttccctgacttgcactctgaactaaacctgagctctctggagctgggggactcagctttgtatttctgtgccagcagc

SEQ ID NO: 427 - DNA, 276 bp, synthetic construct
  source 1..276: mol_type = other DNA
gaagcccaagtgacccagaacccaagatacctcatcacagtgactggaaagaagttaacagtgacttgttctcagaatatgaaccatgagtatatgtcctggtatcgacaagacccagggctgggcttaaggcagatctactattcaatgaatgttgaggtgactgataagggagatgttcctgaagggtacaaagtctctcgaaaagagaagaggaatttccccctgatcctggagtcgcccagccccaaccagacctctctgtacttctgtgcc

SEQ ID NO: 428 - DNA, 282 bp, synthetic construct; identical to SEQ ID NO: 422
  source 1..282: mol_type = other DNA

SEQ ID NO: 429 - DNA, 282 bp, synthetic construct
  source 1..282: mol_type = other DNA
gaacctgaagtcacccagactcccagccatcaggtcacacagatgggacaggaagtgatcttgcgctgtgtccccatctctaatcacttatacttctattggtacagacaaatcttggggcagaaagtcgagtttctggtttccttttataataatgaaatctcagagaagtctgaaatattcgatgatcaattctcagttgaaaggcctgatggatcaaatttcactctgaagatccggtccacaaagctggaggactcagccatgtacttctgtgccagc

SEQ ID NO: 430 - DNA, 276 bp, synthetic construct; identical to SEQ ID NO: 427
  source 1..276: mol_type = other DNA

SEQ ID NO: 431 - DNA, 282 bp, synthetic construct; identical to SEQ ID NO: 426
  source 1..282: mol_type = other DNA

SEQ ID NO: 432 - DNA, 285 bp, synthetic construct
  source 1..285: mol_type = other DNA
gatgctggagttatccagtcaccccgccatgaggtgacagagatgggacaagaagtgactctgagatgtaaaccaatttcaggccacaactcccttttctggtacagacagaccatgatgcggggactggagttgctcatttactttaacaacaacgttccgatagatgattcagggatgcccgaggatcgattctcagctaagatgcctaatgcatcattctccactctgaagatccagccctcagaacccagggactcagctgtgtacttctgtgccagcagt

SEQ ID NO: 433 - DNA, 285 bp, synthetic construct
  source 1..285: mol_type = other DNA
gattctggagtcacacaaaccccaaagcacctgatcacagcaactggacagcgagtgacgctgagatgctcccctaggtctggagacctctctgtgtactggtaccaacagagcctggaccagggcctccagttcctcattcagtattataatggagaagagagagcaaaaggaaacattcttgaacgattctccgcacaacagttccctgacttgcactctgaactaaacctgagctctctggagctgggggactcagctttgtatttctgtgccagcagcgta

SEQ ID NO: 434 - DNA, 279 bp, synthetic construct
  source 1..279: mol_type = other DNA
gaagcccaagtgacccagaacccaagatacctcatcacagtgactggaaagaagttaacagtgacttgttctcagaatatgaaccatgagtatatgtcctggtatcgacaagacccagggctgggcttaaggcagatctactattcaatgaatgttgaggtgactgataagggagatgttcctgaagggtacaaagtctctcgaaaagagaagaggaatttccccctgatcctggagtcgcccagccccaaccagacctctctgtacttctgtgccagc

SEQ ID NO: 435 - DNA, 282 bp, synthetic construct; identical to SEQ ID NO: 426
  source 1..282: mol_type = other DNA

SEQ ID NO: 436 - DNA, 276 bp, synthetic construct; identical to SEQ ID NO: 427
  source 1..276: mol_type = other DNA

SEQ ID NO: 437 - DNA, 285 bp, synthetic construct
  source 1..285: mol_type = other DNA
gacgctggagtcacccaaagtcccacacacctgatcaaaacgagaggacagcaagtgactctgagatgctctcctaagtctgggcatgacactgtgtcctggtaccaacaggccctgggtcaggggccccagtttatctttcagtattatgaggaggaagagagacagagaggcaacttccctgatcgattctcaggtcaccagttccctaactatagctctgagctgaatgtgaacgccttgttgctgggggactcggccctctatctctgtgccagcagcttg

SEQ ID NO: 438 - DNA, 276 bp, synthetic construct
  source 1..276: mol_type = other DNA
gatggtggaatcactcagtccccaaagtacctgttcagaaaggaaggacagaatgtgaccctgagttgtgaacagaatttgaaccacgatgccatgtactggtaccgacaggacccagggcaagggctgagattgatctactactcacagatagtaaatgactttcagaaaggagatatagctgaagggtacagcgtctctcgggagaagaaggaatcctttcctctcactgtgacatcggcccaaaagaacccgacagctttctatctctgtgcc

SEQ ID NO: 439 - DNA, 279 bp, synthetic construct; identical to SEQ ID NO: 434
  source 1..279: mol_type = other DNA

SEQ ID NO: 440 - DNA, 288 bp, synthetic construct
  source 1..288: mol_type = other DNA
ggtgctgtcgtctctcaacatccgagctgggttatctgcaagagtggaacctctgtgaagatcgagtgccgttccctggactttcaggccacaactatgttttggtatcgtcagttcccgaaacagagtctcatgctgatggcaacttccaatgagggctccaaggccacatacgagcaaggcgtcgagaaggacaagtttctcatcaaccatgcaagcctgaccttgtccactctgacagtgaccagtgcccatcctgaagacagcagcttctacatctgcagtgct

SEQ ID NO: 441 - DNA, 282 bp, synthetic construct; identical to SEQ ID NO: 426
  source 1..282: mol_type = other DNA

SEQ ID NO: 442 - DNA, 282 bp, synthetic construct; identical to SEQ ID NO: 422
  source 1..282: mol_type = other DNA

SEQ ID NO: 443 - DNA, 285 bp, synthetic construct
  source 1..285: mol_type = other DNA
gaagcccaagtgacccagaacccaagatacctcatcacagtgactggaaagaagttaacagtgacttgttctcagaatatgaaccatgagtatatgtcctggtatcgacaagacccagggctgggcttaaggcagatctactattcaatgaatgttgaggtgactgataagggagatgttcctgaagggtacaaagtctctcgaaaagagaagaggaatttccccctgatcctggagtcgcccagccccaaccagacctctctgtacttctgtgccagcagttta

SEQ ID NO: 444 - DNA, 279 bp, synthetic construct; identical to SEQ ID NO: 434
  source 1..279: mol_type = other DNA

SEQ ID NO: 445 - DNA, 282 bp, synthetic construct
  source 1..282: mol_type = other DNA
gctgctggagtcatccagtccccaagacatctgatcaaagaaaagagggaaacagccactctgaaatgctatcctatccctagacacgacactgtctactggtaccagcagggtccaggtcaggacccccagttcctcatttcgttttatgaaaagatgcagagcgataaaggaagcatccctgatcgattctcagctcaacagttcagtgactatcattctgaactgaacatgagctccttggagctgggggactcagccctgtacttctgtgccagcagc

SEQ ID NO: 446 - DNA, 282 bp, synthetic construct; identical to SEQ ID NO: 422
  source 1..282: mol_type = other DNA

SEQ ID NO: 447 - DNA, 282 bp, synthetic construct
  source 1..282: mol_type = other DNA
gattctggagtcacacaaaccccaaagcacctgatcacagcaactggacagcgagtgacgctgagatgctcccctaggtctggtgacctctctgtgtactggtaccaacagagcctggaccagggcctccagttcctcattcagtattataatggagaagagagagcaaaaggaaacattcttgaacgattctccgcacaacagttccctgacttgcactctgaactaaacctgagctctctggagctgggggactcagctttgtatttctgtgccagcagc

SEQ ID NO: 448 - DNA, 282 bp, synthetic construct; identical to SEQ ID NO: 422
  source 1..282: mol_type = other DNA

SEQ ID NO: 449 - DNA, 285 bp, synthetic construct
  source 1..285: mol_type = other DNA
gctgctggagtcatccagtccccaagacatctgatcaaagaaaagagggaaacagccactctgaaatgctatcctatccctagacacgacactgtctactggtaccagcagggtccaggtcaggacccccagttcctcatttcgttttatgaaaagatgcagagcgataaaggaagcatccctgatcgattctcagctcaacagttcagtgactatcattctgaactgaacatgagctccttggagctgggggactcagccctgtacttctgtgccagcagctta

SEQ ID NO: 450 - DNA, 282 bp, synthetic construct
  source 1..282: mol_type = other DNA
gacacagctgtttcccagactccaaaatacctggtcacacagatgggaaacgacaagtccattaaatgtgaacaaaatctgggccatgatactatgtattggtataaacaggactctaagaaatttctgaagataatgtttagctacaataataaggagctcattataaatgaaacagttccaaatcgcttctcacctaaatctccagacaaagctcacttaaatcttcacatcaattccctggagcttggtgactctgctgtgtatttctgtgccagcagc

SEQ ID NO: 451 - DNA, 282 bp, synthetic construct; identical to SEQ ID NO: 450
  source 1..282: mol_type = other DNA

SEQ ID NO: 452 - DNA, 282 bp, synthetic construct; identical to SEQ ID NO: 422
  source 1..282: mol_type = other DNA

SEQ ID NO: 453 - DNA, 285 bp, synthetic construct
  source 1..285: mol_type = other DNA
agtgctgtcatctctcaaaagccaagcagggatatctgtcaacgtggaacctccctgacgatccagtgtcaagtcgatagccaagtcaccatgatgttctggtaccgtcagcaacctggacagagcctgacactgatcgcaactgcaaatcagggctctgaggccacatatgagagtggatttgtcattgacaagtttcccatcagccgcccaaacctaacattctcaactctgactgtgagcaacatgagccctgaagacagcagcatatatctctgcagcgtt

SEQ ID NO: 454 - DNA, 282 bp, synthetic construct
  source 1..282: mol_type = other DNA
gatgtgaaagtaacccagagctcgagatatctagtcaaaaggacgggagagaaagtttttctggaatgtgtccaggatatggaccatgaaaatatgttctggtatcgacaagacccaggtctggggctacggctgatctatttctcatatgatgttaaaatgaaagaaaaaggagatattcctgaggggtacagtgtctctagagagaagaaggagcgcttctccctgattctggagtccgccagcaccaaccagacatctatgtacctctgtgccagcagt

SEQ ID NO: 455 - DNA, 282 bp, synthetic construct; identical to SEQ ID NO: 422
  source 1..282: mol_type = other DNA

SEQ ID NO: 456 - DNA, 288 bp, synthetic construct
  source 1..288: mol_type = other DNA
gaacctgaagtcacccagactcccagccatcaggtcacacagatgggacaggaagtgatcttgcgctgtgtccccatctctaatcacttatacttctattggtacagacaaatcttggggcagaaagtcgagtttctggtttccttttataataatgaaatctcagagaagtctgaaatattcgatgatcaattctcagttgaaaggcctgatggatcaaatttcactctgaagatccggtccacaaagctggaggactcagccatgtacttctgtgccagcagtgaa

SEQ ID NO: 457 - protein, 20 aa, synthetic construct
YGGSQGNLIFGKGTKLSVKP

SEQ ID NO: 458 - DNA, 60 bp, synthetic construct
  source 1..60: mol_type = other DNA
tatggaggaagccaaggaaatctcatctttggaaaaggcactaaactctctgttaaacca

SEQ ID NO: 459 - protein, 289 aa, synthetic construct
DADVTQTPRNRITKTGKRIMLECSQTKGHDRMYWYRQDPGLGLRLIYYSFDVKDINKGEISDGYSVSRQAQAKFSLSLESAIPNQTALYFCATSDLLGRAQHFGDGTRLSILEDLNKVFPPEVAVFEPSEAEISHTQKATLVCLATGFFPDHVELSWWVNGKEVHSGVSTDPQPLKEQPALNDSRYCLSSRLRVSATFWQNPRNHFRCQVQFYGLSENDEWTQDRAKPVTQIVSAEAWGRADCGFTSVSYQQGVLSATILYEILLGKATLYAVLVSALVLMAMVKRKDF

SEQ ID NO: 460 - protein, 292 aa, synthetic construct
DADVTQTPRNRITKTGKRIMLECSQTKGHDRMYWYRQDPGLGLRLIYYSFDVKDINKGEISDGYSVSRQAQAKFSLSLESAIPNQTALYFCATSDSRGGVEQYFGPGTRLTVTEDLKNVFPPEVAVFEPSEAEISHTQKATLVCLATGFYPDHVELSWWVNGKEVHSGVSTDPQPLKEQPALNDSRYCLSSRLRVSATFWQNPRNHFRCQVQFYGLSENDEWTQDRAKPVTQIVSAEAWGRADCGFTSESYQQGVLSATILYEILLGKATLYAVLVSALVLMAMVKRKDSRG

SEQ ID NO: 461 - protein, 294 aa, synthetic construct
DTEVTQTPKHLVMGMTNKKSLKCEQHMGHRAMYWYKQKAKKPPELMFVYSYEKLSINESVPSRFSPECPNSSLLNLHLHALQPEDSALYLCASSQDPFWGAGELFFGEGSRLTVLEDLKNVFPPEVAVFEPSEAEISHTQKATLVCLATGFYPDHVELSWWVNGKEVHSGVSTDPQPLKEQPALNDSRYCLSSRLRVSATFWQNPRNHFRCQVQFYGLSENDEWTQDRAKPVTQIVSAEAWGRADCGFTSESYQQGVLSATILYEILLGKATLYAVLVSALVLMAMVKRKDSRG

SEQ ID NO: 462 - protein, 292 aa, synthetic construct
EAQVTQNPRYLITVTGKKLTVTCSQNMNHEYMSWYRQDPGLGLRQIYYSMNVEVTDKGDVPEGYKVSRKEKRNFPLILESPSPNQTSLYFCASSPGTSGNEQFFGPGTRLTVLEDLKNVFPPEVAVFEPSEAEISHTQKATLVCLATGFYPDHVELSWWVNGKEVHSGVSTDPQPLKEQPALNDSRYCLSSRLRVSATFWQNPRNHFRCQVQFYGLSENDEWTQDRAKPVTQIVSAEAWGRADCGFTSESYQQGVLSATILYEILLGKATLYAVLVSALVLMAMVKRKDSRG

SEQ ID NO: 463 - protein, 291 aa, synthetic construct
GAVVSQHPSRVICKSGTSVKIECRSLDFQATTMFWYRQFPKQSLMLMATSNEGSKATYEQGVEKDKFLINHASLTLSTLTVTSAHPEDSSFYICSATEDNEKLFFGSGTQLSVLEDLNKVFPPEVAVFEPSEAEISHTQKATLVCLATGFFPDHVELSWWVNGKEVHSGVSTDPQPLKEQPALNDSRYCLSSRLRVSATFWQNPRNHFRCQVQFYGLSENDEWTQDRAKPVTQIVSAEAWGRADCGFTSVSYQQGVLSATILYEILLGKATLYAVLVSALVLMAMVKRKDF

SEQ ID NO: 464 - protein, 293 aa, synthetic construct
KAGVTQTPRYLIKTRGQQVTLSCSPISGHRSVSWYQQTPGQGLQFLFEYFSETQRNKGNFPGRFSGRQFSNSRSEMNVSTLELGDSALYLCASSLEAGSFYEQYFGPGTRLTVTEDLKNVFPPEVAVFEPSEAEISHTQKATLVCLATGFYPDHVELSWWVNGKEVHSGVSTDPQPLKEQPALNDSRYCLSSRLRVSATFWQNPRNHFRCQVQFYGLSENDEWTQDRAKPVTQIVSAEAWGRADCGFTSESYQQGVLSATILYEILLGKATLYAVLVSALVLMAMVKRKDSRG

SEQ ID NO: 465 - protein, 290 aa, synthetic construct
DTAVSQTPKYLVTQMGNDKSIKCEQNLGHDTMYWYKQDSKKFLKIMFSYNNKELIINETVPNRFSPKSPDKAHLNLHINSLELGDSAVYFCASSQGISGNTIYFGEGSWLTVVEDLNKVFPPEVAVFEPSEAEISHTQKATLVCLATGFFPDHVELSWWVNGKEVHSGVSTDPQPLKEQPALNDSRYCLSSRLRVSATFWQNPRNHFRCQVQFYGLSENDEWTQDRAKPVTQIVSAEAWGRADCGFTSVSYQQGVLSATILYEILLGKATLYAVLVSALVLMAMVKRKDF

SEQ ID NO: 466 - protein, 293 aa, synthetic construct
DSGVTQTPKHLITATGQRVTLRCSPRSGDLSVYWYQQSLDQGLQFLIQYYNGEERAKGNILERFSAQQFPDLHSELNLSSLELGDSALYFCASSPWTSGSYEQYFGPGTRLTVTEDLKNVFPPEVAVFEPSEAEISHTQKATLVCLATGFYPDHVELSWWVNGKEVHSGVSTDPQPLKEQPALNDSRYCLSSRLRVSATFWQNPRNHFRCQVQFYGLSENDEWTQDRAKPVTQIVSAEAWGRADCGFTSESYQQGVLSATILYEILLGKATLYAVLVSALVLMAMVKRKDSRG

SEQ ID NO: 467 - protein, 293 aa, synthetic construct
EAQVTQNPRYLITVTGKKLTVTCSQNMNHEYMSWYRQDPGLGLRQIYYSMNVEVTDKGDVPEGYKVSRKEKRNFPLILESPSPNQTSLYFCATQWASGSTDTQYFGPGTRLTVLEDLKNVFPPEVAVFEPSEAEISHTQKATLVCLATGFYPDHVELSWWVNGKEVHSGVSTDPQPLKEQPALNDSRYCLSSRLRVSATFWQNPRNHFRCQVQFYGLSENDEWTQDRAKPVTQIVSAEAWGRADCGFTSESYQQGVLSATILYEILLGKATLYAVLVSALVLMAMVKRKDSRG

SEQ ID NO: 468 - protein, 291 aa, synthetic construct
EAQVTQNPRYLITVTGKKLTVTCSQNMNHEYMSWYRQDPGLGLRQIYYSMNVEVTDKGDVPEGYKVSRKEKRNFPLILESPSPNQTSLYFCASSSGTSDEQYFGPGTRLTVTEDLKNVFPPEVAVFEPSEAEISHTQKATLVCLATGFYPDHVELSWWVNGKEVHSGVSTDPQPLKEQPALNDSRYCLSSRLRVSATFWQNPRNHFRCQVQFYGLSENDEWTQDRAKPVTQIVSAEAWGRADCGFTSESYQQGVLSATILYEILLGKATLYAVLVSALVLMAMVKRKDSRG

SEQ ID NO: 469 - protein, 291 aa, synthetic construct
EPEVTQTPSHQVTQMGQEVILRCVPISNHLYFYWYRQILGQKVEFLVSFYNNEISEKSEIFDDQFSVERPDGSNFTLKIRSTKLEDSAMYFCASREDGYEQYFGPGTRLTVTEDLKNVFPPEVAVFEPSEAEISHTQKATLVCLATGFYPDHVELSWWVNGKEVHSGVSTDPQPLKEQPALNDSRYCLSSRLRVSATFWQNPRNHFRCQVQFYGLSENDEWTQDRAKPVTQIVSAEAWGRADCGFTSESYQQGVLSATILYEILLGKATLYAVLVSALVLMAMVKRKDSRG

SEQ ID NO: 470 - protein, 291 aa, synthetic construct
EAQVTQNPRYLITVTGKKLTVTCSQNMNHEYMSWYRQDPGLGLRQIYYSMNVEVTDKGDVPEGYKVSRKEKRNFPLILESPSPNQTSLYFCATSPGTLYEQYFGPGTRLTVTEDLKNVFPPEVAVFEPSEAEISHTQKATLVCLATGFYPDHVELSWWVNGKEVHSGVSTDPQPLKEQPALNDSRYCLSSRLRVSATFWQNPRNHFRCQVQFYGLSENDEWTQDRAKPVTQIVSAEAWGRADCGFTSESYQQGVLSATILYEILLGKATLYAVLVSALVLMAMVKRKDSRG

SEQ ID NO: 471 - protein, 293 aa, synthetic construct
DSGVTQTPKHLITATGQRVTLRCSPRSGDLSVYWYQQSLDQGLQFLIQYYNGEERAKGNILERFSAQQFPDLHSELNLSSLELGDSALYFCASSPWLQGGNEQFFGPGTRLTVLEDLKNVFPPEVAVFEPSEAEISHTQKATLVCLATGFYPDHVELSWWVNGKEVHSGVSTDPQPLKEQPALNDSRYCLSSRLRVSATFWQNPRNHFRCQVQFYGLSENDEWTQDRAKPVTQIVSAEAWGRADCGFTSESYQQGVLSATILYEILLGKATLYAVLVSALVLMAMVKRKDSRG

SEQ ID NO: 472 - protein, 294 aa, synthetic construct
DAGVIQSPRHEVTEMGQEVTLRCKPISGHNSLFWYRQTMMRGLELLIYFNNNVPIDDSGMPEDRFSAKMPNASFSTLKIQPSEPRDSAVYFCASSIAALGFGELFFGEGSRLTVLEDLKNVFPPEVAVFEPSEAEISHTQKATLVCLATGFYPDHVELSWWVNGKEVHSGVSTDPQPLKEQPALNDSRYCLSSRLRVSATFWQNPRNHFRCQVQFYGLSENDEWTQDRAKPVTQIVSAEAWGRADCGFTSESYQQGVLSATILYEILLGKATLYAVLVSALVLMAMVKRKDSRG

SEQ ID NO: 473 - protein, 293 aa, synthetic construct
DSGVTQTPKHLITATGQRVTLRCSPRSGDLSVYWYQQSLDQGLQFLIQYYNGEERAKGNILERFSAQQFPDLHSELNLSSLELGDSALYFCASSVWSSGGNEQFFGPGTRLTVLEDLKNVFPPEVAVFEPSEAEISHTQKATLVCLATGFYPDHVELSWWVNGKEVHSGVSTDPQPLKEQPALNDSRYCLSSRLRVSATFWQNPRNHFRCQVQFYGLSENDEWTQDRAKPVTQIVSAEAWGRADCGFTSESYQQGVLSATILYEILLGKATLYAVLVSALVLMAMVKRKDSRG

SEQ ID NO: 474 - protein, 292 aa, synthetic construct
EAQVTQNPRYLITVTGKKLTVTCSQNMNHEYMSWYRQDPGLGLRQIYYSMNVEVTDKGDVPEGYKVSRKEKRNFPLILESPSPNQTSLYFCASSPSSGYNEQFFGPGTRLTVLEDLKNVFPPEVAVFEPSEAEISHTQKATLVCLATGFYPDHVELSWWVNGKEVHSGVSTDPQPLKEQPALNDSRYCLSSRLRVSATFWQNPRNHFRCQVQFYGLSENDEWTQDRAKPVTQIVSAEAWGRADCGFTSESYQQGVLSATILYEILLGKATLYAVLVSALVLMAMVKRKDSRG

SEQ ID NO: 475 - protein, 293 aa, synthetic construct
DSGVTQTPKHLITATGQRVTLRCSPRSGDLSVYWYQQSLDQGLQFLIQYYNGEERAKGNILERFSAQQFPDLHSELNLSSLELGDSALYFCASSPWLAGGREQYFGPGTRLTVTEDLKNVFPPEVAVFEPSEAEISHTQKATLVCLATGFYPDHVELSWWVNGKEVHSGVSTDPQPLKEQPALNDSRYCLSSRLRVSATFWQNPRNHFRCQVQFYGLSENDEWTQDRAKPVTQIVSAEAWGRADCGFTSESYQQGVLSATILYEILLGKATLYAVLVSALVLMAMVKRKDSRG

SEQ ID NO: 476 - protein, 291 aa, synthetic construct
EAQVTQNPRYLITVTGKKLTVTCSQNMNHEYMSWYRQDPGLGLRQIYYSMNVEVTDKGDVPEGYKVSRKEKRNFPLILESPSPNQTSLYFCASRWGLGGELFFGEGSRLTVLEDLKNVFPPEVAVFEPSEAEISHTQKATLVCLATGFYPDHVELSWWVNGKEVHSGVSTDPQPLKEQPALNDSRYCLSSRLRVSATFWQNPRNHFRCQVQFYGLSENDEWTQDRAKPVTQIVSAEAWGRADCGFTSESYQQGVLSATILYEILLGKATLYAVLVSALVLMAMVKRKDSRG

SEQ ID NO: 477 - protein, 290 aa, synthetic construct
DAGVTQSPTHLIKTRGQQVTLRCSPKSGHDTVSWYQQALGQGPQFIFQYYEEEERQRGNFPDRFSGHQFPNYSSELNVNALLLGDSALYLCASSLVDYEQYFGPGTRLTVTEDLKNVFPPEVAVFEPSEAEISHTQKATLVCLATGFYPDHVELSWWVNGKEVHSGVSTDPQPLKEQPALNDSRYCLSSRLRVSATFWQNPRNHFRCQVQFYGLSENDEWTQDRAKPVTQIVSAEAWGRADCGFTSESYQQGVLSATILYEILLGKATLYAVLVSALVLMAMVKRKDSRG

SEQ ID NO: 478 - protein, 291 aa, synthetic construct
DGGITQSPKYLFRKEGQNVTLSCEQNLNHDAMYWYRQDPGQGLRLIYYSQIVNDFQKGDIAEGYSVSREKKESFPLTVTSAQKNPTAFYLCASLGLNYNEQFFGPGTRLTVLEDLKNVFPPEVAVFEPSEAEISHTQKATLVCLATGFYPDHVELSWWVNGKEVHSGVSTDPQPLKEQPALNDSRYCLSSRLRVSATFWQNPRNHFRCQVQFYGLSENDEWTQDRAKPVTQIVSAEAWGRADCGFTSESYQQGVLSATILYEILLGKATLYAVLVSALVLMAMVKRKDSRG

SEQ ID NO: 479 - protein, 291 aa, synthetic construct
EAQVTQNPRYLITVTGKKLTVTCSQNMNHEYMSWYRQDPGLGLRQIYYSMNVEVTDKGDVPEGYKVSRKEKRNFPLILESPSPNQTSLYFCASRISLGANYGYTFGSGTRLTVVEDLNKVFPPEVAVFEPSEAEISHTQKATLVCLATGFFPDHVELSWWVNGKEVHSGVSTDPQPLKEQPALNDSRYCLSSRLRVSATFWQNPRNHFRCQVQFYGLSENDEWTQDRAKPVTQIVSAEAWGRADCGFTSVSYQQGVLSATILYEILLGKATLYAVLVSALVLMAMVKRKDF

SEQ ID NO: 480 - protein, 295 aa, synthetic construct
GAVVSQHPSWVICKSGTSVKIECRSLDFQATTMFWYRQFPKQSLMLMATSNEGSKATYEQGVEKDKFLINHASLTLSTLTVTSAHPEDSSFYICSATRDSSYNEQFFGPGTRLTVLEDLKNVFPPEVAVFEPSEAEISHTQKATLVCLATGFYPDHVELSWWVNGKEVHSGVSTDPQPLKEQPALNDSRYCLSSRLRVSATFWQNPRNHFRCQVQFYGLSENDEWTQDRAKPVTQIVSAEAWGRADCGFTSESYQQGVLSATILYEILLGKATLYAVLVSALVLMAMVKRKDSRG

SEQ ID NO: 481 - protein, 291 aa, synthetic construct
DSGVTQTPKHLITATGQRVTLRCSPRSGDLSVYWYQQSLDQGLQFLIQYYNGEERAKGNILERFSAQQFPDLHSELNLSSLELGDSALYFCASSPWTAGGNTIYFGEGSWLTVVEDLNKVFPPEVAVFEPSEAEISHTQKATLVCLATGFFPDHVELSWWVNGKEVHSGVSTDPQPLKEQPALNDSRYCLSSRLRVSATFWQNPRNHFRCQVQFYGLSENDEWTQDRAKPVTQIVSAEAWGRADCGFTSVSYQQGVLSATILYEILLGKATLYAVLVSALVLMAMVKRKDF

SEQ ID NO: 482 - protein, 291 aa, synthetic construct
EAQVTQNPRYLITVTGKKLTVTCSQNMNHEYMSWYRQDPGLGLRQIYYSMNVEVTDKGDVPEGYKVSRKEKRNFPLILESPSPNQTSLYFCASSWGSGYEQYFGPGTRLTVTEDLKNVFPPEVAVFEPSEAEISHTQKATLVCLATGFYPDHVELSWWVNGKEVHSGVSTDPQPLKEQPALNDSRYCLSSRLRVSATFWQNPRNHFRCQVQFYGLSENDEWTQDRAKPVTQIVSAEAWGRADCGFTSESYQQGVLSATILYEILLGKATLYAVLVSALVLMAMVKRKDSRG

SEQ ID NO: 483 - protein, 292 aa, synthetic construct
EAQVTQNPRYLITVTGKKLTVTCSQNMNHEYMSWYRQDPGLGLRQIYYSMNVEVTDKGDVPEGYKVSRKEKRNFPLILESPSPNQTSLYFCASSLGTGFGELFFGEGSRLTVLEDLKNVFPPEVAVFEPSEAEISHTQKATLVCLATGFYPDHVELSWWVNGKEVHSGVSTDPQPLKEQPALNDSRYCLSSRLRVSATFWQNPRNHFRCQVQFYGLSENDEWTQDRAKPVTQIVSAEAWGRADCGFTSESYQQGVLSATILYEILLGKATLYAVLVSALVLMAMVKRKDSRG

SEQ ID NO: 484 - protein, 291 aa, synthetic construct
EAQVTQNPRYLITVTGKKLTVTCSQNMNHEYMSWYRQDPGLGLRQIYYSMNVEVTDKGDVPEGYKVSRKEKRNFPLILESPSPNQTSLYFCASSPGTIGELFFGEGSRLTVLEDLKNVFPPEVAVFEPSEAEISHTQKATLVCLATGFYPDHVELSWWVNGKEVHSGVSTDPQPLKEQPALNDSRYCLSSRLRVSATFWQNPRNHFRCQVQFYGLSENDEWTQDRAKPVTQIVSAEAWGRADCGFTSESYQQGVLSATILYEILLGKATLYAVLVSALVLMAMVKRKDSRG

SEQ ID NO: 485 - protein, 289 aa, synthetic construct
AAGVIQSPRHLIKEKRETATLKCYPIPRHDTVYWYQQGPGQDPQFLISFYEKMQSDKGSIPDRFSAQQFSDYHSELNMSSLELGDSALYFCASSLGRPEKLFFGSGTQLSVLEDLNKVFPPEVAVFEPSEAEISHTQKATLVCLATGFFPDHVELSWWVNGKEVHSGVSTDPQPLKEQPALNDSRYCLSSRLRVSATFWQNPRNHFRCQVQFYGLSENDEWTQDRAKPVTQIVSAEAWGRADCGFTSVSYQQGVLSATILYEILLGKATLYAVLVSALVLMAMVKRKDF

SEQ ID NO: 486 - protein, 291 aa, synthetic construct
EAQVTQNPRYLITVTGKKLTVTCSQNMNHEYMSWYRQDPGLGLRQIYYSMNVEVTDKGDVPEGYKVSRKEKRNFPLILESPSPNQTSLYFCASSFWSAGELFFGEGSRLTVLEDLKNVFPPEVAVFEPSEAEISHTQKATLVCLATGFYPDHVELSWWVNGKEVHSGVSTDPQPLKEQPALNDSRYCLSSRLRVSATFWQNPRNHFRCQVQFYGLSENDEWTQDRAKPVTQIVSAEAWGRADCGFTSESYQQGVLSATILYEILLGKATLYAVLVSALVLMAMVKRKDSRG

SEQ ID NO: 487 - protein, 294 aa, synthetic construct
DSGVTQTPKHLITATGQRVTLRCSPRSGDLSVYWYQQSLDQGLQFLIQYYNGEERAKGNILERFSAQQFPDLHSELNLSSLELGDSALYFCASSPWTSGGDGELFFGEGSRLTVLEDLKNVFPPEVAVFEPSEAEISHTQKATLVCLATGFYPDHVELSWWVNGKEVHSGVSTDPQPLKEQPALNDSRYCLSSRLRVSATFWQNPRNHFRCQVQFYGLSENDEWTQDRAKPVTQIVSAEAWGRADCGFTSESYQQGVLSATILYEILLGKATLYAVLVSALVLMAMVKRKDSRG

SEQ ID NO: 488 - protein, 290 aa, synthetic construct
EAQVTQNPRYLITVTGKKLTVTCSQNMNHEYMSWYRQDPGLGLRQIYYSMNVEVTDKGDVPEGYKVSRKEKRNFPLILESPSPNQTSLYFCASSPGTGGYGYTFGSGTRLTVVEDLNKVFPPEVAVFEPSEAEISHTQKATLVCLATGFFPDHVELSWWVNGKEVHSGVSTDPQPLKEQPALNDSRYCLSSRLRVSATFWQNPRNHFRCQVQFYGLSENDEWTQDRAKPVTQIVSAEAWGRADCGFTSVSYQQGVLSATILYEILLGKATLYAVLVSALVLMAMVKRKDF

SEQ ID NO: 489 - protein, 292 aa, synthetic construct
AAGVIQSPRHLIKEKRETATLKCYPIPRHDTVYWYQQGPGQDPQFLISFYEKMQSDKGSIPDRFSAQQFSDYHSELNMSSLELGDSALYFCASSLGLLGNEQFFGPGTRLTVLEDLKNVFPPEVAVFEPSEAEISHTQKATLVCLATGFYPDHVELSWWVNGKEVHSGVSTDPQPLKEQPALNDSRYCLSSRLRVSATFWQNPRNHFRCQVQFYGLSENDEWTQDRAKPVTQIVSAEAWGRADCGFTSESYQQGVLSATILYEILLGKATLYAVLVSALVLMAMVKRKDSRG

SEQ ID NO: 490 - protein, 294 aa, synthetic construct
DTAVSQTPKYLVTQMGNDKSIKCEQNLGHDTMYWYKQDSKKFLKIMFSYNNKELIINETVPNRFSPKSPDKAHLNLHINSLELGDSAVYFCASSPWTSGGNGELFFGEGSRLTVLEDLKNVFPPEVAVFEPSEAEISHTQKATLVCLATGFYPDHVELSWWVNGKEVHSGVSTDPQPLKEQPALNDSRYCLSSRLRVSATFWQNPRNHFRCQVQFYGLSENDEWTQDRAKPVTQIVSAEAWGRADCGFTSESYQQGVLSATILYEILLGKATLYAVLVSALVLMAMVKRKDSRG

SEQ ID NO: 491 - protein, 291 aa, synthetic construct
DTAVSQTPKYLVTQMGNDKSIKCEQNLGHDTMYWYKQDSKKFLKIMFSYNNKELIINETVPNRFSPKSPDKAHLNLHINSLELGDSAVYFCASSPGLAYEQYFGPGTRLTVTEDLKNVFPPEVAVFEPSEAEISHTQKATLVCLATGFYPDHVELSWWVNGKEVHSGVSTDPQPLKEQPALNDSRYCLSSRLRVSATFWQNPRNHFRCQVQFYGLSENDEWTQDRAKPVTQIVSAEAWGRADCGFTSESYQQGVLSATILYEILLGKATLYAVLVSALVLMAMVKRKDSRG

SEQ ID NO: 492 - protein, 291 aa, synthetic construct
EAQVTQNPRYLITVTGKKLTVTCSQNMNHEYMSWYRQDPGLGLRQIYYSMNVEVTDKGDVPEGYKVSRKEKRNFPLILESPSPNQTSLYFCASSAGTGGFVGYTFGSGTRLTVVEDLNKVFPPEVAVFEPSEAEISHTQKATLVCLATGFFPDHVELSWWVNGKEVHSGVSTDPQPLKEQPALNDSRYCLSSRLRVSATFWQNPRNHFRCQVQFYGLSENDEWTQDRAKPVTQIVSAEAWGRADCGFTSVSYQQGVLSATILYEILLGKATLYAVLVSALVLMAMVKRKDF

SEQ ID NO: 493 - protein, 296 aa, synthetic construct
SAVISQKPSRDICQRGTSLTIQCQVDSQVTMMFWYRQQPGQSLTLIATANQGSEATYESGFVIDKFPISRPNLTFSTLTVSNMSPEDSSIYLCSVWGAGLAIYNEQFFGPGTRLTVLEDLKNVFPPEVAVFEPSEAEISHTQKATLVCLATGFYPDHVELSWWVNGKEVHSGVSTDPQPLKEQPALNDSRYCLSSRLRVSATFWQNPRNHFRCQVQFYGLSENDEWTQDRAKPVTQIVSAEAWGRADCGFTSESYQQGVLSATILYEILLGKATLYAVLVSALVLMAMVKRKDSRG

SEQ ID NO: 494 - protein, 293 aa, synthetic construct
DVKVTQSSRYLVKRTGEKVFLECVQDMDHENMFWYRQDPGLGLRLIYFSYDVKMKEKGDIPEGYSVSREKKERFSLILESASTNQTSMYLCASSSATSGSGEQYFGPGTRLTVTEDLKNVFPPEVAVFEPSEAEISHTQKATLVCLATGFYPDHVELSWWVNGKEVHSGVSTDPQPLKEQPALNDSRYCLSSRLRVSATFWQNPRNHFRCQVQFYGLSENDEWTQDRAKPVTQIVSAEAWGRADCGFTSESYQQGVLSATILYEILLGKATLYAVLVSALVLMAMVKRKDSRG

SEQ ID NO: 495 - protein, 294 aa, synthetic construct
EAQVTQNPRYLITVTGKKLTVTCSQNMNHEYMSWYRQDPGLGLRQIYYSMNVEVTDKGDVPEGYKVSRKEKRNFPLILESPSPNQTSLYFCASSIDSGSSYNEQFFGPGTRLTVLEDLKNVFPPEVAVFEPSEAEISHTQKATLVCLATGFYPDHVELSWWVNGKEVHSGVSTDPQPLKEQPALNDSRYCLSSRLRVSATFWQNPRNHFRCQVQFYGLSENDEWTQDRAKPVTQIVSAEAWGRADCGFTSESYQQGVLSATILYEILLGKATLYAVLVSALVLMAMVKRKDSRG

SEQ ID NO: 496 - protein, 291 aa, synthetic construct
EPEVTQTPSHQVTQMGQEVILRCVPISNHLYFYWYRQILGQKVEFLVSFYNNEISEKSEIFDDQFSVERPDGSNFTLKIRSTKLEDSAMYFCASSEGWGGTEAFFGQGTRLTVVEDLNKVFPPEVAVFEPSEAEISHTQKATLVCLATGFFPDHVELSWWVNGKEVHSGVSTDPQPLKEQPALNDSRYCLSSRLRVSATFWQNPRNHFRCQVQFYGLSENDEWTQDRAKPVTQIVSAEAWGRADCGFTSVSYQQGVLSATILYEILLGKATLYAVLVSALVLMAMVKRKDF

SEQ ID NO: 497 - DNA, 867 bp, synthetic construct
  source 1..867: mol_type = other DNA
gatgctgatgttacccagaccccaaggaataggatcacaaagacaggaaagaggattatgctggaatgttctcagactaagggtcatgatagaatgtactggtatcgacaagacccaggactgggcctacggttgatctattactcctttgatgtcaaagatataaacaaaggagagatctctgatggatacagtgtctctcgacaggcacaggctaaattctccctgtccctagagtctgccatccccaaccagacagctctttacttctgtgccaccagtgatttactaggccgggcccagcattttggtgatgggactcgactctccatcctagaggacctgaacaaggtgttcccacccgaggtcgctgtgtttgagccatcagaagcagagatctcccacacccaaaaggccacactggtgtgcctggccacaggcttcttccctgaccacgtggagctgagctggtgggtgaatgggaaggaggtgcacagtggggtcagcacggacccgcagcccctcaaggagcagcccgccctcaatgactccagatactgcctgtcctcccgcctgagggtctcggccaccttctggcagaacccccgcaaccacttccgctgtcaagtccagttctacgggctctcggagaatgacgagtggacccaggatagggccaaacccgtcacccagatcgtcagcgccgaggcctggggtagagcagactgtggctttacctcggtgtcctaccagcaaggggtcctgtctgccaccatcctctatgagatcctgctagggaaggccaccctgtatgctgtgctggtcagcgcccttgtgttgatggccatggtcaagagaaaggatttc

SEQ ID NO: 498 - DNA, 876 bp, synthetic construct
  source 1..876: mol_type = other DNA
gatgctgatgttacccagaccccaaggaataggatcacaaagacaggaaagaggattatgctggaatgttctcagactaagggtcatgatagaatgtactggtatcgacaagacccaggactgggcctacggttgatctattactcctttgatgtcaaagatataaacaaaggagagatctctgatggatacagtgtctctcgacaggcacaggctaaattctccctgtccctagagtctgccatccccaaccagacagctctttacttctgtgccaccagtgattcccgagggggggtcgagcagtacttcgggccgggcaccaggctcacggtcacagaggacctgaaaaacgtgttcccacccgaggtcgctgtgtttgagccatcagaagcagagatctcccacacccaaaaggccacactggtgtgcctggccacaggcttctaccccgaccacgtggagctgagctggtgggtgaatgggaaggaggtgcacagtggggtcagcacagacccgcagcccctcaaggagcagcccgccctcaatgactccagatactgcctgtcctcccgcctgagggtctcggccaccttctggcagaacccccgcaaccacttccgctgtcaagtccagttctacgggctctcggagaatgacgagtggacccaggatagggccaaacctgtcacccagatcgtcagcgccgaggcctggggtagagcagactgtggcttcacctccgagtcttaccagcaaggggtcctgtctgccaccatcctctatgagatcttgctagggaaggccaccttgtatgccgtgctggtcagtgccctcgtgctgatggccatggtcaagagaaaggattccagaggc

SEQ ID NO: 499 - DNA, 882 bp, synthetic construct
  source 1..882: mol_type = other DNA
gacactgaagttacccagacaccaaaacacctggtcatgggaatgacaaataagaagtctttgaaatgtgaacaacatatggggcacagggctatgtattggtacaagcagaaagctaagaagccaccggagctcatgtttgtctacagctatgagaaactctctataaatgaaagtgtgccaagtcgcttctcacctgaatgccccaacagctctctcttaaaccttcacctacacgccctgcagccagaagactcagccctgtatctctgcgccagcagccaagatccgttctggggggccggggagctgttttttggagaaggctctaggctgaccgtactggaggacctgaaaaacgtgttcccacccgaggtcgctgtgtttgagccatcagaagcagagatctcccacacccaaaaggccacactggtgtgcctggccacaggcttctaccccgaccacgtggagctgagctggtgggtgaatgggaaggaggtgcacagtggggtcagcacagacccgcagcccctcaaggagcagcccgccctcaatgactccagatactgcctgtcctcccgcctgagggtctcggccaccttctggcagaacccccgcaaccacttccgctgtcaagtccagttctacgggctctcggagaatgacgagtggacccaggatagggccaaacctgtcacccagatcgtcagcgccgaggcctggggtagagcagactgtggcttcacctccgagtcttaccagcaaggggtcctgtctgccaccatcctctatgagatcttgctagggaaggccaccttgtatgccgtgctggtcagtgccctcgtgctgatggccatggtcaagagaaaggattccagaggc

SEQ ID NO: 500 - DNA, 876 bp, synthetic construct
  source 1..876: mol_type = other DNA
gaagcccaagtgacccagaacccaagatacctcatcacagtgactggaaagaagttaacagtgacttgttctcagaatatgaaccatgagtatatgtcctggtatcgacaagacccagggctgggcttaaggcagatctactattcaatgaatgttgaggtgactgataagggagatgttcctgaagggtacaaagtctctcgaaaagagaagaggaatttccccctgatcctggagtcgcccagccccaaccagacctctctgtacttctgtgccagcagtcccgggactagcggcaatgagcagttcttcgggccagggacacggctcaccgtgctagaggacctgaaaaacgtgttcccacccgaggtcgctgtgtttgagccatcagaagcagagatctcccacacccaaaaggccacactggtgtgcctggccacaggcttctaccccgaccacgtggagctgagctggtgggtgaatgggaaggaggtgcacagtggggtcagcacagacccgcagcccctcaaggagcagcccgccctcaatgactccagatactgcctgtcctcccgcctgagggtctcggccaccttctggcagaacccccgcaaccacttccgctgtcaagtccagttctacgggctctcggagaatgacgagtggacccaggatagggccaaacctgtcacccagatcgtcagcgccgaggcctggggtagagcagactgtggcttcacctccgagtcttaccagcaaggggtcctgtctgccaccatcctctatgagatcttgctagggaaggccaccttgtatgccgtgctggtcagtgccctcgtgctgatggccatggtcaagagaaaggattccagaggc

SEQ ID NO: 501 - DNA, 873 bp, synthetic construct
  source 1..873: mol_type = other DNA
ggtgctgtcgtctctcaacatccgagcagggttatctgtaagagtggaacctctgtgaagatcgagtgccgttccctggactttcaggccacaactatgttttggtatcgtcagttcccgaaacagagtctcatgctgatggcaacttccaatgagggctccaaggccacatacgagcaaggcgtcgagaaggacaagtttctcatcaaccatgcaagcctgaccttgtccactctgacagtgaccagtgcccatcctgaagacagcagcttctacatctgcagtgctacagaagataatgaaaaactgttttttggcagtggaacccagctctctgtcttggaggacctgaacaaggtgttcccacccgaggtcgctgtgtttgagccatcagaagcagagatctcccacacccaaaaggccacactggtgtgcctggccacaggcttcttccctgaccacgtggagctgagctggtgggtgaatgggaaggaggtgcacagtggggtcagcacggacccgcagcccctcaaggagcagcccgccctcaatgactccagatactgcctgtcctcccgcctgagggtctcggccaccttctggcagaacccccgcaaccacttccgctgtcaagtccagttctacgggctctcggagaatgacgagtggacccaggatagggccaaacccgtcacccagatcgtcagcgccgaggcctggggtagagcagactgtggctttacctcggtgtcctaccagcaaggggtcctgtctgccaccatcctctatgagatcctgctagggaaggccaccctgtatgctgtgctggtcagcgcccttgtgttgatggccatggtcaagagaaaggatttc

SEQ ID NO: 502 - DNA, 879 bp, synthetic construct
  source 1..879: mol_type = other DNA
aaggctggagtcactcaaactccaagatatctgatcaaaacgagaggacagcaagtgacactgagctgctcccctatctctgggcataggagtgtatcctggtaccaacagaccccaggacagggccttcagttcctctttgaatacttcagtgagacacagagaaacaaaggaaacttccctggtcgattctcagggcgccagttctctaactctcgctctgagatgaatgtgagcaccttggagctgggggactcggccctttatctttgcgccagcagcttggaggcagggtcattctacgagcagtacttcgggccgggcaccaggctcacggtcacagaggacctgaaaaacgtgttcccacccgaggtcgctgtgtttgagccatcagaagcagagatctcccacacccaaaaggccacactggtgtgcctggccacaggcttctaccccgaccacgtggagctgagctggtgggtgaatgggaaggaggtgcacagtggggtcagcacagacccgcagcccctcaaggagcagcccgccctcaatgactccagatactgcctgtcctcccgcctgagggtctcggccaccttctggcagaacccccgcaaccacttccgctgtcaagtccagttctacgggctctcggagaatgacgagtggacccaggatagggccaaacctgtcacccagatcgtcagcgccgaggcctggggtagagcagactgtggcttcacctccgagtcttaccagcaaggggtcctgtctgccaccatcctctatgagatcttgctagggaaggccaccttgtatgccgtgctggtcagtgccctcgtgctgatggccatggtcaagagaaaggattccagaggc

SEQ ID NO: 503 - DNA, 870 bp, synthetic construct
  source 1..870: mol_type = other DNA
gacacagctgtttcccagactccaaaatacctggtcacacagatgggaaacgacaagtccattaaatgtgaacaaaatctgggccatgatactatgtattggtataaacaggactctaagaaatttctgaagataatgtttagctacaataataaggagctcattataaatgaaacagttccaaatcgcttctcacctaaatctccagacaaagctcacttaaatcttcacatcaattccctggagcttggtgactctgctgtgtatttctgtgccagcagccaaggcatctctggaaacaccatatattttggagagggaagttggctcactgttgtagaggacctgaacaaggtgttcccacccgaggtcgctgtgtttgagccatcagaagcagagatctcccacacccaaaaggccacactggtgtgcctggccacaggcttcttccctgaccacgtggagctgagctggtgggtgaatgggaaggaggtgcacagtggggtcagcacggacccgcagcccctcaaggagcagcccgccctcaatgactccagatactgcctgtcctcccgcctgagggtctcggccaccttctggcagaacccccgcaaccacttccgctgtcaagtccagttctacgggctctcggagaatgacgagtggacccaggatagggccaaacccgtcacccagatcgtcagcgccgaggcctggggtagagcagactgtggctttacctcggtgtcctaccagcaaggggtcctgtctgccaccatcctctatgagatcctgctagggaaggccaccctgtatgctgtgctggtcagcgcccttgtgttgatggccatggtcaagagaaaggatttc

SEQ ID NO: 504 - DNA, 879 bp, synthetic construct
  source 1..879: mol_type = other DNA
gattctggagtcacacaaaccccaaagcacctgatcacagcaactggacagcgagtgacgctgagatgctcccctaggtctggagacctctctgtgtactggtaccaacagagcctggaccagggcctccagttcctcattcagtattataatggagaagagagagcaaaaggaaacattcttgaacgattctccgcacaacagttccctgacttgcactctgaactaaacctgagctctctggagctgggggactcagctttgtatttctgtgccagcagcccttggactagcgggagctacgagcagtacttcgggccgggcaccaggctcacggtcacagaggacctgaaaaacgtgttcccacccgaggtcgctgtgtttgagccatcagaagcagagatctcccacacccaaaaggccacactggtgtgcctggccacaggcttctaccccgaccacgtggagctgagctggtgggtgaatgggaaggaggtgcacagtggggtcagcacagacccgcagcccctcaaggagcagcccgccctcaatgactccagatactgcctgtcctcccgcctgagggtctcggccaccttctggcagaacccccgcaaccacttccgctgtcaagtccagttctacgggctctcggagaatgacgagtggacccaggatagggccaaacctgtcacccagatcgtcagcgccgaggcctggggtagagcagactgtggcttcacctccgagtcttaccagcaaggggtcctgtctgccaccatcctctatgagatcttgctagggaaggccaccttgtatgccgtgctggtcagtgccctcgtgctgatggccatggtcaagagaaaggattccagaggc

SEQ ID NO: 505 - DNA, 879 bp, synthetic construct
  source 1..879: mol_type = other DNA
gaagcccaagtgacccagaacccaagatacctcatcacagtgactggaaagaagttaacagtgacttgttctcagaatatgaaccatgagtatatgtcctggtatcgacaagacccagggctgggcttaaggcagatctactattcaatgaatgttgaggtgactgataagggagatgttcctgaagggtacaaagtctctcgaaaagagaagaggaatttccccctgatcctggagtcgcccagccccaaccagacctctctgtacttctgtgccactcaatgggctagcgggagcacagatacgcagtattttggcccaggcacccggctgacagtgctcgaggacctgaaaaacgtgttcccacccgaggtcgctgtgtttgagccatcagaagcagagatctcccacacccaaaaggccacactggtgtgcctggccacaggcttctaccccgaccacgtggagctgagctggtgggtgaatgggaaggaggtgcacagtggggtcagcacagacccgcagcccctcaaggagcagcccgccctcaatgactccagatactgcctgtcctcccgcctgagggtctcggccaccttctggcagaacccccgcaaccacttccgctgtcaagtccagttctacgggctctcggagaatgacgagtggacccaggatagggccaaacctgtcacccagatcgtcagcgccgaggcctggggtagagcagactgtggcttcacctccgagtcttaccagcaaggggtcctgtctgccaccatcctctatgagatcttgctagggaaggccaccttgtatgccgtgctggtcagtgccctcgtgctgatggccatggtcaagagaaaggattccagaggc

SEQ ID NO: 506 - DNA, 873 bp, synthetic construct
  source 1..873: mol_type = other DNA
gaagcccaagtgacccagaacccaagatacctcatcacagtgactggaaagaagttaacagtgacttgttctcagaatatgaaccatgagtatatgtcctggtatcgacaagacccagggctgggcttaaggcagatctactattcaatgaatgttgaggtgactgataagggagatgttcctgaagggtacaaagtctctcgaaaagagaagaggaatttccccctgatcctggagtcgcccagccccaaccagacctctctgtacttctgtgccagcagttccgggactagcgacgagcagtacttcgggccgggcaccaggctcacggtcacagaggacctgaaaaacgtgttcccacccgaggtcgctgtgtttgagccatcagaagcagagatctcccacacccaaaaggccacactggtgtgcctggccacaggcttctaccccgaccacgtggagctgagctggtgggtgaatgggaaggaggtgcacagtggggtcagcacagacccgcagcccctcaaggagcagcccgccctcaatgactccagatactgcctgtcctcccgcctgagggtctcggccaccttctggcagaacccccgcaaccacttccgctgtcaagtccagttctacgggctctcggagaatgacgagtggacccaggatagggccaaacctgtcacccagatcgtcagcgccgaggcctggggtagagcagactgtggcttcacctccgagtcttaccagcaaggggtcctgtctgccaccatcctctatgagatcttgctagggaaggccaccttgtatgccgtgctggtcagtgccctcgtgctgatggccatggtcaagagaaaggattccagaggc

SEQ ID NO: 507 - DNA, 873 bp, synthetic construct
  source 1..873: mol_type = other DNA
gaacctgaagtcacccagactcccagccatcaggtcacacagatgggacaggaagtgatcttgcgctgtgtccccatctctaatcacttatacttctattggtacagacaaatcttggggcagaaagtcgagtttctggtttccttttataataatgaaatctcagagaagtctgaaatattcgatgatcaattctcagttgaaaggcctgatggatcaaatttcactctgaagatccggtccacaaagctggaggactcagccatgtacttctgtgccagcagggaggacggatacgagcagtacttcgggccgggcaccaggctcacggtcacagaggacctgaaaaacgtgttcccacccgaggtcgctgtgtttgagccatcagaagcagagatctcccacacccaaaaggccacactggtgtgcctggccacaggcttctaccccgaccacgtggagctgagctggtgggtgaatgggaaggaggtgcacagtggggtcagcacagacccgcagcccctcaaggagcagcccgccctcaatgactccagatactgcctgtcctcccgcctgagggtctcggccaccttctggcagaacccccgcaaccacttccgctgtcaagtccagttctacgggctctcggagaatgacgagtggacccaggatagggccaaacctgtcacccagatcgtcagcgccgaggcctggggtagagcagactgtggcttcacctccgagtcttaccagcaaggggtcctgtctgccaccatcctctatgagatcttgctagggaaggccaccttgtatgccgtgctggtcagtgccctcgtgctgatggccatggtcaagagaaaggattccagaggc

SEQ ID NO: 508 - DNA, 873 bp, synthetic construct
  source 1..873: mol_type = other DNA
gaagcccaagtgacccagaacccaagatacctcatcacagtgactggaaagaagttaacagtgacttgttctcagaatatgaaccatgagtatatgtcctggtatcgacaagacccagggctgggcttaaggcagatctactattcaatgaatgttgaggtgactgataagggagatgttcctgaagggtacaaagtctctcgaaaagagaagaggaatttccccctgatcctggagtcgcccagccccaaccagacctctctgtacttctgtgccacctcacccgggaccctatacgagcagtacttcgggccgggcaccaggctcacggtcacagaggacctgaaaaacgtgttcccacccgaggtcgctgtgtttgagccatcagaagcagagatctcccacacccaaaaggccacactggtgtgcctggccacaggcttctaccccgaccacgtggagctgagctggtgggtgaatgggaaggaggtgcacagtggggtcagcacagacccgcagcccctcaaggagcagcccgccctcaatgactccagatactgcctgtcctcccgcctgagggtctcggccaccttctggcagaacccccgcaaccacttccgctgtcaagtccagttctacgggctctcggagaatgacgagtggacccaggatagggccaaacctgtcacccagatcgtcagcgccgaggcctggggtagagcagactgtggcttcacctccgagtcttaccagcaaggggtcctgtctgccaccatcctctatgagatcttgctagggaaggccaccttgtatgccgtgctggtcagtgccctcgtgctgatggccatggtcaagagaaaggattccagaggc

SEQ ID NO: 509 - DNA, 879 bp, synthetic construct
  source 1..879: mol_type = other DNA
gattctggagtcacacaaaccccaaagcacctgatcacagcaactggacagcgagtgacgctgagatgctcccctaggtctggagacctctctgtgtactggtaccaacagagcctggaccagggcctccagttcctcattcagtattataatggagaagagagagcaaaaggaaacattcttgaacgattctccgcacaacagttccctgacttgcactctgaactaaacctgagctctctggagctgggggactcagctttgtatttctgtgccagcagcccgtggctacagggtggcaatgagcagttcttcgggccagggacacggctcaccgtgctagaggacctgaaaaacgtgttcccacccgaggtcgctgtgtttgagccatcagaagcagagatctcccacacccaaaaggccacactggtgtgcctggccacaggcttctaccccgaccacgtggagctgagctggtgggtgaatgggaaggaggtgcacagtggggtcagcacagacccgcagcccctcaaggagcagcccgccctcaatgactccagatactgcctgtcctcccgcctgagggtctcggccaccttctggcagaacccccgcaaccacttccgctgtcaagtccagttctacgggctctcggagaatgacgagtggacccaggatagggccaaacctgtcacccagatcgtcagcgccgaggcctggggtagagcagactgtggcttcacctccgagtcttaccagcaaggggtcctgtctgccaccatcctctatgagatcttgctagggaaggccaccttgtatgccgtgctggtcagtgccctcgtgctgatggccatggtcaagagaaaggattccagaggc

SEQ ID NO: 510 - DNA, 882 bp, synthetic construct
  source 1..882: mol_type = other DNA
gatgctggagttatccagtcaccccgccatgaggtgacagagatgggacaagaagtgactctgagatgtaaaccaatttcaggccacaactcccttttctggtacagacagaccatgatgcggggactggagttgctcatttactttaacaacaacgttccgatagatgattcagggatgcccgaggatcgattctcagctaagatgcctaatgcatcattctccactctgaagatccagccctcagaacccagggactcagctgtgtacttctgtgccagcagtatcgccgccctaggattcggggagctgttttttggagaaggctctaggctgaccgtactggaggacctgaaaaacgtgttcccacccgaggtcgctgtgtttgagccatcagaagcagagatctcccacacccaaaaggccacactggtgtgcctggccacaggcttctaccccgaccacgtggagctgagctggtgggtgaatgggaaggaggtgcacagtggggtcagcacagacccgcagcccctcaaggagcagcccgccctcaatgactccagatactgcctgtcctcccgcctgagggtctcggccaccttctggcagaacccccgcaaccacttccgctgtcaagtccagttctacgggctctcggagaatgacgagtggacccaggatagggccaaacctgtcacccagatcgtcagcgccgaggcctggggtagagcagactgtggcttcacctccgagtcttaccagcaaggggtcctgtctgccaccatcctctatgagatcttgctagggaaggccaccttgtatgccgtgctggtcagtgccctcgtgctgatggccatggtcaagagaaaggattccagaggc

SEQ ID NO: 511 - DNA, 879 bp, synthetic construct
  source 1..879: mol_type = other DNA
gattctggagtcacacaaaccccaaagcacctgatcacagcaactggacagcgagtgacgctgagatgctcccctaggtctggagacctctctgtgtactggtaccaacagagcctggaccagggcctccagttcctcattcagtattataatggagaagagagagcaaaaggaaacattcttgaacgattctccgcacaacagttccctgacttgcactctgaactaaacctgagctctctggagctgggggactcagctttgtatttctgtgccagcagcgtatggtctagcgggggaaatgagcagttcttcgggccagggacacggctcaccgtgctagaggacctgaaaaacgtgttcccacccgaggtcgctgtgtttgagccatcagaagcagagatctcccacacccaaaaggccacactggtgtgcctggccacaggcttctaccccgaccacgtggagctgagctggtgggtgaatgggaaggaggtgcacagtggggtcagcacagacccgcagcccctcaaggagcagcccgccctcaatgactccagatactgcctgtcctcccgcctgagggtctcggccaccttctggcagaacccccgcaaccacttccgctgtcaagtccagttctacgggctctcggagaatgacgagtggacccaggatagggccaaacctgtcacccagatcgtcagcgccgaggcctggggtagagcagactgtggcttcacctccgagtcttaccagcaaggggtcctgtctgccaccatcctctatgagatcttgctagggaaggccaccttgtatgccgtgctggtcagtgccctcgtgctgatggccatggtcaagagaaaggattccagaggc

SEQ ID NO: 512 - DNA, 876 bp, synthetic construct
  source 1..876: mol_type = other DNA
gaagcccaagtgacccagaacccaagatacctcatcacagtgactggaaagaagttaacagtgacttgttctcagaatatgaaccatgagtatatgtcctggtatcgacaagacccagggctgggcttaaggcagatctactattcaatgaatgttgaggtgactgataagggagatgttcctgaagggtacaaagtctctcgaaaagagaagaggaatttccccctgatcctggagtcgcccagccccaaccagacctctctgtacttctgtgccagcagcccctcatcaggctacaatgagcagttcttcgggccagggacacggctcaccgtgctagaggacctgaaaaacgtgttcccacccgaggtcgctgtgtttgagccatcagaagcagagatctcccacacccaaaaggccacactggtgtgcctggccacaggcttctaccccgaccacgtggagctgagctggtgggtgaatgggaaggaggtgcacagtggggtcagcacagacccgcagcccctcaaggagcagcccgccctcaatgactccagatactgcctgtcctcccgcctgagggtctcggccaccttctggcagaacccccgcaaccacttccgctgtcaagtccagttctacgggctctcggagaatgacgagtggacccaggatagggccaaacctgtcacccagatcgtcagcgccgaggcctggggtagagcagactgtggcttcacctccgagtcttaccagcaaggggtcctgtctgccaccatcctctatgagatcttgctagggaaggccaccttgtatgccgtgctggtcagtgccctcgtgctgatggccatggtcaagagaaaggattccagaggc

SEQ ID NO: 513 - DNA, 879 bp, synthetic construct
  source 1..879: mol_type = other DNA
gattctggagtcacacaaaccccaaagcacctgatcacagcaactggacagcgagtgacgctgagatgctcccctaggtctggagacctctctgtgtactggtaccaacagagcctggaccagggcctccagttcctcattcagtattataatggagaagagagagcaaaaggaaacattcttgaacgattctccgcacaacagttccctgacttgcactctgaactaaacctgagctctctggagctgggggactcagctttgtatttctgtgccagcagcccatggttagcgggagggcgggagcagtacttcgggccgggcaccaggctcacggtcacagaggacctgaaaaacgtgttcccacccgaggtcgctgtgtttgagccatcagaagcagagatctcccacacccaaaaggccacactggtgtgcctggccacaggcttctaccccgaccacgtggagctgagctggtgggtgaatgggaaggaggtgcacagtggggtcagcacagacccgcagcccctcaaggagcagcccgccctcaatgactccagatactgcctgtcctcccgcctgagggtctcggccaccttctggcagaacccccgcaaccacttccgctgtcaagtccagttctacgggctctcggagaatgacgagtggacccaggatagggccaaacctgtcacccagatcgtcagcgccgaggcctggggtagagcagactgtggcttcacctccgagtcttaccagcaaggggtcctgtctgccaccatcctctatgagatcttgctagggaaggccaccttgtatgccgtgctggtcagtgccctcgtgctgatggccatggtcaagagaaaggattccagaggc

SEQ ID NO: 514 - DNA, 873 bp, synthetic construct
  source 1..873: mol_type = other DNA
gaagcccaagtgacccagaacccaagatacctcatcacagtgactggaaagaagttaacagtgacttgttctcagaatatgaaccatgagtatatgtcctggtatcgacaagacccagggctgggcttaaggcagatctactattcaatgaatgttgaggtgactgataagggagatgttcctgaagggtacaaagtctctcgaaaagagaagaggaatttccccctgatcctggagtcgcccagccccaaccagacctctctgtacttctgtgccagtcgttgggggctcggcggggagctgttttttggagaaggctctaggctgaccgtactggaggacctgaaaaacgtgttcccacccgaggtcgctgtgtttgagccatcagaagcagagatctcccacacccaaaaggccacactggtgtgcctggccacaggcttctaccccgaccacgtggagctgagctggtgggtgaatgggaaggaggtgcacagtggggtcagcacagacccgcagcccctcaaggagcagcccgccctcaatgactccagatactgcctgtcctcccgcctgagggtctcggccaccttctggcagaacccccgcaaccacttccgctgtcaagtccagttctacgggctctcggagaatgacgagtggacccaggatagggccaaacctgtcacccagatcgtcagcgccgaggcctggggtagagcagactgtggcttcacctccgagtcttaccagcaaggggtcctgtctgccaccatcctctatgagatcttgctagggaaggccaccttgtatgccgtgctggtcagtgccctcgtgctgatggccatggtcaagagaaaggattccagaggc

SEQ ID NO: 515 - DNA, 870 bp, synthetic construct
  source 1..870: mol_type = other DNA
gacgctggagtcacccaaagtcccacacacctgatcaaaacgagaggacagcaagtgactctgagatgctctcctaagtctgggcatgacactgtgtcctggtaccaacaggccctgggtcaggggccccagtttatctttcagtattatgaggaggaagagagacagagaggcaacttccctgatcgattctcaggtcaccagttccctaactatagctctgagctgaatgtgaacgccttgttgctgggggactcggccctctatctctgtgccagcagcttggtggactacgagcagtacttcgggccgggcaccaggctcacggtcacagaggacctgaaaaacgtgttcccacccgaggtcgctgtgtttgagccatcagaagcagagatctcccacacccaaaaggccacactggtgtgcctggccacaggcttctaccccgaccacgtggagctgagctggtgggtgaatgggaaggaggtgcacagtggggtcagcacagacccgcagcccctcaaggagcagcccgccctcaatgactccagatactgcctgtcctcccgcctgagggtctcggccaccttctggcagaacccccgcaaccacttccgctgtcaagtccagttctacgggctctcggagaatgacgagtggacccaggatagggccaaacctgtcacccagatcgtcagcgccgaggcctggggtagagcagactgtggcttcacctccgagtcttaccagcaaggggtcctgtctgccaccatcctctatgagatcttgctagggaaggccaccttgtatgccgtgctggtcagtgccctcgtgctgatggccatggtcaagagaaaggattccagaggc

SEQ ID NO: 516 - DNA, 873 bp, synthetic construct
  source 1..873: mol_type = other DNA
gatggtggaatcactcagtccccaaagtacctgttcagaaaggaaggacagaatgtgaccctgagttgtgaacagaatttgaaccacgatgccatgtactggtaccgacaggacccagggcaagggctgagattgatctactactcacagatagtaaatgactttcagaaaggagatatagctgaagggtacagcgtctctcgggagaagaaggaatcctttcctctcactgtgacatcggcccaaaagaacccgacagctttctatctctgtgccagcctcggactaaattacaatgagcagttcttcgggccagggacacggctcaccgtgctagaggacctgaaaaacgtgttcccacccgaggtcgctgtgtttgagccatcagaagcagagatctcccacacccaaaaggccacactggtgtgcctggccacaggcttctaccccgaccacgtggagctgagctggtgggtgaatgggaaggaggtgcacagtggggtcagcacagacccgcagcccctcaaggagcagcccgccctcaatgactccagatactgcctgtcctcccgcctgagggtctcggccaccttctggcagaacccccgcaaccacttccgctgtcaagtccagttctacgggctctcggagaatgacgagtggacccaggatagggccaaacctgtcacccagatcgtcagcgccgaggcctggggtagagcagactgtggcttcacctccgagtcttaccagcaaggggtcctgtctgccaccatcctctatgagatcttgctagggaaggccaccttgtatgccgtgctggtcagtgccctcgtgctgatggccatggtcaagagaaaggattccagaggc

SEQ ID NO: 517 - DNA, 873 bp, synthetic construct
  source 1..873: mol_type = other DNA
gaagcccaagtgacccagaacccaagatacctcatcacagtgactggaaagaagttaacagtgacttgttctcagaatatgaaccatgagtatatgtcctggtatcgacaagacccagggctgggcttaaggcagatctactattcaatgaatgttgaggtgactgataagggagatgttcctgaagggtacaaagtctctcgaaaagagaagaggaatttccccctgatcctggagtcgcccagccccaaccagacctctctgtacttctgtgccagcagaatctccttaggagctaactatggctacaccttcggttcggggaccaggttaaccgttgtagaggacctgaacaaggtgttcccacccgaggtcgctgtgtttgagccatcagaagcagagatctcccacacccaaaaggccacactggtgtgcctggccacaggcttcttccctgaccacgtggagctgagctggtgggtgaatgggaaggaggtgcacagtggggtcagcacggacccgcagcccctcaaggagcagcccgccctcaatgactccagatactgcctgtcctcccgcctgagggtctcggccaccttctggcagaacccccgcaaccacttccgctgtcaagtccagttctacgggctctcggagaatgacgagtggacccaggatagggccaaacccgtcacccagatcgtcagcgccgaggcctggggtagagcagactgtggctttacctcggtgtcctaccagcaaggggtcctgtctgccaccatcctctatgagatcctgctagggaaggccaccctgtatgctgtgctggtcagcgcccttgtgttgatggccatggtcaagagaaaggatttc

SEQ ID NO: 518 - DNA, 885 bp, synthetic construct
  source 1..885: mol_type = other DNA
ggtgctgtcgtctctcaacatccgagctgggttatctgcaagagtggaacctctgtgaagatcgagtgccgttccctggactttcaggccacaactatgttttggtatcgtcagttcccgaaacagagtctcatgctgatggcaacttccaatgagggctccaaggccacatacgagcaaggcgtcgagaaggacaagtttctcatcaaccatgcaagcctgaccttgtccactctgacagtgaccagtgcccatcctgaagacagcagcttctacatctgcagtgctactagggacagctcctacaatgagcagttcttcgggccagggacacggctcaccgtgctagaggacctgaaaaacgtgttcccacccgaggtcgctgtgtttgagccatcagaagcagagatctcccacacccaaaaggccacactggtgtgcctggccacaggcttctaccccgaccacgtggagctgagctggtgggtgaatgggaaggaggtgcacagtggggtcagcacagacccgcagcccctcaaggagcagcccgccctcaatgactccagatactgcctgtcctcccgcctgagggtctcggccaccttctggcagaacccccgcaaccacttccgctgtcaagtccagttctacgggctctcggagaatgacgagtggacccaggatagggccaaacctgtcacccagatcgtcagcgccgaggcctggggtagagcagactgtggcttcacctccgagtcttaccagcaaggggtcctgtctgccaccatcctctatgagatcttgctagggaaggccaccttgtatgccgtgctggtcagtgccctcgtgctgatggccatggtcaagagaaaggattccagaggc

SEQ ID NO: 519 - DNA, 873 bp, synthetic construct
  source 1..873: mol_type = other DNA
gattctggagtcacacaaaccccaaagcacctgatcacagcaactggacagcgagtgacgctgagatgctcccctaggtctggagacctctctgtgtactggtaccaacagagcctggaccagggcctccagttcctcattcagtattataatggagaagagagagcaaaaggaaacattcttgaacgattctccgcacaacagttccctgacttgcactctgaactaaacctgagctctctggagctgggggactcagctttgtatttctgtgccagcagcccttggacagcagggggaaacaccatatattttggagagggaagttggctcactgtcgtagaggacctgaacaaggtgttcccacccgaggtcgctgtgtttgagccatcagaagcagagatctcccacacccaaaaggccacactggtgtgcctggccacaggcttcttccctgaccacgtggagctgagctggtgggtgaatgggaaggaggtgcacagtggggtcagcacggacccgcagcccctcaaggagcagcccgccctcaatgactccagatactgcctgtcctcccgcctgagggtctcggccaccttctggcagaacccccgcaaccacttccgctgtcaagtccagttctacgggctctcggagaatgacgagtggacccaggatagggccaaacccgtcacccagatcgtcagcgccgaggcctggggtagagcagactgtggctttacctcggtgtcctaccagcaaggggtcctgtctgccaccatcctctatgagatcctgctagggaaggccaccctgtatgctgtgctggtcagcgcccttgtgttgatggccatggtcaagagaaaggatttc

SEQ ID NO: 520 - DNA, 873 bp, synthetic construct
  source 1..873: mol_type = other DNA
gaagcccaagtgacccagaacccaagatacctcatcacagtgactggaaagaagttaacagtgacttgttctcagaatatgaaccatgagtatatgtcctggtatcgacaagacccagggctgggcttaaggcagatctactattcaatgaatgttgaggtgactgataagggagatgttcctgaagggtacaaagtctctcgaaaagagaagaggaatttccccctgatcctggagtcgcccagccccaaccagacctctctgtacttctgtgccagcagttggggttcggggtacgagcagtacttcgggccgggcaccaggctcacggtcacagaggacctgaaaaacgtgttcccacccgaggtcgctgtgtttgagccatcagaagcagagatctcccacacccaaaaggccacactggtgtgcctggccacaggcttctaccccgaccacgtggagctgagctggtgggtgaatgggaaggaggtgcacagtggggtcagcacagacccgcagcccctcaaggagcagcccgccctcaatgactccagatactgcctgtcctcccgcctgagggtctcggccaccttctggcagaacccccgcaaccacttccgctgtcaagtccagttctacgggctctcggagaatgacgagtggacccaggatagggccaaacctgtcacccagatcgtcagcgccgaggcctggggtagagcagactgtggcttcacctccgagtcttaccagcaaggggtcctgtctgccaccatcctctatgagatcttgctagggaaggccaccttgtatgccgtgctggtcagtgccctcgtgctgatggccatggtcaagagaaaggattccagaggc

SEQ ID NO: 521 - DNA, 876 bp, synthetic construct
  source 1..876: mol_type = other DNA
gaagcccaagtgacccagaacccaagatacctcatcacagtgactggaaagaagttaacagtgacttgttctcagaatatgaaccatgagtatatgtcctggtatcgacaagacccagggctgggcttaaggcagatctactattcaatgaatgttgaggtgactgataagggagatgttcctgaagggtacaaagtctctcgaaaagagaagaggaatttccccctgatcctggagtcgcccagccccaaccagacctctctgtacttctgtgccagcagtttagggacaggttttggggagctgttttttggagaaggctctaggctgaccgtactggaggacctgaaaaacgtgttcccacccgaggtcgctgtgtttgagccatcagaagcagagatctcccacacccaaaaggccacactggtgtgcctggccacaggcttctaccccgaccacgtggagctgagctggtgggtgaatgggaaggaggtgcacagtggggtcagcacagacccgcagcccctcaaggagcagcccgccctcaatgactccagatactgcctgtcctcccgcctgagggtctcggccaccttctggcagaacccccgcaaccacttccgctgtcaagtccagttctacgggctctcggagaatgacgagtggacccaggatagggccaaacctgtcacccagatcgtcagcgccgaggcctggggtagagcagactgtggcttcacctccgagtcttaccagcaaggggtcctgtctgccaccatcctctatgagatcttgctagggaaggccaccttgtatgccgtgctggtcagtgccctcgtgctgatggccatggtcaagagaaaggattccagaggc

SEQ ID NO: 522 - DNA, 873 bp, synthetic construct
  source 1..873: mol_type = other DNA
gaagcccaagtgacccagaacccaagatacctcatcacagtgactggaaagaagttaacagtgacttgttctcagaatatgaaccatgagtatatgtcctggtatcgacaagacccagggctgggcttaaggcagatctactattcaatgaatgttgaggtgactgataagggagatgttcctgaagggtacaaagtctctcgaaaagagaagaggaatttccccctgatcctggagtcgcccagccccaaccagacctctctgtacttctgtgccagcagcccgggaacgatcggggagctgttttttggagaaggctctaggctgaccgtactggaggacctgaaaaacgtgttcccacccgaggtcgctgtgtttgagccatcagaagcagagatctcccacacccaaaaggccacactggtgtgcctggccacaggcttctaccccgaccacgtggagctgagctggtgggtgaatgggaaggaggtgcacagtggggtcagcacagacccgcagcccctcaaggagcagcccgccctcaatgactccagatactgcctgtcctcccgcctgagggtctcggccaccttctggcagaacccccgcaaccacttccgctgtcaagtccagttctacgggctctcggagaatgacgagtggacccaggatagggccaaacctgtcacccagatcgtcagcgccgaggcctggggtagagcagactgtggcttcacctccgagtcttaccagcaaggggtcctgtctgccaccatcctctatgagatcttgctagggaaggccaccttgtatgccgtgctggtcagtgccctcgtgctgatggccatggtcaagagaaaggattccagaggc

SEQ ID NO: 523 - DNA, 867 bp, synthetic construct
  source 1..867: mol_type = other DNA
gctgctggagtcatccagtccccaagacatctgatcaaagaaaagagggaaacagccactctgaaatgctatcctatccctagacacgacactgtctactggtaccagcagggtccaggtcaggacccccagttcctcatttcgttttatgaaaagatgcagagcgataaaggaagcatccctgatcgattctcagctcaacagttcagtgactatcattctgaactgaacatgagctccttggagctgggggactcagccctgtacttctgtgccagcagcctggggcggccagaaaaactgttttttggcagtggaacccagctctctgtcttggaggacctgaacaaggtgttcccacccgaggtcgctgtgtttgagccatcagaagcagagatctcccacacccaaaaggccacactggtgtgcctggccacaggcttcttccctgaccacgtggagctgagctggtgggtgaatgggaaggaggtgcacagtggggtcagcacggacccgcagcccctcaaggagcagcccgccctcaatgactccagatactgcctgtcctcccgcctgagggtctcggccaccttctggcagaacccccgcaaccacttccgctgtcaagtccagttctacgggctctcggagaatgacgagtggacccaggatagggccaaacccgtcacccagatcgtcagcgccgaggcctggggtagagcagactgtggctttacctcggtgtcctaccagcaaggggtcctgtctgccaccatcctctatgagatcctgctagggaaggccaccctgtatgctgtgctggtcagcgcccttgtgttgatggccatggtcaagagaaaggatttc

SEQ ID NO: 524 - DNA, 873 bp, synthetic construct
  source 1..873: mol_type = other DNA
gaagcccaagtgacccagaacccaagatacctcatcacagtgactggaaagaagttaacagtgacttgttctcagaatatgaaccatgagtatatgtcctggtatcgacaagacccagggctgggcttaaggcagatctactattcaatgaatgttgaggtgactgataagggagatgttcctgaagggtacaaagtctctcgaaaagagaagaggaatttccccctgatcctggagtcgcccagccccaaccagacctctctgtacttctgtgccagcagtttttggtcggccggggagctgttttttggagaaggctctaggctgaccgtactggaggacctgaaaaacgtgttcccacccgaggtcgctgtgtttgagccatcagaagcagagatctcccacacccaaaaggccacactggtgtgcctggccacaggcttctaccccgaccacgtggagctgagctggtgggtgaatgggaaggaggtgcacagtggggtcagcacagacccgcagcccctcaaggagcagcccgccctcaatgactccagatactgcctgtcctcccgcctgagggtctcggccaccttctggcagaacccccgcaaccacttccgctgtcaagtccagttctacgggctctcggagaatgacgagtggacccaggatagggccaaacctgtcacccagatcgtcagcgccgaggcctggggtagagcagactgtggcttcacctccgagtcttaccagcaaggggtcctgtctgccaccatcctctatgagatcttgctagggaaggccaccttgtatgccgtgctggtcagtgccctcgtgctgatggccatggtcaagagaaaggattccagaggc

SEQ ID NO: 525 - DNA, 882 bp, synthetic construct
  source 1..882: mol_type = other DNA
gattctggagtcacacaaaccccaaagcacctgatcacagcaactggacagcgagtgacgctgagatgctcccctaggtctggtgacctctctgtgtactggtaccaacagagcctggaccagggcctccagttcctcattcagtattataatggagaagagagagcaaaaggaaacattcttgaacgattctccgcacaacagttccctgacttgcactctgaactaaacctgagctctctggagctgggggactcagctttgtatttctgtgccagcagcccctggactagcgggggagacggggagctgttttttggagaaggctctaggctgaccgtactggaggacctgaaaaacgtgttcccacccgaggtcgctgtgtttgagccatcagaagcagagatctcccacacccaaaaggccacactggtgtgcctggccacaggcttctaccccgaccacgtggagctgagctggtgggtgaatgggaaggaggtgcacagtggggtcagcacagacccgcagcccctcaaggagcagcccgccctcaatgactccagatactgcctgtcctcccgcctgagggtctcggccaccttctggcagaacccccgcaaccacttccgctgtcaagtccagttctacgggctctcggagaatgacgagtggacccaggatagggccaaacctgtcacccagatcgtcagcgccgaggcctggggtagagcagactgtggcttcacctccgagtcttaccagcaaggggtcctgtctgccaccatcctctatgagatcttgctagggaaggccaccttgtatgccgtgctggtcagtgccctcgtgctgatggccatggtcaagagaaaggattccagaggc

SEQ ID NO: 526 - DNA, 870 bp, synthetic construct
  source 1..870: mol_type = other DNA
gaagcccaagtgacccagaacccaagatacctcatcacagtgactggaaagaagttaacagtgacttgttctcagaatatgaaccatgagtatatgtcctggtatcgacaagacccagggctgggcttaaggcagatctactattcaatgaatgttgaggtgactgataagggagatgttcctgaagggtacaaagtctctcgaaaagagaagaggaatttccccctgatcctggagtcgcccagccccaaccagacctctctgtacttctgtgccagcagtcccgggacagggggctatggctacaccttcggttcggggaccaggttaaccgttgtagaggacctgaacaaggtgttcccacccgaggtcgctgtgtttgagccatcagaagcagagatctcccacacccaaaaggccacactggtgtgcctggccacaggcttcttccctgaccacgtggagctgagctggtgggtgaatgggaaggaggtgcacagtggggtcagcacggacccgcagcccctcaaggagcagcccgccctcaatgactccagatactgcctgtcctcccgcctgagggtctcggccaccttctggcagaacccccgcaaccacttccgctgtcaagtccagttctacgggctctcggagaatgacgagtggacccaggatagggccaaacccgtcacccagatcgtcagcgccgaggcctggggtagagcagactgtggctttacctcggtgtcctaccagcaaggggtcctgtctgccaccatcctctatgagatcctgctagggaaggccaccctgtatgctgtgctggtcagcgcccttgtgttgatggccatggtcaagagaaaggatttc

SEQ ID NO: 527 - DNA, 876 bp, synthetic construct
  source 1..876: mol_type = other DNA
gctgctggagtcatccagtccccaagacatctgatcaaagaaaagagggaaacagccactctgaaatgctatcctatccctagacacgacactgtctactggtaccagcagggtccaggtcaggacccccagttcctcatttcgttttatgaaaagatgcagagcgataaaggaagcatccctgatcgattctcagctcaacagttcagtgactatcattctgaactgaacatgagctccttggagctgggggactcagccctgtacttctgtgccagcagcttaggcctactggggaatgagcagttcttcgggccagggacacggctcaccgtgctagaggacctgaaaaacgtgttcccacccgaggtcgctgtgtttgagccatcagaagcagagatctcccacacccaaaaggccacactggtgtgcctggccacaggcttctaccccgaccacgtggagctgagctggtgggtgaatgggaaggaggtgcacagtggggtcagcacagacccgcagcccctcaaggagcagcccgccctcaatgactccagatactgcctgtcctcccgcctgagggtctcggccaccttctggcagaacccccgcaaccacttccgctgtcaagtccagttctacgggctctcggagaatgacgagtggacccaggatagggccaaacctgtcacccagatcgtcagcgccgaggcctggggtagagcagactgtggcttcacctccgagtcttaccagcaaggggtcctgtctgccaccatcctctatgagatcttgctagggaaggccaccttgtatgccgtgctggtcagtgccctcgtgctgatggccatggtcaagagaaaggattccagaggc

SEQ ID NO: 528 - DNA, 882 bp, synthetic construct
  source 1..882: mol_type = other DNA
gacacagctgtttcccagactccaaaatacctggtcacacagatgggaaacgacaagtccattaaatgtgaacaaaatctgggccatgatactatgtattggtataaacaggactctaagaaatttctgaagataatgtttagctacaataataaggagctcattataaatgaaacagttccaaatcgcttctcacctaaatctccagacaaagctcacttaaatcttcacatcaattccctggagcttggtgactctgctgtgtatttctgtgccagcagcccgtggactagcgggggaaacggggagctgttttttggagaaggctctaggctgaccgtactggaggacctgaaaaacgtgttcccacccgaggtcgctgtgtttgagccatcagaagcagagatctcccacacccaaaaggccacactggtgtgcctggccacaggcttctaccccgaccacgtggagctgagctggtgggtgaatgggaaggaggtgcacagtggggtcagcacagacccgcagcccctcaaggagcagcccgccctcaatgactccagatactgcctgtcctcccgcctgagggtctcggccaccttctggcagaacccccgcaaccacttccgctgtcaagtccagttctacgggctctcggagaatgacgagtggacccaggatagggccaaacctgtcacccagatcgtcagcgccgaggcctggggtagagcagactgtggcttcacctccgagtcttaccagcaaggggtcctgtctgccaccatcctctatgagatcttgctagggaaggccaccttgtatgccgtgctggtcagtgccctcgtgctgatggccatggtcaagagaaaggattccagaggc

SEQ ID NO: 529 - DNA, 873 bp, synthetic construct
  source 1..873: mol_type = other DNA
gacacagctgtttcccagactccaaaatacctggtcacacagatgggaaacgacaagtccattaaatgtgaacaaaatctgggccatgatactatgtattggtataaacaggactctaagaaatttctgaagataatgtttagctacaataataaggagctcattataaatgaaacagttccaaatcgcttctcacctaaatctccagacaaagctcacttaaatcttcacatcaattccctggagcttggtgactctgctgtgtatttctgtgccagcagccccggactagcctacgagcagtacttcgggccgggcaccaggctcacggtcacagaggacctgaaaaacgtgttcccacccgaggtcgctgtgtttgagccatcagaagcagagatctcccacacccaaaaggccacactggtgtgcctggccacaggcttctaccccgaccacgtggagctgagctggtgggtgaatgggaaggaggtgcacagtggggtcagcacagacccgcagcccctcaaggagcagcccgccctcaatgactccagatactgcctgtcctcccgcctgagggtctcggccaccttctggcagaacccccgcaaccacttccgctgtcaagtccagttctacgggctctcggagaatgacgagtggacccaggatagggccaaacctgtcacccagatcgtcagcgccgaggcctggggtagagcagactgtggcttcacctccgagtcttaccagcaaggggtcctgtctgccaccatcctctatgagatcttgctagggaaggccaccttgtatgccgtgctggtcagtgccctcgtgctgatggccatggtcaagagaaaggattccagaggc

SEQ ID NO: 530 - DNA, 873 bp, synthetic construct
  source 1..873: mol_type = other DNA
gaagcccaagtgacccagaacccaagatacctcatcacagtgactggaaagaagttaacagtgacttgttctcagaatatgaaccatgagtatatgtcctggtatcgacaagacccagggctgggcttaaggcagatctactattcaatgaatgttgaggtgactgataagggagatgttcctgaagggtacaaagtctctcgaaaagagaagaggaatttccccctgatcctggagtcgcccagccccaaccagacctctctgtacttctgtgccagcagtgccgggacagggggcttcgttggctacaccttcggttcggggaccaggttaaccgttgtagaggacctgaacaaggtgttcccacccgaggtcgctgtgtttgagccatcagaagcagagatctcccacacccaaaaggccacactggtgtgcctggccacaggcttcttccctgaccacgtggagctgagctggtgggtgaatgggaaggaggtgcacagtggggtcagcacggacccgcagcccctcaaggagcagcccgccctcaatgactccagatactgcctgtcctcccgcctgagggtctcggccaccttctggcagaacccccgcaaccacttccgctgtcaagtccagttctacgggctctcggagaatgacgagtggacccaggatagggccaaacccgtcacccagatcgtcagcgccgaggcctggggtagagcagactgtggctttacctcggtgtcctaccagcaaggggtcctgtctgccaccatcctctatgagatcctgctagggaaggccaccctgtatgctgtgctggtcagcgcccttgtgttgatggccatggtcaagagaaaggatttc

SEQ ID NO: 531 - DNA, 888 bp, synthetic construct
  source 1..888: mol_type = other DNA
agtgctgtcatctctcaaaagccaagcagggatatctgtcaacgtggaacctccctgacgatccagtgtcaagtcgatagccaagtcaccatgatgttctggtaccgtcagcaacctggacagagcctgacactgatcgcaactgcaaatcagggctctgaggccacatatgagagtggatttgtcattgacaagtttcccatcagccgcccaaacctaacattctcaactctgactgtgagcaacatgagccctgaagacagcagcatatatctctgcagcgtttggggagcgggactagcgatctacaatgagcagttcttcgggccagggacacggctcaccgtgctagaggacctgaaaaacgtgttcccacccgaggtcgctgtgtttgagccatcagaagcagagatctcccacacccaaaaggccacactggtgtgcctggccacaggcttctaccccgaccacgtggagctgagctggtgggtgaatgggaaggaggtgcacagtggggtcagcacagacccgcagcccctcaaggagcagcccgccctcaatgactccagatactgcctgtcctcccgcctgagggtctcggccaccttctggcagaacccccgcaaccacttccgctgtcaagtccagttctacgggctctcggagaatgacgagtggacccaggatagggccaaacctgtcacccagatcgtcagcgccgaggcctggggtagagcagactgtggcttcacctccgagtcttaccagcaaggggtcctgtctgccaccatcctctatgagatcttgctagggaaggccaccttgtatgccgtgctggtcagtgccctcgtgctgatggccatggtcaagagaaaggattccagaggc

SEQ ID NO: 532 - DNA, 879 bp, synthetic construct
  source 1..879: mol_type = other DNA
gatgtgaaagtaacccagagctcgagatatctagtcaaaaggacgggagagaaagtttttctggaatgtgtccaggatatggaccatgaaaatatgttctggtatcgacaagacccaggtctggggctacggctgatctatttctcatatgatgttaaaatgaaagaaaaaggagatattcctgaggggtacagtgtctctagagagaagaaggagcgcttctccctgattctggagtccgccagcaccaaccagacatctatgtacctctgtgccagcagttccgcgactagcgggagcggcgagcagtacttcgggccgggcaccaggctcacggtcacagaggacctgaaaaacgtgttcccacccgaggtcgctgtgtttgagccatcagaagcagagatctcccacacccaaaaggccacactggtgtgcctggccacaggcttctaccccgaccacgtggagctgagctggtgggtgaatgggaaggaggtgcacagtggggtcagcacagacccgcagcccctcaaggagcagcccgccctcaatgactccagatactgcctgtcctcccgcctgagggtctcggccaccttctggcagaacccccgcaaccacttccgctgtcaagtccagttctacgggctctcggagaatgacgagtggacccaggatagggccaaacctgtcacccagatcgtcagcgccgaggcctggggtagagcagactgtggcttcacctccgagtcttaccagcaaggggtcctgtctgccaccatcctctatgagatcttgctagggaaggccaccttgtatgccgtgctggtcagtgccctcgtgctgatggccatggtcaagagaaaggattccagaggc

SEQ ID NO: 533 - DNA, 882 bp, synthetic construct
  source 1..882: mol_type = other DNA
gaagcccaagtgacccagaacccaagatacctcatcacagtgactggaaagaagttaacagtgacttgttctcagaatatgaaccatgagtatatgtcctggtatcgacaagacccagggctgggcttaaggcagatctactattcaatgaatgttgaggtgactgataagggagatgttcctgaagggtacaaagtctctcgaaaagagaagaggaatttccccctgatcctggagtcgcccagccccaaccagacctctctgtacttctgtgccagcagtatcgatagcgggagctcctacaatgagcagttcttcgggccagggacacggctcaccgtgctagaggacctgaaaaacgtgttcccacccgaggtcgctgtgtttgagccatcagaagcagagatctcccacacccaaaaggccacactggtgtgcctggccacaggcttctaccccgaccacgtggagctgagctggtgggtgaatgggaaggaggtgcacagtggggtcagcacagacccgcagcccctcaaggagcagcccgccctcaatgactccagatactgcctgtcctcccgcctgagggtctcggccaccttctggcagaacccccgcaaccacttccgctgtcaagtccagttctacgggctctcggagaatgacgagtggacccaggatagggccaaacctgtcacccagatcgtcagcgccgaggcctggggtagagcagactgtggcttcacctccgagtcttaccagcaaggggtcctgtctgccaccatcctctatgagatcttgctagggaaggccaccttgtatgccgtgctggtcagtgccctcgtgctgatggccatggtcaagagaaaggattccagaggc

SEQ ID NO: 534 - DNA, 873 bp, synthetic construct
  source 1..873: mol_type = other DNA
gaacctgaagtcacccagactcccagccatcaggtcacacagatgggacaggaagtgatcttgcgctgtgtccccatctctaatcacttatacttctattggtacagacaaatcttggggcagaaagtcgagtttctggtttccttttataataatgaaatctcagagaagtctgaaatattcgatgatcaattctcagttgaaaggcctgatggatcaaatttcactctgaagatccggtccacaaagctggaggactcagccatgtacttctgtgccagcagtgaagggtgggggggcactgaagctttctttggacaaggcaccagactcacagttgtagaggacctgaacaaggtgttcccacccgaggtcgctgtgtttgagccatcagaagcagagatctcccacacccaaaaggccacactggtgtgcctggccacaggcttcttccctgaccacgtggagctgagctggtgggtgaatgggaaggaggtgcacagtggggtcagcacggacccgcagcccctcaaggagcagcccgccctcaatgactccagatactgcctgtcctcccgcctgagggtctcggccaccttctggcagaacccccgcaaccacttccgctgtcaagtccagttctacgggctctcggagaatgacgagtggacccaggatagggccaaacccgtcacccagatcgtcagcgccgaggcctggggtagagcagactgtggctttacctcggtgtcctaccagcaaggggtcctgtctgccaccatcctctatgagatcctgctagggaaggccaccctgtatgctgtgctggtcagcgcccttgtgttgatggccatggtcaagagaaaggatttc

SEQ ID NO: 535 - protein, 235 aa, synthetic construct
MALPVTALLLPLALLLHAARPSQFRVSPLDRTWNLGETVELKCQVLLSNPTSGCSWLFQPRGAAASPTFLLYLSQNKPKAAEGLDTQRFSGKRLGDTFVLTLSDFRRENEGYYFCSALSNSIMYFSHFVPVFLPAKPTTTPAPRPPTPAPTIASQPLSLRPEACRPAAGGAVHTRGLDFACDIYIWAPLAGTCGVLLLSLVITLYCNHRNRRRVCKCPRPVVKSGDKPSLSARYV

SEQ ID NO: 536 - DNA, 705 bp, synthetic construct
  source 1..705: mol_type = other DNA
atggccttaccagtgaccgccttgctcctgccgctggccttgctgctccacgccgccaggccgagccagttccgggtgtcgccgctggatcggacctggaacctgggcgagacagtggagctgaagtgccaggtgctgctgtccaacccgacgtcgggctgctcgtggctcttccagccgcgcggcgccgccgccagtcccaccttcctcctatacctctcccaaaacaagcccaaggcggccgaggggctggacacccagcggttctcgggcaagaggttgggggacaccttcgtcctcaccctgagcgacttccgccgagagaacgagggctactatttctgctcggccctgagcaactccatcatgtacttcagccacttcgtgccggtcttcctgccagcgaagcccaccacgacgccagcgccgcgaccaccaacaccggcgcccaccatcgcgtcgcagcccctgtccctgcgcccagaggcgtgccggccagcggcggggggcgcagtgcacacgagggggctggacttcgcctgtgatatctacatctgggcgcccttggccgggacttgtggggtccttctcctgtcactggttatcaccctttactgcaaccacaggaaccgaagacgtgtttgcaaatgtccccggcctgtggtcaaatcgggagacaagcccagcctttcggcgagatacgtc

SEQ ID NO: 537 - protein, 210 aa, synthetic construct
MRPRLWLLLAAQLTVLHGNSVLQQTPAYIKVQTNKMVMLSCEAKISLSNMRIYWLRQRQAPSSDSHHEFLALWDSAKGTIHGEEVEQEKIAVFRDASRFILNLTSVKPEDSGIYFCMIVGSPELTFGKGTQLSVVDFLPTTAQPTKKSTLKKRVCRLPRPETQKGPLCSPITLGLLVAGVLVLLVSLGVAIHLCCRRRRARLRFMKQFYK

SEQ ID NO: 538 - DNA, 630 bp, synthetic construct
  source 1..630: mol_type = other DNA
atgcggccgcggctgtggctcctcttggccgcgcagctgacagttctccatggcaactcagtcctccagcagacccctgcatacataaaggtgcaaaccaacaagatggtgatgctgtcctgcgaggctaaaatctccctcagtaacatgcgcatctactggctgagacagcgccaggcaccgagcagtgacagtcaccacgagttcctggccctctgggattccgcaaaagggactatccacggtgaagaggtggaacaggagaagatagctgtgtttcgggatgcaagccggttcattctcaatctcacaagcgtgaagccggaagacagtggcatctacttctgcatgatcgtcgggagccccgagctgaccttcgggaagggaactcagctgagtgtggttgatttccttcccaccactgcccagcccaccaagaagtccaccctcaagaagagagtgtgccggttacccaggccagagacccagaagggcccactttgtagccccatcacccttggcctgctggtggctggcgtcctggttctgctggtttccctgggagtggccatccacctgtgctgccggcggaggagagcccggcttcgtttcatgaaacaattttacaaa

SEQ ID NO: 539 - protein, 1004 aa, synthetic construct
GSGATNFSLLKQAGDVEENPGPMALPVTALLLPLALLLHAARPSQFRVSPLDRTWNLGETVELKCQVLLSNPTSGCSWLFQPRGAAASPTFLLYLSQNKPKAAEGLDTQRFSGKRLGDTFVLTLSDFRRENEGYYFCSALSNSIMYFSHFVPVFLPAKPTTTPAPRPPTPAPTIASQPLSLRPEACRPAAGGAVHTRGLDFACDIYIWAPLAGTCGVLLLSLVITLYCNHRNRRRVCKCPRPVVKSGDKPSLSARYVRAKRGSGQCTNYALLKLAGDVESNPGPMRPRLWLLLAAQLTVLHGNSVLQQTPAYIKVQTNKMVMLSCEAKISLSNMRIYWLRQRQAPSSDSHHEFLALWDSAKGTIHGEEVEQEKIAVFRDASRFILNLTSVKPEDSGIYFCMIVGSPELTFGKGTQLSVVDFLPTTAQPTKKSTLKKRVCRLPRPETQKGPLCSPITLGLLVAGVLVLLVSLGVAIHLCCRRRRARLRFMKQFYKRAKRGSGEGRGSLLTCGDVEENPGPMATGSRTSLLLAFGLLCLPWLQEGSAKAGVTQTPRYLIKTRGQQVTLSCSPISGHRSVSWYQQTPGQGLQFLFEYFSETQRNKGNFPGRFSGRQFSNSRSEMNVSTLELGDSALYLCASSLEAGSFYEQYFGPGTRLTVTEDLKNVFPPEVAVFEPSEAEISHTQKATLVCLATGFYPDHVELSWWVNGKEVHSGVSTDPQPLKEQPALNDSRYCLSSRLRVSATFWQNPRNHFRCQVQFYGLSENDEWTQDRAKPVTQIVSAEAWGRADCGFTSESYQQGVLSATILYEILLGKATLYAVLVSALVLMAMVKRKDSRGRAKRGSGATNFSLLKQAGDVEENPGPMATGSRTSLLLAFGLLCLPWLQEGSAGEDVEQSLFLSVREGDSSVINCTYTDSSSTYLYWYKQEPGAGLQLLTYIFSNMDMKQDQRLTVLLNKKDKHLSLRIADTQTGDSAIYFCAESVGYGGSQGNLIFGKGTKLSVKP

SEQ ID NO: 540 - DNA, 3013 bp, synthetic construct
  source 1..3013: mol_type = other DNA
ggcagcggcgccaccaacttcagcctgctgaagcaggccggcgacgtggaggagaaccccggccccatggccttaccagtgaccgccttgctcctgccgctggccttgctgctccacgccgccaggccgagccagttccgggtgtcgccgctggatcggacctggaacctgggcgagacagtggagctgaagtgccaggtgctgctgtccaacccgacgtcgggctgctcgtggctcttccagccgcgcggcgccgccgccagtcccaccttcctcctatacctctcccaaaacaagcccaaggcggccgaggggctggacacccagcggttctcgggcaagaggttgggggacaccttcgtcctcaccctgagcgacttccgccgagagaacgagggctactatttctgctcggccctgagcaactccatcatgtacttcagccacttcgtgccggtcttcctgccagcgaagcccaccacgacgccagcgccgcgaccaccaacaccggcgcccaccatcgcgtcgcagcccctgtccctgcgcccagaggcgtgccggccagcggcggggggcgcagtgcacacgagggggctggacttcgcctgtgatatctacatctgggcgcccttggccgggacttgtggggtccttctcctgtcactggttatcaccctttactgcaaccacaggaaccgaagacgtgtttgcaaatgtccccggcctgtggtcaaatcgggagacaagcccagcctttcggcgagatacgtcagagccaaaagaggaagcggacagtgtactaattatgctctcttgaaattggctggagatgttgagagcaacccaggtcccatgcggccgcggctgtggctcctcttggccgcgcagctgacagttctccatggcaactcagtcctccagcagacccctgcatacataaaggtgcaaaccaacaagatggtgatgctgtcctgcgaggctaaaatctccctcagtaacatgcgcatctactggctgagacagcgccaggcaccgagcagtgacagtcaccacgagttcctggccctctgggattccgcaaaagggactatccacggtgaagaggtggaacaggagaagatagctgtgtttcgggatgcaagccggttcattctcaatctcacaagcgtgaagccggaagacagtggcatctacttctgcatgatcgtcgggagccccgagctgaccttcgggaagggaactcagctgagtgtggttgatttccttcccaccactgcccagcccaccaagaagtccaccctcaagaagagagtgtgccggttacccaggccagagacccagaagggcccactttgtagccccatcacccttggcctgctggtggctggcgtcctggttctgctggtttccctgggagtggccatccacctgtgctgccggcggaggagagcccggcttcgtttcatgaaacaattttacaaaagagccaaaagaggaagcggagagggcaggggaagtcttctaacatgcggggacgtggaggaaaatcccggccccatggccaccggcagcaggaccagcctgctgctggccttcggcctgctgtgcctgccctggctgcaggagggcagcgccaaggctggagtcactcaaactccaagatatctgatcaaaacgagaggacagcaagtgacactgagctgctcccctatctctgggcataggagtgtatcctggtaccaacagaccccaggacagggccttcagttcctctttgaatacttcagtgagacacagagaaacaaaggaaacttccctggtcgattctcagggcgccagttctctaactctcgctctgagatgaatgtgagcaccttggagctgggggactcggccctttatctttgcgccagcagcttggaggcagggtcattctacgagcagtacttcgggccgggcaccaggctcacggtcacagaggacctgaaaaacgtgttcccacccgaggtcgctgtgtttgagccatcagaagcagagatctcccacacccaaaaggccacactggtgtgcctggccacaggcttctaccccgaccacgtggagctgagctggtgggtgaatgggaaggaggtgcacagtggggtcagcacagacccgcagcccctcaaggagcagcccgccctcaatgactccagatactgcctgtcctcccgcctgagggtctcggccaccttctggcagaacccccgcaaccacttccgctgtcaagtccagttctacgggctctcggagaatgacgagtggacccaggatagggccaaacctgtcacccagatcgtcagcgccgaggcctggggtagagcagactgtggcttcacctccgagtcttaccagcaaggggtcctgtctgccaccatcctctatgagatcttgctagggaaggccaccttgtatgccgtgctggtcagtgccctcgtgctgatggccatggtcaagagaaaggattccagaggccgggccaagcggggatccggagccacaaatttctccctgctgaaacaggccggcgatgtggaggagaatcctggacctatggccaccggcagcaggaccagcctgctgctggccttcggcctgctgtgcctgccctggctgcaggagggcagcgccggagaggatgtggagcagagtcttttcctgagtgtccgagagggagacagctccgttataaactgcacttacacagacagctcctccacctacttatactggtataagcaagaacctggagcaggtctccagttgctgacgtatattttttcaaatatggacatgaaacaagaccaaagactcactgttctattgaataaaaaggataaacatctgtctctgcgcattgcagacacccagactggggactcagctatctacttctgtgcagagagcgtggggtatggaggaagccaaggaaatctcatctttggaaaaggcactaaactctctgttaaaccaa

SEQ ID NO: 541 - protein, 9 aa, synthetic construct
SLLQHLIGL

SEQ ID NO: 542 - DNA, 20 bp, synthetic construct
  source 1..20: mol_type = other DNA
tcagggttctggatatctgt

SEQ ID NO: 543 - DNA, 20 bp, synthetic construct
  source 1..20: mol_type = other DNA
ctgcctgagcagccgcctga

SEQ ID NO: 544 - skipped

SEQ ID NO: 545 - DNA, 1524 bp, synthetic construct
  source 1..1524: mol_type = other DNA
ggcagcggcgccaccaacttcagcctgctgaagcaggccggcgacgtggaggagaaccccggccccatggccaccggcagcaggaccagcctgctgctggccttcggcctgctgtgcctgccctggctgcaggagggcagcgccaaggctggagtcactcaaactccaagatatctgatcaaaacgagaggacagcaagtgacactgagctgctcccctatctctgggcataggagtgtatcctggtaccaacagaccccaggacagggccttcagttcctctttgaatacttcagtgagacacagagaaacaaaggaaacttccctggtcgattctcagggcgccagttctctaactctcgctctgagatgaatgtgagcaccttggagctgggggactcggccctttatctttgcgccagcagcttggaggcagggtcattctacgagcagtacttcgggccgggcaccaggctcacggtcacagaggacctgaaaaacgtgttcccacccgaggtcgctgtgtttgagccatcagaagcagagatctcccacacccaaaaggccacactggtgtgcctggccacaggcttctaccccgaccacgtggagctgagctggtgggtgaatgggaaggaggtgcacagtggggtcagcacagacccgcagcccctcaaggagcagcccgccctcaatgactccagatactgcctgtcctcccgcctgagggtctcggccaccttctggcagaacccccgcaaccacttccgctgtcaagtccagttctacgggctctcggagaatgacgagtggacccaggatagggccaaacctgtcacccagatcgtcagcgccgaggcctggggtagagcagactgtggcttcacctccgagtcttaccagcaaggggtcctgtctgccaccatcctctatgagatcttgctagggaaggccaccttgtatgccgtgctggtcagtgccctcgtgctgatggccatggtcaagagaaaggattccagaggccgggccaagcggggatccggagccacaaatttctccctgctgaaacaggccggcgatgtggaggagaatcctggacctatggccaccggcagcaggaccagcctgctgctggccttcggcctgctgtgcctgccctggctgcaggagggcagcgccggagaggatgtggagcagagtcttttcctgagtgtccgagagggagacagctccgttataaactgcacttacacagacagctcctccacctacttatactggtataagcaagaacctggagcaggtctccagttgctgacgtatattttttcaaatatggacatgaaacaagaccaaagactcactgttctattgaataaaaaggataaacatctgtctctgcgcattgcagacacccagactggggactcagctatctacttctgtgcagagagcgtggggtatggaggaagccaaggaaatctcatctttggaaaaggcactaaactctctgttaaaccaaat

SEQ ID NO: 546 - protein, 508 aa, synthetic construct
GSGATNFSLLKQAGDVEENPGPMATGSRTSLLLAFGLLCLPWLQEGSAKAGVTQTPRYLIKTRGQQVTLSCSPISGHRSVSWYQQTPGQGLQFLFEYFSETQRNKGNFPGRFSGRQFSNSRSEMNVSTLELGDSALYLCASSLEAGSFYEQYFGPGTRLTVTEDLKNVFPPEVAVFEPSEAEISHTQKATLVCLATGFYPDHVELSWWVNGKEVHSGVSTDPQPLKEQPALNDSRYCLSSRLRVSATFWQNPRNHFRCQVQFYGLSENDEWTQDRAKPVTQIVSAEAWGRADCGFTSESYQQGVLSATILYEILLGKATLYAVLVSALVLMAMVKRKDSRGRAKRGSGATNFSLLKQAGDVEENPGPMATGSRTSLLLAFGLLCLPWLQEGSAGEDVEQSLFLSVREGDSSVINCTYTDSSSTYLYWYKQEPGAGLQLLTYIFSNMDMKQDQRLTVLLNKKDKHLSLRIADTQTGDSAIYFCAESVGYGGSQGNLIFGKGTKLSVKPN

SEQ ID NO: 547 - DNA, 66 bp, synthetic construct
  source 1..66: mol_type = other DNA
ggcagcggcgccaccaacttcagcctgctgaagcaggccggcgacgtggaggagaaccccggcccc

SEQ ID NO: 548 - DNA, 78 bp, synthetic construct
  source 1..78: mol_type = other DNA
atggccaccggcagcaggaccagcctgctgctggccttcggcctgctgtgcctgccctggctgcaggagggcagcgcc

SEQ ID NO: 549 - DNA, 78 bp, synthetic construct
  source 1..78: mol_type = other DNA
cgggccaagcggggatccggagccacaaatttctccctgctgaaacaggccggcgatgtggaggagaatcctggacct

SEQ ID NO: 550 - protein, 1368 aa, synthetic construct [sequence omitted]